European Patent Application EP 4 707 395 A1, published March 11, 2026. Title: 光スイッチタンパク質. Applicant: 国立大学法人　東京大学. Application JP. The sequence listing filed with the application follows.

SEQUENCE LISTING (38 sequences)

SEQ ID NO: 1 - protein, 186 aa, Neurospora crassa
MSHTVNSSTMNPWEVEAYQQYHYDPRTAPTANPLFFHTLYAPGGYDIMGYLIQIMNRPNPQVELGPVDTSCALILCDLKQKDTPIVYASEAFLYMTGYSNAEVLGRNCRFLQSPDGMVKPKSTRKYVDSNTINTMRKAIDRNAEVQVEVVNFKKNGQRFVNFLTMIPVRDETGEYRYSMGFQCETE

SEQ ID NO: 2 - DNA, 24 bp, synthetic construct
  source 1..24: mol_type = other DNA
caccggtgagtgagtgtgtgcgtg

SEQ ID NO: 3 - DNA, 24 bp, synthetic construct
  source 1..24: mol_type = other DNA
aaaccacgcacacactcactcacc

SEQ ID NO: 4 - DNA, 25 bp, synthetic construct
  source 1..25: mol_type = other DNA
caccgccgtttccctcactcctgct

SEQ ID NO: 5 - DNA, 25 bp, synthetic construct
  source 1..25: mol_type = other DNA
aaacagcaggagtgagggaaacggc

SEQ ID NO: 6 - DNA, 24 bp, synthetic construct
  source 1..24: mol_type = other DNA
caccgagtccgagcagaagaagaa

SEQ ID NO: 7 - DNA, 24 bp, synthetic construct
  source 1..24: mol_type = other DNA
aaacttcttcttctgctcggactc

SEQ ID NO: 8 - DNA, 24 bp, synthetic construct
  source 1..24: mol_type = other DNA
caccgctaattcagaatcactttg

SEQ ID NO: 9 - DNA, 24 bp, synthetic construct
  source 1..24: mol_type = other DNA
aaaccaaagtgattctgaattagc

SEQ ID NO: 10 - DNA, 20 bp, synthetic construct
  source 1..20: mol_type = other DNA
tccagatggcacattgtcag

SEQ ID NO: 11 - DNA, 20 bp, synthetic construct
  source 1..20: mol_type = other DNA
agggagcaggaaagtgaggt

SEQ ID NO: 12 - DNA, 22 bp, synthetic construct
  source 1..22: mol_type = other DNA
agcccgagagagtgcctcaggt

SEQ ID NO: 13 - DNA, 26 bp, synthetic construct
  source 1..26: mol_type = other DNA
ccacacatgtgaacggacagattgac

SEQ ID NO: 14 - DNA, 20 bp, synthetic construct
  source 1..20: mol_type = other DNA
ggagcagctggtcagagggg

SEQ ID NO: 15 - DNA, 20 bp, synthetic construct
  source 1..20: mol_type = other DNA
gggaagggggacactgggga

SEQ ID NO: 16 - DNA, 21 bp, synthetic construct
  source 1..21: mol_type = other DNA
gtcgacaagctcatgcgggtg

SEQ ID NO: 17 - DNA, 28 bp, synthetic construct
  source 1..28: mol_type = other DNA
caaaatgcaaatacaaagcacggatggc

SEQ ID NO: 18 - DNA, 8164 bp, synthetic construct
  source 1..8164: mol_type = other DNA
  misc_feature 923..967: note = NLS
  misc_feature 968..3103: note = Cas9 N-ter
  misc_feature 3140..3589: note = pMag
gacggatcgggagatctcccgatcccctatggtgcactctcagtacaatctgctctgatgccgcatagttaagccagtatctgctccctgcttgtgtgttggaggtcgctgagtagtgcgcgagcaaaatttaagctacaacaaggcaaggcttgaccgacaattgcatgaagaatctgcttagggttaggcgttttgcgctgcttcgcgatgtacgggccagatatacgcgttgacattgattattgactagttattaatagtaatcaattacggggtcattagttcatagcccatatatggagttccgcgttacataacttacggtaaatggcccgcctggctgaccgcccaacgacccccgcccattgacgtcaataatgacgtatgttcccatagtaacgccaatagggactttccattgacgtcaatgggtggagtatttacggtaaactgcccacttggcagtacatcaagtgtatcatatgccaagtacgccccctattgacgtcaatgacggtaaatggcccgcctggcattatgcccagtacatgaccttatgggactttcctacttggcagtacatctacgtattagtcatcgctattaccatggtgatgcggttttggcagtacatcaatgggcgtggatagcggtttgactcacggggatttccaagtctccaccccattgacgtcaatgggagtttgttttggcaccaaaatcaacgggactttccaaaatgtcgtaacaactccgccccattgacgcaaatgggcggtaggcgtgtacggtgggaggtctatataagcagagctctctggctaactagagaacccactgcttactggcttatcgaaattaatacgactcactatagggagacccaagctggctagttaagcttgccaccatgggtaccccaaagaagaagcggaaggtcggtatccacggagtcccagcagccgacaagaagtacagcatcggcctggacatcggcaccaactctgtgggctgggccgtgatcaccgacgagtacaaggtgcccagcaagaaattcaaggtgctgggcaacaccgaccggcacagcatcaagaagaacctgatcggagccctgctgttcgacagcggcgaaacagccgaggccacccggctgaagagaaccgccagaagaagatacaccagacggaagaaccggatctgctatctgcaagagatcttcagcaacgagatggccaaggtggacgacagcttcttccacagactggaagagtccttcctggtggaagaggataagaagcacgagcggcaccccatcttcggcaacatcgtggacgaggtggcctaccacgagaagtaccccaccatctaccacctgagaaagaaactggtggacagcaccgacaaggccgacctgcggctgatctatctggccctggcccacatgatcaagttccggggccacttcctgatcgagggcgacctgaaccccgacaacagcgacgtggacaagctgttcatccagctggtgcagacctacaaccagctgttcgaggaaaaccccatcaacgccagcggcgtggacgccaaggccatcctgtctgccagactgagcaagagcagacggctggaaaatctgatcgcccagctgcccggcgagaagaagaatggcctgttcggaaacctgattgccctgagcctgggcctgacccccaacttcaagagcaacttcgacctggccgaggatgccaaactgcagctgagcaaggacacctacgacgacgacctggacaacctgctggcccagatcggcgaccagtacgccgacctgtttctggccgccaagaacctgtccgacgccatcctgctgagcgacatcctgagagtgaacaccgagatcaccaaggcccccctgagcgcctctatgatcaagagatacgacgagcaccaccaggacctgaccctgctgaaagctctcgtgcggcagcagctgcctgagaagtacaaagagattttcttcgaccagagcaagaacggctacgccggctacattgacggcggagccagccaggaagagttctacaagttcatcaagcccatcctggaaaagatggacggcaccgaggaactgctcgtgaagctgaacagagaggacctgctgcggaagcagcggaccttcgacaacggcagcatcccccaccagatccacctgggagagctgcacgccattctgcggcggcaggaagatttttacccattcctgaaggacaaccgggaaaagatcgagaagatcctgaccttccgcatcccctactacgtgggccctctggccaggggaaacagcagattcgcctggatgaccagaaagagcgaggaaaccatcaccccctggaacttcgaggaagtggtggacaagggcgcttccgcccagagcttcatcgagcggatgaccaacttcgataagaacctgcccaacgagaaggtgctgcccaagcacagcctgctgtacgagtacttcaccgtgtataacgagctgaccaaagtgaaatacgtgaccgagggaatgagaaagcccgccttcctgagcggcgagcagaaaaaggccatcgtggacctgctgttcaagaccaaccggaaagtgaccgtgaagcagctgaaagaggactacttcaagaaaatcgagtgcttcgactccgtggaaatctccggcgtggaagatcggttcaacgcctccctgggcacataccacgatctgctgaaaattatcaaggacaaggacttcctggacaatgaggaaaacgaggacattctggaagatatcgtgctgaccctgacactgtttgaggacagagagatgatcgaggaacggctgaaaacctatgcccacctgttcgacgacaaagtgatgaagcagctgaagcggcggagatacaccggctggggcaggctgagccggaagctgatcaacggcatccgggacaagcagtccggcaagacaatcctggatttcctgaagtccgacggcttcgccaacagaaacttcatgcagctgatccacgacgacagcctgacctttaaagaggacatccagaaagcccaggtggaattcggaggaagtggcagctctggcggcagcggacatactctttatgcccccggtggatatgacattatgggatatctgaggcagatcaggaaccggccaaacccgcaggtggaactgggccccgtggatacatcctgcgccttgattctttgtgacctgaaacagaaagacaccccgatagtttacgcgagtgaagccttcctctacatgacaggttacagcaacgcagaggtgctgggccggaattgccggtttctgcaaagccctgacggcatggtgaagcccaagagcacccggaagtacgtggatagtaacacaatcaatactatgcgcaaggcaatcgacaggaatgccgaggtgcaggttgaagtagtcaattttaaaaagaatggacagcgatttgttaatttcctgactatgatacctgttagggacgaaacaggcgagtatcgatactctatgggattccagtgcgaaacagaagggggttctggggggagcggcgggggatctggaagtggcagcggaggcctcgagtctagagggcccttcgaaggtaagcctatccctaaccctctcctcggtctcgattctacgcgtaccggtcatcatcaccatcaccattgagtttaaacccgctgatcagcctcgactgtgccttctagttgccagccatctgttgtttgcccctcccccgtgccttccttgaccctggaaggtgccactcccactgtcctttcctaataaaatgaggaaattgcatcgcattgtctgagtaggtgtcattctattctggggggtggggtggggcaggacagcaagggggaggattgggaagacaatagcaggcatgctggggatgcggtgggctctatggcttctgaggcggaaagaaccagctggggctctagggggtatccccacgcgccctgtagcggcgcattaagcgcggcgggtgtggtggttacgcgcagcgtgaccgctacacttgccagcgccctagcgcccgctcctttcgctttcttcccttcctttctcgccacgttcgccggctttccccgtcaagctctaaatcgggggctccctttagggttccgatttagtgctttacggcacctcgaccccaaaaaacttgattagggtgatggttcacgtagtgggccatcgccctgatagacggtttttcgccctttgacgttggagtccacgttctttaatagtggactcttgttccaaactggaacaacactcaaccctatctcggtctattcttttgatttataagggattttgccgatttcggcctattggttaaaaaatgagctgatttaacaaaaatttaacgcgaattaattctgtggaatgtgtgtcagttagggtgtggaaagtccccaggctccccagcaggcagaagtatgcaaagcatgcatctcaattagtcagcaaccaggtgtggaaagtccccaggctccccagcaggcagaagtatgcaaagcatgcatctcaattagtcagcaaccatagtcccgcccctaactccgcccatcccgcccctaactccgcccagttccgcccattctccgccccatggctgactaattttttttatttatgcagaggccgaggccgcctctgcctctgagctattccagaagtagtgaggaggcttttttggaggcctaggcttttgcaaaaagctcccgggagcttgtatatccattttcggatctgatcaagagacaggatgaggatcgtttcgcatgattgaacaagatggattgcacgcaggttctccggccgcttgggtggagaggctattcggctatgactgggcacaacagacaatcggctgctctgatgccgccgtgttccggctgtcagcgcaggggcgcccggttctttttgtcaagaccgacctgtccggtgccctgaatgaactgcaggacgaggcagcgcggctatcgtggctggccacgacgggcgttccttgcgcagctgtgctcgacgttgtcactgaagcgggaagggactggctgctattgggcgaagtgccggggcaggatctcctgtcatctcaccttgctcctgccgagaaagtatccatcatggctgatgcaatgcggcggctgcatacgcttgatccggctacctgcccattcgaccaccaagcgaaacatcgcatcgagcgagcacgtactcggatggaagccggtcttgtcgatcaggatgatctggacgaagagcatcaggggctcgcgccagccgaactgttcgccaggctcaaggcgcgcatgcccgacggcgaggatctcgtcgtgacccatggcgatgcctgcttgccgaatatcatggtggaaaatggccgcttttctggattcatcgactgtggccggctgggtgtggcggaccgctatcaggacatagcgttggctacccgtgatattgctgaagagcttggcggcgaatgggctgaccgcttcctcgtgctttacggtatcgccgctcccgattcgcagcgcatcgccttctatcgccttcttgacgagttcttctgagcgggactctggggttcgcgaaatgaccgaccaagcgacgcccaacctgccatcacgagatttcgattccaccgccgccttctatgaaaggttgggcttcggaatcgttttccgggacgccggctggatgatcctccagcgcggggatctcatgctggagttcttcgcccaccccaacttgtttattgcagcttataatggttacaaataaagcaatagcatcacaaatttcacaaataaagcatttttttcactgcattctagttgtggtttgtccaaactcatcaatgtatcttatcatgtctgtataccgtcgacctctagctagagcttggcgtaatcatggtcatagctgtttcctgtgtgaaattgttatccgctcacaattccacacaacatacgagccggaagcataaagtgtaaagcctggggtgcctaatgagtgagctaactcacattaattgcgttgcgctcactgcccgctttccagtcgggaaacctgtcgtgccagctgcattaatgaatcggccaacgcgcggggagaggcggtttgcgtattgggcgctcttccgcttcctcgctcactgactcgctgcgctcggtcgttcggctgcggcgagcggtatcagctcactcaaaggcggtaatacggttatccacagaatcaggggataacgcaggaaagaacatgtgagcaaaaggccagcaaaaggccaggaaccgtaaaaaggccgcgttgctggcgtttttccataggctccgcccccctgacgagcatcacaaaaatcgacgctcaagtcagaggtggcgaaacccgacaggactataaagataccaggcgtttccccctggaagctccctcgtgcgctctcctgttccgaccctgccgcttaccggatacctgtccgcctttctcccttcgggaagcgtggcgctttctcatagctcacgctgtaggtatctcagttcggtgtaggtcgttcgctccaagctgggctgtgtgcacgaaccccccgttcagcccgaccgctgcgccttatccggtaactatcgtcttgagtccaacccggtaagacacgacttatcgccactggcagcagccactggtaacaggattagcagagcgaggtatgtaggcggtgctacagagttcttgaagtggtggcctaactacggctacactagaagaacagtatttggtatctgcgctctgctgaagccagttaccttcggaaaaagagttggtagctcttgatccggcaaacaaaccaccgctggtagcggtggtttttttgtttgcaagcagcagattacgcgcagaaaaaaaggatctcaagaagatcctttgatcttttctacggggtctgacgctcagtggaacgaaaactcacgttaagggattttggtcatgagattatcaaaaaggatcttcacctagatccttttaaattaaaaatgaagttttaaatcaatctaaagtatatatgagtaaacttggtctgacagttaccaatgcttaatcagtgaggcacctatctcagcgatctgtctatttcgttcatccatagttgcctgactccccgtcgtgtagataactacgatacgggagggcttaccatctggccccagtgctgcaatgataccgcgagacccacgctcaccggctccagatttatcagcaataaaccagccagccggaagggccgagcgcagaagtggtcctgcaactttatccgcctccatccagtctattaattgttgccgggaagctagagtaagtagttcgccagttaatagtttgcgcaacgttgttgccattgctacaggcatcgtggtgtcacgctcgtcgtttggtatggcttcattcagctccggttcccaacgatcaaggcgagttacatgatcccccatgttgtgcaaaaaagcggttagctccttcggtcctccgatcgttgtcagaagtaagttggccgcagtgttatcactcatggttatggcagcactgcataattctcttactgtcatgccatccgtaagatgcttttctgtgactggtgagtactcaaccaagtcattctgagaatagtgtatgcggcgaccgagttgctcttgcccggcgtcaatacgggataataccgcgccacatagcagaactttaaaagtgctcatcattggaaaacgttcttcggggcgaaaactctcaaggatcttaccgctgttgagatccagttcgatgtaacccactcgtgcacccaactgatcttcagcatcttttactttcaccagcgtttctgggtgagcaaaaacaggaaggcaaaatgccgcaaaaaagggaataagggcgacacggaaatgttgaatactcatactcttcctttttcaatattattgaagcatttatcagggttattgtctcatgagcggatacatatttgaatgtatttagaaaaataaacaaataggggttccgcgcacatttccccgaaaagtgccacctgacgtc

SEQ ID NO: 19 - DNA, 7993 bp, synthetic construct
  source 1..7993: mol_type = other DNA
  misc_feature 965..1414: note = nMagHigh1
  misc_feature 1469..3433: note = Cas9 C-term
  misc_feature 3440..3466: note = NLS
gacggatcgggagatctcccgatcccctatggtgcactctcagtacaatctgctctgatgccgcatagttaagccagtatctgctccctgcttgtgtgttggaggtcgctgagtagtgcgcgagcaaaatttaagctacaacaaggcaaggcttgaccgacaattgcatgaagaatctgcttagggttaggcgttttgcgctgcttcgcgatgtacgggccagatatacgcgttgacattgattattgactagttattaatagtaatcaattacggggtcattagttcatagcccatatatggagttccgcgttacataacttacggtaaatggcccgcctggctgaccgcccaacgacccccgcccattgacgtcaataatgacgtatgttcccatagtaacgccaatagggactttccattgacgtcaatgggtggagtatttacggtaaactgcccacttggcagtacatcaagtgtatcatatgccaagtacgccccctattgacgtcaatgacggtaaatggcccgcctggcattatgcccagtacatgaccttatgggactttcctacttggcagtacatctacgtattagtcatcgctattaccatggtgatgcggttttggcagtacatcaatgggcgtggatagcggtttgactcacggggatttccaagtctccaccccattgacgtcaatgggagtttgttttggcaccaaaatcaacgggactttccaaaatgtcgtaacaactccgccccattgacgcaaatgggcggtaggcgtgtacggtgggaggtctatataagcagagctctctggctaactagagaacccactgcttactggcttatcgaaattaatacgactcactatagggagacccaagctggctagttaagcttgccaccatgggaggaagtggcagctctggcggcagtggagggtctggtggcagcggacatactctttatgcccccggtggatatgacattatgggatatctggaccagatcggcaaccggccaaacccgcaggtggaactgggccccgtggatacatcctgcgccttgattctttgtgacctgaaacagaaagacaccccgatagtttacgcgagtgaagccttcctctacatgacaggttacagcaacgcagaggtgctgggccggaattgccggtttctgcaaagccctgacggcatggtgaagcccaagagcacccggaagtacgtggatagtaacacaatcaatactatccgcaaggcaatcgacaggaatgccgaggtgcaggttgaagtagtcaattttaaaaagaatggacagcgatttgttaatttcctgactatcatacctgttagggacgaaacaggcgagtatcgatactctatgggattccagtgcgaaacagaagggggttctggggggagcggcgggggatctggaagtggcagcggaggcggtacctccggccagggcgatagcctgcacgagcacattgccaatctggccggcagccccgccattaagaagggcatcctgcagacagtgaaggtggtggacgagctcgtgaaagtgatgggccggcacaagcccgagaacatcgtgatcgaaatggccagagagaaccagaccacccagaagggacagaagaacagccgcgagagaatgaagcggatcgaagagggcatcaaagagctgggcagccagatcctgaaagaacaccccgtggaaaacacccagctgcagaacgagaagctgtacctgtactacctgcagaatgggcgggatatgtacgtggaccaggaactggacatcaaccggctgtccgactacgatgtggaccatatcgtgcctcagagctttctgaaggacgactccatcgacaacaaggtgctgaccagaagcgacaagaaccggggcaagagcgacaacgtgccctccgaagaggtcgtgaagaagatgaagaactactggcggcagctgctgaacgccaagctgattacccagagaaagttcgacaatctgaccaaggccgagagaggcggcctgagcgaactggataaggccggcttcatcaagagacagctggtggaaacccggcagatcacaaagcacgtggcacagatcctggactcccggatgaacactaagtacgacgagaatgacaagctgatccgggaagtgaaagtgatcaccctgaagtccaagctggtgtccgatttccggaaggatttccagttttacaaagtgcgcgagatcaacaactaccaccacgcccacgacgcctacctgaacgccgtcgtgggaaccgccctgatcaaaaagtaccctaagctggaaagcgagttcgtgtacggcgactacaaggtgtacgacgtgcggaagatgatcgccaagagcgagcaggaaatcggcaaggctaccgccaagtacttcttctacagcaacatcatgaactttttcaagaccgagattaccctggccaacggcgagatccggaagcggcctctgatcgagacaaacggcgaaaccggggagatcgtgtgggataagggccgggattttgccaccgtgcggaaagtgctgagcatgccccaagtgaatatcgtgaaaaagaccgaggtgcagacaggcggcttcagcaaagagtctatcctgcccaagaggaacagcgataagctgatcgccagaaagaaggactgggaccctaagaagtacggcggcttcgacagccccaccgtggcctattctgtgctggtggtggccaaagtggaaaagggcaagtccaagaaactgaagagtgtgaaagagctgctggggatcaccatcatggaaagaagcagcttcgagaagaatcccatcgactttctggaagccaagggctacaaagaagtgaaaaaggacctgatcatcaagctgcctaagtactccctgttcgagctggaaaacggccggaagagaatgctggcctctgccggcgaactgcagaagggaaacgaactggccctgccctccaaatatgtgaacttcctgtacctggccagccactatgagaagctgaagggctcccccgaggataatgagcagaaacagctgtttgtggaacagcacaagcactacctggacgagatcatcgagcagatcagcgagttctccaagagagtgatcctggccgacgctaatctggacaaagtgctgtccgcctacaacaagcaccgggataagcccatcagagagcaggccgagaatatcatccacctgtttaccctgaccaatctgggagcccctgccgccttcaagtactttgacaccaccatcgaccggaagaggtacaccagcaccaaagaggtgctggacgccaccctgatccaccagagcatcaccggcctgtacgagacacggatcgacctgtctcagctgggaggcgacgaattcgcttcgccgaagaaaaagcgcaaggtcctcgagtctagagggcccttcgaaggtaagcctatccctaaccctctcctcggtctcgattctacgcgtaccggtcatcatcaccatcaccattgagtttaaacccgctgatcagcctcgactgtgccttctagttgccagccatctgttgtttgcccctcccccgtgccttccttgaccctggaaggtgccactcccactgtcctttcctaataaaatgaggaaattgcatcgcattgtctgagtaggtgtcattctattctggggggtggggtggggcaggacagcaagggggaggattgggaagacaatagcaggcatgctggggatgcggtgggctctatggcttctgaggcggaaagaaccagctggggctctagggggtatccccacgcgccctgtagcggcgcattaagcgcggcgggtgtggtggttacgcgcagcgtgaccgctacacttgccagcgccctagcgcccgctcctttcgctttcttcccttcctttctcgccacgttcgccggctttccccgtcaagctctaaatcgggggctccctttagggttccgatttagtgctttacggcacctcgaccccaaaaaacttgattagggtgatggttcacgtagtgggccatcgccctgatagacggtttttcgccctttgacgttggagtccacgttctttaatagtggactcttgttccaaactggaacaacactcaaccctatctcggtctattcttttgatttataagggattttgccgatttcggcctattggttaaaaaatgagctgatttaacaaaaatttaacgcgaattaattctgtggaatgtgtgtcagttagggtgtggaaagtccccaggctccccagcaggcagaagtatgcaaagcatgcatctcaattagtcagcaaccaggtgtggaaagtccccaggctccccagcaggcagaagtatgcaaagcatgcatctcaattagtcagcaaccatagtcccgcccctaactccgcccatcccgcccctaactccgcccagttccgcccattctccgccccatggctgactaattttttttatttatgcagaggccgaggccgcctctgcctctgagctattccagaagtagtgaggaggcttttttggaggcctaggcttttgcaaaaagctcccgggagcttgtatatccattttcggatctgatcaagagacaggatgaggatcgtttcgcatgattgaacaagatggattgcacgcaggttctccggccgcttgggtggagaggctattcggctatgactgggcacaacagacaatcggctgctctgatgccgccgtgttccggctgtcagcgcaggggcgcccggttctttttgtcaagaccgacctgtccggtgccctgaatgaactgcaggacgaggcagcgcggctatcgtggctggccacgacgggcgttccttgcgcagctgtgctcgacgttgtcactgaagcgggaagggactggctgctattgggcgaagtgccggggcaggatctcctgtcatctcaccttgctcctgccgagaaagtatccatcatggctgatgcaatgcggcggctgcatacgcttgatccggctacctgcccattcgaccaccaagcgaaacatcgcatcgagcgagcacgtactcggatggaagccggtcttgtcgatcaggatgatctggacgaagagcatcaggggctcgcgccagccgaactgttcgccaggctcaaggcgcgcatgcccgacggcgaggatctcgtcgtgacccatggcgatgcctgcttgccgaatatcatggtggaaaatggccgcttttctggattcatcgactgtggccggctgggtgtggcggaccgctatcaggacatagcgttggctacccgtgatattgctgaagagcttggcggcgaatgggctgaccgcttcctcgtgctttacggtatcgccgctcccgattcgcagcgcatcgccttctatcgccttcttgacgagttcttctgagcgggactctggggttcgcgaaatgaccgaccaagcgacgcccaacctgccatcacgagatttcgattccaccgccgccttctatgaaaggttgggcttcggaatcgttttccgggacgccggctggatgatcctccagcgcggggatctcatgctggagttcttcgcccaccccaacttgtttattgcagcttataatggttacaaataaagcaatagcatcacaaatttcacaaataaagcatttttttcactgcattctagttgtggtttgtccaaactcatcaatgtatcttatcatgtctgtataccgtcgacctctagctagagcttggcgtaatcatggtcatagctgtttcctgtgtgaaattgttatccgctcacaattccacacaacatacgagccggaagcataaagtgtaaagcctggggtgcctaatgagtgagctaactcacattaattgcgttgcgctcactgcccgctttccagtcgggaaacctgtcgtgccagctgcattaatgaatcggccaacgcgcggggagaggcggtttgcgtattgggcgctcttccgcttcctcgctcactgactcgctgcgctcggtcgttcggctgcggcgagcggtatcagctcactcaaaggcggtaatacggttatccacagaatcaggggataacgcaggaaagaacatgtgagcaaaaggccagcaaaaggccaggaaccgtaaaaaggccgcgttgctggcgtttttccataggctccgcccccctgacgagcatcacaaaaatcgacgctcaagtcagaggtggcgaaacccgacaggactataaagataccaggcgtttccccctggaagctccctcgtgcgctctcctgttccgaccctgccgcttaccggatacctgtccgcctttctcccttcgggaagcgtggcgctttctcatagctcacgctgtaggtatctcagttcggtgtaggtcgttcgctccaagctgggctgtgtgcacgaaccccccgttcagcccgaccgctgcgccttatccggtaactatcgtcttgagtccaacccggtaagacacgacttatcgccactggcagcagccactggtaacaggattagcagagcgaggtatgtaggcggtgctacagagttcttgaagtggtggcctaactacggctacactagaagaacagtatttggtatctgcgctctgctgaagccagttaccttcggaaaaagagttggtagctcttgatccggcaaacaaaccaccgctggtagcggtggtttttttgtttgcaagcagcagattacgcgcagaaaaaaaggatctcaagaagatcctttgatcttttctacggggtctgacgctcagtggaacgaaaactcacgttaagggattttggtcatgagattatcaaaaaggatcttcacctagatccttttaaattaaaaatgaagttttaaatcaatctaaagtatatatgagtaaacttggtctgacagttaccaatgcttaatcagtgaggcacctatctcagcgatctgtctatttcgttcatccatagttgcctgactccccgtcgtgtagataactacgatacgggagggcttaccatctggccccagtgctgcaatgataccgcgagacccacgctcaccggctccagatttatcagcaataaaccagccagccggaagggccgagcgcagaagtggtcctgcaactttatccgcctccatccagtctattaattgttgccgggaagctagagtaagtagttcgccagttaatagtttgcgcaacgttgttgccattgctacaggcatcgtggtgtcacgctcgtcgtttggtatggcttcattcagctccggttcccaacgatcaaggcgagttacatgatcccccatgttgtgcaaaaaagcggttagctccttcggtcctccgatcgttgtcagaagtaagttggccgcagtgttatcactcatggttatggcagcactgcataattctcttactgtcatgccatccgtaagatgcttttctgtgactggtgagtactcaaccaagtcattctgagaatagtgtatgcggcgaccgagttgctcttgcccggcgtcaatacgggataataccgcgccacatagcagaactttaaaagtgctcatcattggaaaacgttcttcggggcgaaaactctcaaggatcttaccgctgttgagatccagttcgatgtaacccactcgtgcacccaactgatcttcagcatcttttactttcaccagcgtttctgggtgagcaaaaacaggaaggcaaaatgccgcaaaaaagggaataagggcgacacggaaatgttgaatactcatactcttcctttttcaatattattgaagcatttatcagggttattgtctcatgagcggatacatatttgaatgtatttagaaaaataaacaaataggggttccgcgcacatttccccgaaaagtgccacctgacgtc

SEQ ID NO: 20 - DNA, 10696 bp, synthetic construct
  source 1..10696: mol_type = other DNA
  misc_feature 923..967: note = NLS
  misc_feature 968..3103: note = Cas9 N-ter
  misc_feature 3158..3607: note = pMag
  misc_feature 3608..3667: note = flexible linker
  misc_feature 3668..3727: note = nMagHigh1
  misc_feature 3782..5746: note = Cas9 C-ter
  misc_feature 5753..5779: note = NLS
gacggatcgggagatctcccgatcccctatggtgcactctcagtacaatctgctctgatgccgcatagttaagccagtatctgctccctgcttgtgtgttggaggtcgctgagtagtgcgcgagcaaaatttaagctacaacaaggcaaggcttgaccgacaattgcatgaagaatctgcttagggttaggcgttttgcgctgcttcgcgatgtacgggccagatatacgcgttgacattgattattgactagttattaatagtaatcaattacggggtcattagttcatagcccatatatggagttccgcgttacataacttacggtaaatggcccgcctggctgaccgcccaacgacccccgcccattgacgtcaataatgacgtatgttcccatagtaacgccaatagggactttccattgacgtcaatgggtggagtatttacggtaaactgcccacttggcagtacatcaagtgtatcatatgccaagtacgccccctattgacgtcaatgacggtaaatggcccgcctggcattatgcccagtacatgaccttatgggactttcctacttggcagtacatctacgtattagtcatcgctattaccatggtgatgcggttttggcagtacatcaatgggcgtggatagcggtttgactcacggggatttccaagtctccaccccattgacgtcaatgggagtttgttttggcaccaaaatcaacgggactttccaaaatgtcgtaacaactccgccccattgacgcaaatgggcggtaggcgtgtacggtgggaggtctatataagcagagctctctggctaactagagaacccactgcttactggcttatcgaaattaatacgactcactatagggagacccaagctggctagttaagcttgccaccatgggtaccccaaagaagaagcggaaggtcggtatccacggagtcccagcagccgacaagaagtacagcatcggcctggacatcggcaccaactctgtgggctgggccgtgatcaccgacgagtacaaggtgcccagcaagaaattcaaggtgctgggcaacaccgaccggcacagcatcaagaagaacctgatcggagccctgctgttcgacagcggcgaaacagccgaggccacccggctgaagagaaccgccagaagaagatacaccagacggaagaaccggatctgctatctgcaagagatcttcagcaacgagatggccaaggtggacgacagcttcttccacagactggaagagtccttcctggtggaagaggataagaagcacgagcggcaccccatcttcggcaacatcgtggacgaggtggcctaccacgagaagtaccccaccatctaccacctgagaaagaaactggtggacagcaccgacaaggccgacctgcggctgatctatctggccctggcccacatgatcaagttccggggccacttcctgatcgagggcgacctgaaccccgacaacagcgacgtggacaagctgttcatccagctggtgcagacctacaaccagctgttcgaggaaaaccccatcaacgccagcggcgtggacgccaaggccatcctgtctgccagactgagcaagagcagacggctggaaaatctgatcgcccagctgcccggcgagaagaagaatggcctgttcggaaacctgattgccctgagcctgggcctgacccccaacttcaagagcaacttcgacctggccgaggatgccaaactgcagctgagcaaggacacctacgacgacgacctggacaacctgctggcccagatcggcgaccagtacgccgacctgtttctggccgccaagaacctgtccgacgccatcctgctgagcgacatcctgagagtgaacaccgagatcaccaaggcccccctgagcgcctctatgatcaagagatacgacgagcaccaccaggacctgaccctgctgaaagctctcgtgcggcagcagctgcctgagaagtacaaagagattttcttcgaccagagcaagaacggctacgccggctacattgacggcggagccagccaggaagagttctacaagttcatcaagcccatcctggaaaagatggacggcaccgaggaactgctcgtgaagctgaacagagaggacctgctgcggaagcagcggaccttcgacaacggcagcatcccccaccagatccacctgggagagctgcacgccattctgcggcggcaggaagatttttacccattcctgaaggacaaccgggaaaagatcgagaagatcctgaccttccgcatcccctactacgtgggccctctggccaggggaaacagcagattcgcctggatgaccagaaagagcgaggaaaccatcaccccctggaacttcgaggaagtggtggacaagggcgcttccgcccagagcttcatcgagcggatgaccaacttcgataagaacctgcccaacgagaaggtgctgcccaagcacagcctgctgtacgagtacttcaccgtgtataacgagctgaccaaagtgaaatacgtgaccgagggaatgagaaagcccgccttcctgagcggcgagcagaaaaaggccatcgtggacctgctgttcaagaccaaccggaaagtgaccgtgaagcagctgaaagaggactacttcaagaaaatcgagtgcttcgactccgtggaaatctccggcgtggaagatcggttcaacgcctccctgggcacataccacgatctgctgaaaattatcaaggacaaggacttcctggacaatgaggaaaacgaggacattctggaagatatcgtgctgaccctgacactgtttgaggacagagagatgatcgaggaacggctgaaaacctatgcccacctgttcgacgacaaagtgatgaagcagctgaagcggcggagatacaccggctggggcaggctgagccggaagctgatcaacggcatccgggacaagcagtccggcaagacaatcctggatttcctgaagtccgacggcttcgccaacagaaacttcatgcagctgatccacgacgacagcctgacctttaaagaggacatccagaaagcccaggtggaattcgggggttctggggggagcggcgggggatctggaagtggcagcggaggccatactctttatgcccccggtggatatgacattatgggatatctgaggcagatcaggaaccggccaaacccgcaggtggaactgggccccgtggatacatcctgcgccttgattctttgtgacctgaaacagaaagacaccccgatagtttacgcgagtgaagccttcctctacatgacaggttacagcaacgcagaggtgctgggccggaattgccggtttctgcaaagccctgacggcatggtgaagcccaagagcacccggaagtacgtggatagtaacacaatcaatactatgcgcaaggcaatcgacaggaatgccgaggtgcaggttgaagtagtcaattttaaaaagaatggacagcgatttgttaatttcctgactatgatacctgttagggacgaaacaggcgagtatcgatactctatgggattccagtgcgaaacagaaggatctggcggaggaagcggtggcggaagcggcggaggttcaggcggaggatctggatctcacaccctttatgcccctggtggttatgacattatggggtatctcgaccaaataggcaacaggcccaatccacaggttgaattggggcccgttgacacttcttgcgcccttatactctgtgacttgaaacaaaaggatacacccatagtgtacgccagcgaggcatttctctatatgacaggctactccaacgcagaggtcctgggtaggaactgtcggtttcttcaaagtccagatggtatggtcaaacccaagtccacaaggaaatacgtagactccaatacaatcaacacaatcaggaaggccatagatcgaaacgcagaggttcaggtggaagtggttaactttaagaaaaatggacaacgattcgttaacttcttgactatcatacctgtgcgggacgagactggggagtataggtattcaatggggttccagtgtgaaaccgaagggggttctggggggagcggcgggggatctggaagtggcagcggaggcggtacctccggccagggcgatagcctgcacgagcacattgccaatctggccggcagccccgccattaagaagggcatcctgcagacagtgaaggtggtggacgagctcgtgaaagtgatgggccggcacaagcccgagaacatcgtgatcgaaatggccagagagaaccagaccacccagaagggacagaagaacagccgcgagagaatgaagcggatcgaagagggcatcaaagagctgggcagccagatcctgaaagaacaccccgtggaaaacacccagctgcagaacgagaagctgtacctgtactacctgcagaatgggcgggatatgtacgtggaccaggaactggacatcaaccggctgtccgactacgatgtggaccatatcgtgcctcagagctttctgaaggacgactccatcgacaacaaggtgctgaccagaagcgacaagaaccggggcaagagcgacaacgtgccctccgaagaggtcgtgaagaagatgaagaactactggcggcagctgctgaacgccaagctgattacccagagaaagttcgacaatctgaccaaggccgagagaggcggcctgagcgaactggataaggccggcttcatcaagagacagctggtggaaacccggcagatcacaaagcacgtggcacagatcctggactcccggatgaacactaagtacgacgagaatgacaagctgatccgggaagtgaaagtgatcaccctgaagtccaagctggtgtccgatttccggaaggatttccagttttacaaagtgcgcgagatcaacaactaccaccacgcccacgacgcctacctgaacgccgtcgtgggaaccgccctgatcaaaaagtaccctaagctggaaagcgagttcgtgtacggcgactacaaggtgtacgacgtgcggaagatgatcgccaagagcgagcaggaaatcggcaaggctaccgccaagtacttcttctacagcaacatcatgaactttttcaagaccgagattaccctggccaacggcgagatccggaagcggcctctgatcgagacaaacggcgaaaccggggagatcgtgtgggataagggccgggattttgccaccgtgcggaaagtgctgagcatgccccaagtgaatatcgtgaaaaagaccgaggtgcagacaggcggcttcagcaaagagtctatcctgcccaagaggaacagcgataagctgatcgccagaaagaaggactgggaccctaagaagtacggcggcttcgacagccccaccgtggcctattctgtgctggtggtggccaaagtggaaaagggcaagtccaagaaactgaagagtgtgaaagagctgctggggatcaccatcatggaaagaagcagcttcgagaagaatcccatcgactttctggaagccaagggctacaaagaagtgaaaaaggacctgatcatcaagctgcctaagtactccctgttcgagctggaaaacggccggaagagaatgctggcctctgccggcgaactgcagaagggaaacgaactggccctgccctccaaatatgtgaacttcctgtacctggccagccactatgagaagctgaagggctcccccgaggataatgagcagaaacagctgtttgtggaacagcacaagcactacctggacgagatcatcgagcagatcagcgagttctccaagagagtgatcctggccgacgctaatctggacaaagtgctgtccgcctacaacaagcaccgggataagcccatcagagagcaggccgagaatatcatccacctgtttaccctgaccaatctgggagcccctgccgccttcaagtactttgacaccaccatcgaccggaagaggtacaccagcaccaaagaggtgctggacgccaccctgatccaccagagcatcaccggcctgtacgagacacggatcgacctgtctcagctgggaggcgacgaattcgcttcgccgaagaaaaagcgcaaggtcctcgagtctagagggcccttcgaaggtaagcctatccctaaccctctcctcggtctcgattctacgcgtaccggtcatcatcaccatcaccattgagtttaaacccgctgatcagcctcgactgtgccttctagttgccagccatctgttgtttgcccctcccccgtgccttccttgaccctggaaggtgccactcccactgtcctttcctaataaaatgaggaaattgcatcgcattgtctgagtaggtgtcattctattctggggggtggggtggggcaggacagcaagggggaggattgggaagacaatagcaggcatgctggggatgcggtgggctctatggcttctgaggcggaaagaaccagctggggctctagggggtatccccacgcgccctgtagcggcgcattaagcgcggcgggtgtggtggttacgcgcagcgtgaccgctacacttgccagcgccctagcgcccgctcctttcgctttcttcccttcctttctcgccacgttcgccggctttccccgtcaagctctaaatcgggggctccctttagggttccgatttagtgctttacggcacctcgaccccaaaaaacttgattagggtgatggttcacgtagtgggccatcgccctgatagacggtttttcgccctttgacgttggagtccacgttctttaatagtggactcttgttccaaactggaacaacactcaaccctatctcggtctattcttttgatttataagggattttgccgatttcggcctattggttaaaaaatgagctgatttaacaaaaatttaacgcgaattaattctgtggaatgtgtgtcagttagggtgtggaaagtccccaggctccccagcaggcagaagtatgcaaagcatgcatctcaattagtcagcaaccaggtgtggaaagtccccaggctccccagcaggcagaagtatgcaaagcatgcatctcaattagtcagcaaccatagtcccgcccctaactccgcccatcccgcccctaactccgcccagttccgcccattctccgccccatggctgactaattttttttatttatgcagaggccgaggccgcctctgcctctgagctattccagaagtagtgaggaggcttttttggaggcctaggcttttgcaaaaagctcccgggagcttgtatatccattttcggatctgatcaagagacaggatgaggatcgtttcgcatgattgaacaagatggattgcacgcaggttctccggccgcttgggtggagaggctattcggctatgactgggcacaacagacaatcggctgctctgatgccgccgtgttccggctgtcagcgcaggggcgcccggttctttttgtcaagaccgacctgtccggtgccctgaatgaactgcaggacgaggcagcgcggctatcgtggctggccacgacgggcgttccttgcgcagctgtgctcgacgttgtcactgaagcgggaagggactggctgctattgggcgaagtgccggggcaggatctcctgtcatctcaccttgctcctgccgagaaagtatccatcatggctgatgcaatgcggcggctgcatacgcttgatccggctacctgcccattcgaccaccaagcgaaacatcgcatcgagcgagcacgtactcggatggaagccggtcttgtcgatcaggatgatctggacgaagagcatcaggggctcgcgccagccgaactgttcgccaggctcaaggcgcgcatgcccgacggcgaggatctcgtcgtgacccatggcgatgcctgcttgccgaatatcatggtggaaaatggccgcttttctggattcatcgactgtggccggctgggtgtggcggaccgctatcaggacatagcgttggctacccgtgatattgctgaagagcttggcggcgaatgggctgaccgcttcctcgtgctttacggtatcgccgctcccgattcgcagcgcatcgccttctatcgccttcttgacgagttcttctgagcgggactctggggttcgcgaaatgaccgaccaagcgacgcccaacctgccatcacgagatttcgattccaccgccgccttctatgaaaggttgggcttcggaatcgttttccgggacgccggctggatgatcctccagcgcggggatctcatgctggagttcttcgcccaccccaacttgtttattgcagcttataatggttacaaataaagcaatagcatcacaaatttcacaaataaagcatttttttcactgcattctagttgtggtttgtccaaactcatcaatgtatcttatcatgtctgtataccgtcgacctctagctagagcttggcgtaatcatggtcatagctgtttcctgtgtgaaattgttatccgctcacaattccacacaacatacgagccggaagcataaagtgtaaagcctggggtgcctaatgagtgagctaactcacattaattgcgttgcgctcactgcccgctttccagtcgggaaacctgtcgtgccagctgcattaatgaatcggccaacgcgcggggagaggcggtttgcgtattgggcgctcttccgcttcctcgctcactgactcgctgcgctcggtcgttcggctgcggcgagcggtatcagctcactcaaaggcggtaatacggttatccacagaatcaggggataacgcaggaaagaacatgtgagcaaaaggccagcaaaaggccaggaaccgtaaaaaggccgcgttgctggcgtttttccataggctccgcccccctgacgagcatcacaaaaatcgacgctcaagtcagaggtggcgaaacccgacaggactataaagataccaggcgtttccccctggaagctccctcgtgcgctctcctgttccgaccctgccgcttaccggatacctgtccgcctttctcccttcgggaagcgtggcgctttctcatagctcacgctgtaggtatctcagttcggtgtaggtcgttcgctccaagctgggctgtgtgcacgaaccccccgttcagcccgaccgctgcgccttatccggtaactatcgtcttgagtccaacccggtaagacacgacttatcgccactggcagcagccactggtaacaggattagcagagcgaggtatgtaggcggtgctacagagttcttgaagtggtggcctaactacggctacactagaagaacagtatttggtatctgcgctctgctgaagccagttaccttcggaaaaagagttggtagctcttgatccggcaaacaaaccaccgctggtagcggtggtttttttgtttgcaagcagcagattacgcgcagaaaaaaaggatctcaagaagatcctttgatcttttctacggggtctgacgctcagtggaacgaaaactcacgttaagggattttggtcatgagattatcaaaaaggatcttcacctagatccttttaaattaaaaatgaagttttaaatcaatctaaagtatatatgagtaaacttggtctgacagttaccaatgcttaatcagtgaggcacctatctcagcgatctgtctatttcgttcatccatagttgcctgactccccgtcgtgtagataactacgatacgggagggcttaccatctggccccagtgctgcaatgataccgcgagacccacgctcaccggctccagatttatcagcaataaaccagccagccggaagggccgagcgcagaagtggtcctgcaactttatccgcctccatccagtctattaattgttgccgggaagctagagtaagtagttcgccagttaatagtttgcgcaacgttgttgccattgctacaggcatcgtggtgtcacgctcgtcgtttggtatggcttcattcagctccggttcccaacgatcaaggcgagttacatgatcccccatgttgtgcaaaaaagcggttagctccttcggtcctccgatcgttgtcagaagtaagttggccgcagtgttatcactcatggttatggcagcactgcataattctcttactgtcatgccatccgtaagatgcttttctgtgactggtgagtactcaaccaagtcattctgagaatagtgtatgcggcgaccgagttgctcttgcccggcgtcaatacgggataataccgcgccacatagcagaactttaaaagtgctcatcattggaaaacgttcttcggggcgaaaactctcaaggatcttaccgctgttgagatccagttcgatgtaacccactcgtgcacccaactgatcttcagcatcttttactttcaccagcgtttctgggtgagcaaaaacaggaaggcaaaatgccgcaaaaaagggaataagggcgacacggaaatgttgaatactcatactcttcctttttcaatattattgaagcatttatcagggttattgtctcatgagcggatacatatttgaatgtatttagaaaaataaacaaataggggttccgcgcacatttccccgaaaagtgccacctgacgtc

SEQ ID NO: 21 - DNA, 10696 bp, synthetic construct
  source 1..10696: mol_type = other DNA
  misc_feature 923..967: note = NLS
  misc_feature 968..3103: note = Cas9 N-ter
  misc_feature 3158..3607: note = pMag
  misc_feature 3608..3667: note = rigid linker
  misc_feature 3668..3727: note = nMagHigh1
  misc_feature 3782..5746: note = Cas9 C-ter
  misc_feature 5753..5779: note = NLS
gacggatcgggagatctcccgatcccctatggtgcactctcagtacaatctgctctgatgccgcatagttaagccagtatctgctccctgcttgtgtgttggaggtcgctgagtagtgcgcgagcaaaatttaagctacaacaaggcaaggcttgaccgacaattgcatgaagaatctgcttagggttaggcgttttgcgctgcttcgcgatgtacgggccagatatacgcgttgacattgattattgactagttattaatagtaatcaattacggggtcattagttcatagcccatatatggagttccgcgttacataacttacggtaaatggcccgcctggctgaccgcccaacgacccccgcccattgacgtcaataatgacgtatgttcccatagtaacgccaatagggactttccattgacgtcaatgggtggagtatttacggtaaactgcccacttggcagtacatcaagtgtatcatatgccaagtacgccccctattgacgtcaatgacggtaaatggcccgcctggcattatgcccagtacatgaccttatgggactttcctacttggcagtacatctacgtattagtcatcgctattaccatggtgatgcggttttggcagtacatcaatgggcgtggatagcggtttgactcacggggatttccaagtctccaccccattgacgtcaatgggagtttgttttggcaccaaaatcaacgggactttccaaaatgtcgtaacaactccgccccattgacgcaaatgggcggtaggcgtgtacggtgggaggtctatataagcagagctctctggctaactagagaacccactgcttactggcttatcgaaattaatacgactcactatagggagacccaagctggctagttaagcttgccaccatgggtaccccaaagaagaagcggaaggtcggtatccacggagtcccagcagccgacaagaagtacagcatcggcctggacatcggcaccaactctgtgggctgggccgtgatcaccgacgagtacaaggtgcccagcaagaaattcaaggtgctgggcaacaccgaccggcacagcatcaagaagaacctgatcggagccctgctgttcgacagcggcgaaacagccgaggccacccggctgaagagaaccgccagaagaagatacaccagacggaagaaccggatctgctatctgcaagagatcttcagcaacgagatggccaaggtggacgacagcttcttccacagactggaagagtccttcctggtggaagaggataagaagcacgagcggcaccccatcttcggcaacatcgtggacgaggtggcctaccacgagaagtaccccaccatctaccacctgagaaagaaactggtggacagcaccgacaaggccgacctgcggctgatctatctggccctggcccacatgatcaagttccggggccacttcctgatcgagggcgacctgaaccccgacaacagcgacgtggacaagctgttcatccagctggtgcagacctacaaccagctgttcgaggaaaaccccatcaacgccagcggcgtggacgccaaggccatcctgtctgccagactgagcaagagcagacggctggaaaatctgatcgcccagctgcccggcgagaagaagaatggcctgttcggaaacctgattgccctgagcctgggcctgacccccaacttcaagagcaacttcgacctggccgaggatgccaaactgcagctgagcaaggacacctacgacgacgacctggacaacctgctggcccagatcggcgaccagtacgccgacctgtttctggccgccaagaacctgtccgacgccatcctgctgagcgacatcctgagagtgaacaccgagatcaccaaggcccccctgagcgcctctatgatcaagagatacgacgagcaccaccaggacctgaccctgctgaaagctctcgtgcggcagcagctgcctgagaagtacaaagagattttcttcgaccagagcaagaacggctacgccggctacattgacggcggagccagccaggaagagttctacaagttcatcaagcccatcctggaaaagatggacggcaccgaggaactgctcgtgaagctgaacagagaggacctgctgcggaagcagcggaccttcgacaacggcagcatcccccaccagatccacctgggagagctgcacgccattctgcggcggcaggaagatttttacccattcctgaaggacaaccgggaaaagatcgagaagatcctgaccttccgcatcccctactacgtgggccctctggccaggggaaacagcagattcgcctggatgaccagaaagagcgaggaaaccatcaccccctggaacttcgaggaagtggtggacaagggcgcttccgcccagagcttcatcgagcggatgaccaacttcgataagaacctgcccaacgagaaggtgctgcccaagcacagcctgctgtacgagtacttcaccgtgtataacgagctgaccaaagtgaaatacgtgaccgagggaatgagaaagcccgccttcctgagcggcgagcagaaaaaggccatcgtggacctgctgttcaagaccaaccggaaagtgaccgtgaagcagctgaaagaggactacttcaagaaaatcgagtgcttcgactccgtggaaatctccggcgtggaagatcggttcaacgcctccctgggcacataccacgatctgctgaaaattatcaaggacaaggacttcctggacaatgaggaaaacgaggacattctggaagatatcgtgctgaccctgacactgtttgaggacagagagatgatcgaggaacggctgaaaacctatgcccacctgttcgacgacaaagtgatgaagcagctgaagcggcggagatacaccggctggggcaggctgagccggaagctgatcaacggcatccgggacaagcagtccggcaagacaatcctggatttcctgaagtccgacggcttcgccaacagaaacttcatgcagctgatccacgacgacagcctgacctttaaagaggacatccagaaagcccaggtggaattcgggggttctggggggagcggcgggggatctggaagtggcagcggaggccatactctttatgcccccggtggatatgacattatgggatatctgaggcagatcaggaaccggccaaacccgcaggtggaactgggccccgtggatacatcctgcgccttgattctttgtgacctgaaacagaaagacaccccgatagtttacgcgagtgaagccttcctctacatgacaggttacagcaacgcagaggtgctgggccggaattgccggtttctgcaaagccctgacggcatggtgaagcccaagagcacccggaagtacgtggatagtaacacaatcaatactatgcgcaaggcaatcgacaggaatgccgaggtgcaggttgaagtagtcaattttaaaaagaatggacagcgatttgttaatttcctgactatgatacctgttagggacgaaacaggcgagtatcgatactctatgggattccagtgcgaaacagaaggatctgctgaagccgccgctaaagctggatctgctgaagctgctgccaaggcaggatctcacaccctttatgcccctggtggttatgacattatggggtatctcgaccaaataggcaacaggcccaatccacaggttgaattggggcccgttgacacttcttgcgcccttatactctgtgacttgaaacaaaaggatacacccatagtgtacgccagcgaggcatttctctatatgacaggctactccaacgcagaggtcctgggtaggaactgtcggtttcttcaaagtccagatggtatggtcaaacccaagtccacaaggaaatacgtagactccaatacaatcaacacaatcaggaaggccatagatcgaaacgcagaggttcaggtggaagtggttaactttaagaaaaatggacaacgattcgttaacttcttgactatcatacctgtgcgggacgagactggggagtataggtattcaatggggttccagtgtgaaaccgaagggggttctggggggagcggcgggggatctggaagtggcagcggaggcggtacctccggccagggcgatagcctgcacgagcacattgccaatctggccggcagccccgccattaagaagggcatcctgcagacagtgaaggtggtggacgagctcgtgaaagtgatgggccggcacaagcccgagaacatcgtgatcgaaatggccagagagaaccagaccacccagaagggacagaagaacagccgcgagagaatgaagcggatcgaagagggcatcaaagagctgggcagccagatcctgaaagaacaccccgtggaaaacacccagctgcagaacgagaagctgtacctgtactacctgcagaatgggcgggatatgtacgtggaccaggaactggacatcaaccggctgtccgactacgatgtggaccatatcgtgcctcagagctttctgaaggacgactccatcgacaacaaggtgctgaccagaagcgacaagaaccggggcaagagcgacaacgtgccctccgaagaggtcgtgaagaagatgaagaactactggcggcagctgctgaacgccaagctgattacccagagaaagttcgacaatctgaccaaggccgagagaggcggcctgagcgaactggataaggccggcttcatcaagagacagctggtggaaacccggcagatcacaaagcacgtggcacagatcctggactcccggatgaacactaagtacgacgagaatgacaagctgatccgggaagtgaaagtgatcaccctgaagtccaagctggtgtccgatttccggaaggatttccagttttacaaagtgcgcgagatcaacaactaccaccacgcccacgacgcctacctgaacgccgtcgtgggaaccgccctgatcaaaaagtaccctaagctggaaagcgagttcgtgtacggcgactacaaggtgtacgacgtgcggaagatgatcgccaagagcgagcaggaaatcggcaaggctaccgccaagtacttcttctacagcaacatcatgaactttttcaagaccgagattaccctggccaacggcgagatccggaagcggcctctgatcgagacaaacggcgaaaccggggagatcgtgtgggataagggccgggattttgccaccgtgcggaaagtgctgagcatgccccaagtgaatatcgtgaaaaagaccgaggtgcagacaggcggcttcagcaaagagtctatcctgcccaagaggaacagcgataagctgatcgccagaaagaaggactgggaccctaagaagtacggcggcttcgacagccccaccgtggcctattctgtgctggtggtggccaaagtggaaaagggcaagtccaagaaactgaagagtgtgaaagagctgctggggatcaccatcatggaaagaagcagcttcgagaagaatcccatcgactttctggaagccaagggctacaaagaagtgaaaaaggacctgatcatcaagctgcctaagtactccctgttcgagctggaaaacggccggaagagaatgctggcctctgccggcgaactgcagaagggaaacgaactggccctgccctccaaatatgtgaacttcctgtacctggccagccactatgagaagctgaagggctcccccgaggataatgagcagaaacagctgtttgtggaacagcacaagcactacctggacgagatcatcgagcagatcagcgagttctccaagagagtgatcctggccgacgctaatctggacaaagtgctgtccgcctacaacaagcaccgggataagcccatcagagagcaggccgagaatatcatccacctgtttaccctgaccaatctgggagcccctgccgccttcaagtactttgacaccaccatcgaccggaagaggtacaccagcaccaaagaggtgctggacgccaccctgatccaccagagcatcaccggcctgtacgagacacggatcgacctgtctcagctgggaggcgacgaattcgcttcgccgaagaaaaagcgcaaggtcctcgagtctagagggcccttcgaaggtaagcctatccctaaccctctcctcggtctcgattctacgcgtaccggtcatcatcaccatcaccattgagtttaaacccgctgatcagcctcgactgtgccttctagttgccagccatctgttgtttgcccctcccccgtgccttccttgaccctggaaggtgccactcccactgtcctttcctaataaaatgaggaaattgcatcgcattgtctgagtaggtgtcattctattctggggggtggggtggggcaggacagcaagggggaggattgggaagacaatagcaggcatgctggggatgcggtgggctctatggcttctgaggcggaaagaaccagctggggctctagggggtatccccacgcgccctgtagcggcgcattaagcgcggcgggtgtggtggttacgcgcagcgtgaccgctacacttgccagcgccctagcgcccgctcctttcgctttcttcccttcctttctcgccacgttcgccggctttccccgtcaagctctaaatcgggggctccctttagggttccgatttagtgctttacggcacctcgaccccaaaaaacttgattagggtgatggttcacgtagtgggccatcgccctgatagacggtttttcgccctttgacgttggagtccacgttctttaatagtggactcttgttccaaactggaacaacactcaaccctatctcggtctattcttttgatttataagggattttgccgatttcggcctattggttaaaaaatgagctgatttaacaaaaatttaacgcgaattaattctgtggaatgtgtgtcagttagggtgtggaaagtccccaggctccccagcaggcagaagtatgcaaagcatgcatctcaattagtcagcaaccaggtgtggaaagtccccaggctccccagcaggcagaagtatgcaaagcatgcatctcaattagtcagcaaccatagtcccgcccctaactccgcccatcccgcccctaactccgcccagttccgcccattctccgccccatggctgactaattttttttatttatgcagaggccgaggccgcctctgcctctgagctattccagaagtagtgaggaggcttttttggaggcctaggcttttgcaaaaagctcccgggagcttgtatatccattttcggatctgatcaagagacaggatgaggatcgtttcgcatgattgaacaagatggattgcacgcaggttctccggccgcttgggtggagaggctattcggctatgactgggcacaacagacaatcggctgctctgatgccgccgtgttccggctgtcagcgcaggggcgcccggttctttttgtcaagaccgacctgtccggtgccctgaatgaactgcaggacgaggcagcgcggctatcgtggctggccacgacgggcgttccttgcgcagctgtgctcgacgttgtcactgaagcgggaagggactggctgctattgggcgaagtgccggggcaggatctcctgtcatctcaccttgctcctgccgagaaagtatccatcatggctgatgcaatgcggcggctgcatacgcttgatccggctacctgcccattcgaccaccaagcgaaacatcgcatcgagcgagcacgtactcggatggaagccggtcttgtcgatcaggatgatctggacgaagagcatcaggggctcgcgccagccgaactgttcgccaggctcaaggcgcgcatgcccgacggcgaggatctcgtcgtgacccatggcgatgcctgcttgccgaatatcatggtggaaaatggccgcttttctggattcatcgactgtggccggctgggtgtggcggaccgctatcaggacatagcgttggctacccgtgatattgctgaagagcttggcggcgaatgggctgaccgcttcctcgtgctttacggtatcgccgctcccgattcgcagcgcatcgccttctatcgccttcttgacgagttcttctgagcgggactctggggttcgcgaaatgaccgaccaagcgacgcccaacctgccatcacgagatttcgattccaccgccgccttctatgaaaggttgggcttcggaatcgttttccgggacgccggctggatgatcctccagcgcggggatctcatgctggagttcttcgcccaccccaacttgtttattgcagcttataatggttacaaataaagcaatagcatcacaaatttcacaaataaagcatttttttcactgcattctagttgtggtttgtccaaactcatcaatgtatcttatcatgtctgtataccgtcgacctctagctagagcttggcgtaatcatggtcatagctgtttcctgtgtgaaattgttatccgctcacaattccacacaacatacgagccggaagcataaagtgtaaagcctggggtgcctaatgagtgagctaactcacattaattgcgttgcgctcactgcccgctttccagtcgggaaacctgtcgtgccagctgcattaatgaatcggccaacgcgcggggagaggcggtttgcgtattgggcgctcttccgcttcctcgctcactgactcgctgcgctcggtcgttcggctgcggcgagcggtatcagctcactcaaaggcggtaatacggttatccacagaatcaggggataacgcaggaaagaacatgtgagcaaaaggccagcaaaaggccaggaaccgtaaaaaggccgcgttgctggcgtttttccataggctccgcccccctgacgagcatcacaaaaatcgacgctcaagtcagaggtggcgaaacccgacaggactataaagataccaggcgtttccccctggaagctccctcgtgcgctctcctgttccgaccctgccgcttaccggatacctgtccgcctttctcccttcgggaagcgtggcgctttctcatagctcacgctgtaggtatctcagttcggtgtaggtcgttcgctccaagctgggctgtgtgcacgaaccccccgttcagcccgaccgctgcgccttatccggtaactatcgtcttgagtccaacccggtaagacacgacttatcgccactggcagcagccactggtaacaggattagcagagcgaggtatgtaggcggtgctacagagttcttgaagtggtggcctaactacggctacactagaagaacagtatttggtatctgcgctctgctgaagccagttaccttcggaaaaagagttggtagctcttgatccggcaaacaaaccaccgctggtagcggtggtttttttgtttgcaagcagcagattacgcgcagaaaaaaaggatctcaagaagatcctttgatcttttctacggggtctgacgctcagtggaacgaaaactcacgttaagggattttggtcatgagattatcaaaaaggatcttcacctagatccttttaaattaaaaatgaagttttaaatcaatctaaagtatatatgagtaaacttggtctgacagttaccaatgcttaatcagtgaggcacctatctcagcgatctgtctatttcgttcatccatagttgcctgactccccgtcgtgtagataactacgatacgggagggcttaccatctggccccagtgctgcaatgataccgcgagacccacgctcaccggctccagatttatcagcaataaaccagccagccggaagggccgagcgcagaagtggtcctgcaactttatccgcctccatccagtctattaattgttgccgggaagctagagtaagtagttcgccagttaatagtttgcgcaacgttgttgccattgctacaggcatcgtggtgtcacgctcgtcgtttggtatggcttcattcagctccggttcccaacgatcaaggcgagttacatgatcccccatgttgtgcaaaaaagcggttagctccttcggtcctccgatcgttgtcagaagtaagttggccgcagtgttatcactcatggttatggcagcactgcataattctcttactgtcatgccatccgtaagatgcttttctgtgactggtgagtactcaaccaagtcattctgagaatagtgtatgcggcgaccgagttgctcttgcccggcgtcaatacgggataataccgcgccacatagcagaactttaaaagtgctcatcattggaaaacgttcttcggggcgaaaactctcaaggatcttaccgctgttgagatccagttcgatgtaacccactcgtgcacccaactgatcttcagcatcttttactttcaccagcgtttctgggtgagcaaaaacaggaaggcaaaatgccgcaaaaaagggaataagggcgacacggaaatgttgaatactcatactcttcctttttcaatattattgaagcatttatcagggttattgtctcatgagcggatacatatttgaatgtatttagaaaaataaacaaataggggttccgcgcacatttccccgaaaagtgccacctgacgtc

SEQ ID NO: 22 - DNA, 10639 bp, synthetic construct
  source 1..10639: mol_type = other DNA
  misc_feature 932..976: note = NLS
  misc_feature 977..3120: note = Cas9 N-ter
  misc_feature 3175..3624: note = pMag
  misc_feature 3625..4068: note = nMagHigh1
  misc_feature 4123..6087: note = Cas9 C-ter
  misc_feature 6094..6120: note = NLS
gacggatcgggagatctcccgatcccctatggtgcactctcagtacaatctgctctgatgccgcatagttaagccagtatctgctccctgcttgtgtgttggaggtcgctgagtagtgcgcgagcaaaatttaagctacaacaaggcaaggcttgaccgacaattgcatgaagaatctgcttagggttaggcgttttgcgctgcttcgcgatgtacgggccagatatacgcgttgacattgattattgactagttattaatagtaatcaattacggggtcattagttcatagcccatatatggagttccgcgttacataacttacggtaaatggcccgcctggctgaccgcccaacgacccccgcccattgacgtcaataatgacgtatgttcccatagtaacgccaatagggactttccattgacgtcaatgggtggagtatttacggtaaactgcccacttggcagtacatcaagtgtatcatatgccaagtacgccccctattgacgtcaatgacggtaaatggcccgcctggcattatgcccagtacatgaccttatgggactttcctacttggcagtacatctacgtattagtcatcgctattaccatggtgatgcggttttggcagtacatcaatgggcgtggatagcggtttgactcacggggatttccaagtctccaccccattgacgtcaatgggagtttgttttggcaccaaaatcaacgggactttccaaaatgtcgtaacaactccgccccattgacgcaaatgggcggtaggcgtgtacggtgggaggtctatataagcagagctctctggctaactagagaacccactgcttactggcttatcgaaattaatacgactcactatagggagacccaagctggctagcgtttaaacttaagcttgccaccatgggtaccccaaagaagaagcggaaggtcggtatccacggagtcccagcagccgacaagaagtacagcatcggcctggacatcggcaccaactctgtgggctgggccgtgatcaccgacgagtacaaggtgcccagcaagaaattcaaggtgctgggcaacaccgaccggcacagcatcaagaagaacctgatcggagccctgctgttcgacagcggcgaaacagccgaggccacccggctgaagagaaccgccagaagaagatacaccagacggaagaaccggatctgctatctgcaagagatcttcagcaacgagatggccaaggtggacgacagcttcttccacagactggaagagtccttcctggtggaagaggataagaagcacgagcggcaccccatcttcggcaacatcgtggacgaggtggcctaccacgagaagtaccccaccatctaccacctgagaaagaaactggtggacagcaccgacaaggccgacctgcggctgatctatctggccctggcccacatgatcaagttccggggccacttcctgatcgagggcgacctgaaccccgacaacagcgacgtggacaagctgttcatccagctggtgcagacctacaaccagctgttcgaggaaaaccccatcaacgccagcggcgtggacgccaaggccatcctgtctgccagactgagcaagagcagacggctggaaaatctgatcgcccagctgcccggcgagaagaagaatggcctgttcggaaacctgattgccctgagcctgggcctgacccccaacttcaagagcaacttcgacctggccgaggatgccaaactgcagctgagcaaggacacctacgacgacgacctggacaacctgctggcccagatcggcgaccagtacgccgacctgtttctggccgccaagaacctgtccgacgccatcctgctgagcgacatcctgagagtgaacaccgagatcaccaaggcccccctgagcgcctctatgatcaagagatacgacgagcaccaccaggacctgaccctgctgaaagctctcgtgcggcagcagctgcctgagaagtacaaagagattttcttcgaccagagcaagaacggctacgccggctacattgacggcggagccagccaggaagagttctacaagttcatcaagcccatcctggaaaagatggacggcaccgaggaactgctcgtgaagctgaacagagaggacctgctgcggaagcagcggaccttcgacaacggcagcatcccccaccagatccacctgggagagctgcacgccattctgcggcggcaggaagatttttacccattcctgaaggacaaccgggaaaagatcgagaagatcctgaccttccgcatcccctactacgtgggccctctggccaggggaaacagcagattcgcctggatgaccagaaagagcgaggaaaccatcaccccctggaacttcgaggaagtggtggacaagggcgcttccgcccagagcttcatcgagcggatgaccaacttcgataagaacctgcccaacgagaaggtgctgcccaagcacagcctgctgtacgagtacttcaccgtgtataacgagctgaccaaagtgaaatacgtgaccgagggaatgagaaagcccgccttcctgagcggcgagcagaaaaaggccatcgtggacctgctgttcaagaccaaccggaaagtgaccgtgaagcagctgaaagaggactacttcaagaaaatcgagtgcttcgactccgtggaaatctccggcgtggaagatcggttcaacgcctccctgggcacataccacgatctgctgaaaattatcaaggacaaggacttcctggacaatgaggaaaacgaggacattctggaagatatcgtgctgaccctgacactgtttgaggacagagagatgatcgaggaacggctgaaaacctatgcccacctgttcgacgacaaagtgatgaagcagctgaagcggcggagatacaccggctggggcaggctgagccggaagctgatcaacggcatccgggacaagcagtccggcaagacaatcctggatttcctgaagtccgacggcttcgccaacagaaacttcatgcagctgatccacgacgacagcctgacctttaaagaggacatccagaaagcccaggtggaattcgggggttctggggggagcggcgggggatctggaagtggcagcggaggccatactctttatgcccccggtggatatgacattatgggatatctgaggcagatcaggaaccggccaaacccgcaggtggaactgggccccgtggatacatcctgcgccttgattctttgtgacctgaaacagaaagacaccccgatagtttacgcgagtgaagccttcctctacatgacaggttacagcaacgcagaggtgctgggccggaattgccggtttctgcaaagccctgacggcatggtgaagcccaagagcacccggaagtacgtggatagtaacacaatcaatactatgcgcaaggcaatcgacaggaatgccgaggtgcaggttgaagtagtcaattttaaaaagaatggacagcgatttgttaatttcctgactatgatacctgttagggacgaaacaggcgagtatcgatactctatgggattccagtgcgaaacagaactttatgcccctggtggttatgacattatggggtatctcgaccaaataggcaacaggcccaatccacaggttgaattggggcccgttgacacttcttgcgcccttatactctgtgacttgaaacaaaaggatacacccatagtgtacgccagcgaggcatttctctatatgacaggctactccaacgcagaggtcctgggtaggaactgtcggtttcttcaaagtccagatggtatggtcaaacccaagtccacaaggaaatacgtagactccaatacaatcaacacaatcaggaaggccatagatcgaaacgcagaggttcaggtggaagtggttaactttaagaaaaatggacaacgattcgttaacttcttgactatcatacctgtgcgggacgagactggggagtataggtattcaatggggttccagtgtgaaaccgaagggggttctggggggagcggcgggggatctggaagtggcagcggaggcggtacctccggccagggcgatagcctgcacgagcacattgccaatctggccggcagccccgccattaagaagggcatcctgcagacagtgaaggtggtggacgagctcgtgaaagtgatgggccggcacaagcccgagaacatcgtgatcgaaatggccagagagaaccagaccacccagaagggacagaagaacagccgcgagagaatgaagcggatcgaagagggcatcaaagagctgggcagccagatcctgaaagaacaccccgtggaaaacacccagctgcagaacgagaagctgtacctgtactacctgcagaatgggcgggatatgtacgtggaccaggaactggacatcaaccggctgtccgactacgatgtggaccatatcgtgcctcagagctttctgaaggacgactccatcgacaacaaggtgctgaccagaagcgacaagaaccggggcaagagcgacaacgtgccctccgaagaggtcgtgaagaagatgaagaactactggcggcagctgctgaacgccaagctgattacccagagaaagttcgacaatctgaccaaggccgagagaggcggcctgagcgaactggataaggccggcttcatcaagagacagctggtggaaacccggcagatcacaaagcacgtggcacagatcctggactcccggatgaacactaagtacgacgagaatgacaagctgatccgggaagtgaaagtgatcaccctgaagtccaagctggtgtccgatttccggaaggatttccagttttacaaagtgcgcgagatcaacaactaccaccacgcccacgacgcctacctgaacgccgtcgtgggaaccgccctgatcaaaaagtaccctaagctggaaagcgagttcgtgtacggcgactacaaggtgtacgacgtgcggaagatgatcgccaagagcgagcaggaaatcggcaaggctaccgccaagtacttcttctacagcaacatcatgaactttttcaagaccgagattaccctggccaacggcgagatccggaagcggcctctgatcgagacaaacggcgaaaccggggagatcgtgtgggataagggccgggattttgccaccgtgcggaaagtgctgagcatgccccaagtgaatatcgtgaaaaagaccgaggtgcagacaggcggcttcagcaaagagtctatcctgcccaagaggaacagcgataagctgatcgccagaaagaaggactgggaccctaagaagtacggcggcttcgacagccccaccgtggcctattctgtgctggtggtggccaaagtggaaaagggcaagtccaagaaactgaagagtgtgaaagagctgctggggatcaccatcatggaaagaagcagcttcgagaagaatcccatcgactttctggaagccaagggctacaaagaagtgaaaaaggacctgatcatcaagctgcctaagtactccctgttcgagctggaaaacggccggaagagaatgctggcctctgccggcgaactgcagaagggaaacgaactggccctgccctccaaatatgtgaacttcctgtacctggccagccactatgagaagctgaagggctcccccgaggataatgagcagaaacagctgtttgtggaacagcacaagcactacctggacgagatcatcgagcagatcagcgagttctccaagagagtgatcctggccgacgctaatctggacaaagtgctgtccgcctacaacaagcaccgggataagcccatcagagagcaggccgagaatatcatccacctgtttaccctgaccaatctgggagcccctgccgccttcaagtactttgacaccaccatcgaccggaagaggtacaccagcaccaaagaggtgctggacgccaccctgatccaccagagcatcaccggcctgtacgagacacggatcgacctgtctcagctgggaggcgacgaattcgcttcgccgaagaaaaagcgcaaggtcctcgagtctagagggcccttcgaaggtaagcctatccctaaccctctcctcggtctcgattctacgcgtaccggtcatcatcaccatcaccattgagtttaaacccgctgatcagcctcgactgtgccttctagttgccagccatctgttgtttgcccctcccccgtgccttccttgaccctggaaggtgccactcccactgtcctttcctaataaaatgaggaaattgcatcgcattgtctgagtaggtgtcattctattctggggggtggggtggggcaggacagcaagggggaggattgggaagacaatagcaggcatgctggggatgcggtgggctctatggcttctgaggcggaaagaaccagctggggctctagggggtatccccacgcgccctgtagcggcgcattaagcgcggcgggtgtggtggttacgcgcagcgtgaccgctacacttgccagcgccctagcgcccgctcctttcgctttcttcccttcctttctcgccacgttcgccggctttccccgtcaagctctaaatcgggggctccctttagggttccgatttagtgctttacggcacctcgaccccaaaaaacttgattagggtgatggttcacgtagtgggccatcgccctgatagacggtttttcgccctttgacgttggagtccacgttctttaatagtggactcttgttccaaactggaacaacactcaaccctatctcggtctattcttttgatttataagggattttgccgatttcggcctattggttaaaaaatgagctgatttaacaaaaatttaacgcgaattaattctgtggaatgtgtgtcagttagggtgtggaaagtccccaggctccccagcaggcagaagtatgcaaagcatgcatctcaattagtcagcaaccaggtgtggaaagtccccaggctccccagcaggcagaagtatgcaaagcatgcatctcaattagtcagcaaccatagtcccgcccctaactccgcccatcccgcccctaactccgcccagttccgcccattctccgccccatggctgactaattttttttatttatgcagaggccgaggccgcctctgcctctgagctattccagaagtagtgaggaggcttttttggaggcctaggcttttgcaaaaagctcccgggagcttgtatatccattttcggatctgatcaagagacaggatgaggatcgtttcgcatgattgaacaagatggattgcacgcaggttctccggccgcttgggtggagaggctattcggctatgactgggcacaacagacaatcggctgctctgatgccgccgtgttccggctgtcagcgcaggggcgcccggttctttttgtcaagaccgacctgtccggtgccctgaatgaactgcaggacgaggcagcgcggctatcgtggctggccacgacgggcgttccttgcgcagctgtgctcgacgttgtcactgaagcgggaagggactggctgctattgggcgaagtgccggggcaggatctcctgtcatctcaccttgctcctgccgagaaagtatccatcatggctgatgcaatgcggcggctgcatacgcttgatccggctacctgcccattcgaccaccaagcgaaacatcgcatcgagcgagcacgtactcggatggaagccggtcttgtcgatcaggatgatctggacgaagagcatcaggggctcgcgccagccgaactgttcgccaggctcaaggcgcgcatgcccgacggcgaggatctcgtcgtgacccatggcgatgcctgcttgccgaatatcatggtggaaaatggccgcttttctggattcatcgactgtggccggctgggtgtggcggaccgctatcaggacatagcgttggctacccgtgatattgctgaagagcttggcggcgaatgggctgaccgcttcctcgtgctttacggtatcgccgctcccgattcgcagcgcatcgccttctatcgccttcttgacgagttcttctgagcgggactctggggttcgcgaaatgaccgaccaagcgacgcccaacctgccatcacgagatttcgattccaccgccgccttctatgaaaggttgggcttcggaatcgttttccgggacgccggctggatgatcctccagcgcggggatctcatgctggagttcttcgcccaccccaacttgtttattgcagcttataatggttacaaataaagcaatagcatcacaaatttcacaaataaagcatttttttcactgcattctagttgtggtttgtccaaactcatcaatgtatcttatcatgtctgtataccgtcgacctctagctagagcttggcgtaatcatggtcatagctgtttcctgtgtgaaattgttatccgctcacaattccacacaacatacgagccggaagcataaagtgtaaagcctggggtgcctaatgagtgagctaactcacattaattgcgttgcgctcactgcccgctttccagtcgggaaacctgtcgtgccagctgcattaatgaatcggccaacgcgcggggagaggcggtttgcgtattgggcgctcttccgcttcctcgctcactgactcgctgcgctcggtcgttcggctgcggcgagcggtatcagctcactcaaaggcggtaatacggttatccacagaatcaggggataacgcaggaaagaacatgtgagcaaaaggccagcaaaaggccaggaaccgtaaaaaggccgcgttgctggcgtttttccataggctccgcccccctgacgagcatcacaaaaatcgacgctcaagtcagaggtggcgaaacccgacaggactataaagataccaggcgtttccccctggaagctccctcgtgcgctctcctgttccgaccctgccgcttaccggatacctgtccgcctttctcccttcgggaagcgtggcgctttctcatagctcacgctgtaggtatctcagttcggtgtaggtcgttcgctccaagctgggctgtgtgcacgaaccccccgttcagcccgaccgctgcgccttatccggtaactatcgtcttgagtccaacccggtaagacacgacttatcgccactggcagcagccactggtaacaggattagcagagcgaggtatgtaggcggtgctacagagttcttgaagtggtggcctaactacggctacactagaagaacagtatttggtatctgcgctctgctgaagccagttaccttcggaaaaagagttggtagctcttgatccggcaaacaaaccaccgctggtagcggtggtttttttgtttgcaagcagcagattacgcgcagaaaaaaaggatctcaagaagatcctttgatcttttctacggggtctgacgctcagtggaacgaaaactcacgttaagggattttggtcatgagattatcaaaaaggatcttcacctagatccttttaaattaaaaatgaagttttaaatcaatctaaagtatatatgagtaaacttggtctgacagttaccaatgcttaatcagtgaggcacctatctcagcgatctgtctatttcgttcatccatagttgcctgactccccgtcgtgtagataactacgatacgggagggcttaccatctggccccagtgctgcaatgataccgcgagacccacgctcaccggctccagatttatcagcaataaaccagccagccggaagggccgagcgcagaagtggtcctgcaactttatccgcctccatccagtctattaattgttgccgggaagctagagtaagtagttcgccagttaatagtttgcgcaacgttgttgccattgctacaggcatcgtggtgtcacgctcgtcgtttggtatggcttcattcagctccggttcccaacgatcaaggcgagttacatgatcccccatgttgtgcaaaaaagcggttagctccttcggtcctccgatcgttgtcagaagtaagttggccgcagtgttatcactcatggttatggcagcactgcataattctcttactgtcatgccatccgtaagatgcttttctgtgactggtgagtactcaaccaagtcattctgagaatagtgtatgcggcgaccgagttgctcttgcccggcgtcaatacgggataataccgcgccacatagcagaactttaaaagtgctcatcattggaaaacgttcttcggggcgaaaactctcaaggatcttaccgctgttgagatccagttcgatgtaacccactcgtgcacccaactgatcttcagcatcttttactttcaccagcgtttctgggtgagcaaaaacaggaaggcaaaatgccgcaaaaaagggaataagggcgacacggaaatgttgaatactcatactcttcctttttcaatattattgaagcatttatcagggttattgtctcatgagcggatacatatttgaatgtatttagaaaaataaacaaataggggttccgcgcacatttccccgaaaagtgccacctgacgtc

SEQ ID NO: 23 - DNA, 7403 bp, synthetic construct
  source 1..7403: mol_type = other DNA
  misc_feature 929..1051: note = Cre N-ter
  misc_feature 1059..1508: note = nMag
  misc_feature 1524..1547: note = NLS
  misc_feature 1554..1619: note = P2A
  misc_feature 1626..1649: note = NLS
  misc_feature 1656..2105: note = pMag
  misc_feature 2112..3016: note = Cre C-ter
gacggatcgggagatctcccgatcccctatggtgcactctcagtacaatctgctctgatgccgcatagttaagccagtatctgctccctgcttgtgtgttggaggtcgctgagtagtgcgcgagcaaaatttaagctacaacaaggcaaggcttgaccgacaattgcatgaagaatctgcttagggttaggcgttttgcgctgcttcgcgatgtacgggccagatatacgcgttgacattgattattgactagttattaatagtaatcaattacggggtcattagttcatagcccatatatggagttccgcgttacataacttacggtaaatggcccgcctggctgaccgcccaacgacccccgcccattgacgtcaataatgacgtatgttcccatagtaacgccaatagggactttccattgacgtcaatgggtggagtatttacggtaaactgcccacttggcagtacatcaagtgtatcatatgccaagtacgccccctattgacgtcaatgacggtaaatggcccgcctggcattatgcccagtacatgaccttatgggactttcctacttggcagtacatctacgtattagtcatcgctattaccatggtgatgcggttttggcagtacatcaatgggcgtggatagcggtttgactcacggggatttccaagtctccaccccattgacgtcaatgggagtttgttttggcaccaaaatcaacgggactttccaaaatgtcgtaacaactccgccccattgacgcaaatgggcggtaggcgtgtacggtgggaggtctatataagcagagctctctggctaactagagaacccactgcttactggcttatcgaaattaatacgactcactatagggagacccaagctggctagcgtttaaacttaagcttaccaccatggccacctctgatgaagtcaggaagaacctgatggacatgttcagggacaggcaggccttctctgaacacacctggaagatgctcctgtctgtgtgcagatcctgggctgcctggtgcaagctgaacggtacccatactctttatgcccccggtggatatgacattatgggatatctggaccagatcggcaaccggccaaacccgcaggtggaactgggccccgtggatacatcctgcgccttgattctttgtgacctgaaacagaaagacaccccgatagtttacgcgagtgaagccttcctctacatgacaggttacagcaacgcagaggtgctgggccggaattgccggtttctgcaaagccctgacggcatggtgaagcccaagagcacccggaagtacgtggatagtaacacaatcaatactatgcgcaaggcaatcgacaggaatgccgaggtgcaggttgaagtagtcaattttaaaaagaatggacagcgatttgttaatttcctgactatgatacctgttagggacgaaacaggcgagtatcgatactctatgggattccagtgcgaaacagaaggcggaagcggtggcgtgcccaagaagaagaggaaagtcggatccggcagcggcgccaccaacttcagcctgctgaagcaggccggcgacgtggaggagaaccccggccccctcgaggtgcccaagaagaagaggaaagtcggcggacatactctttatgcccccggtggatatgacattatgggatatctgaggcagatcaggaaccggccaaacccgcaggtggaactgggccccgtggatacatcctgcgccttgattctttgtgacctgaaacagaaagacaccccgatagtttacgcgagtgaagccttcctctacatgacaggttacagcaacgcagaggtgctgggccggaattgccggtttctgcaaagccctgacggcatggtgaagcccaagagcacccggaagtacgtggatagtaacacaatcaatactatgcgcaaggcaatcgacaggaatgccgaggtgcaggttgaagtagtcaattttaaaaagaatggacagcgatttgttaatttcctgactatgatacctgttagggacgaaacaggcgagtatcgatactctatgggattccagtgcgaaacagaaggtaccaacaggaaatggttccctgctgaacctgaggatgtgagggactacctcctgtacctgcaagccagaggcctggctgtgaagaccatccaacagcacctgggccagctcaacatgctgcacaggagatctggcctgcctcgcccttctgactccaatgctgtgtccctggtgatgaggagaatcagaaaggagaatgtggatgctggggagagagccaagcaggccctggcctttgaacgcactgactttgaccaagtcagatccctgatggagaactctgacagatgccaggacatcaggaacctggccttcctgggcattgcctacaacaccctgctgcgcattgccgaaattgccagaatcagagtgaaggacatctcccgcaccgatggtgggagaatgctgatccacattggcaggaccaagaccctggtgtccacagctggtgtggagaaggccctgtccctgggggttaccaagctggtggagagatggatctctgtgtctggtgtggctgatgaccccaacaactacctgttctgccgggtcagaaagaatggtgtggctgccccttctgccacctcccaactgtccacccgggccctggaagggatctttgaggccacccaccgcctgatctatggtgccaaggatgactctgggcagagatacctggcctggtctggccactctgccagagtgggtgctgccagggacatggccagggctggtgtgtccatccctgaaatcatgcaggctggtggctggaccaatgtgaacattgtgatgaactacatcagaaacctggactctgagactggggccatggtgaggctgctcgaagatggggactaatctagagggcccgtttaaacccgctgatcagcctcgactgtgccttctagttgccagccatctgttgtttgcccctcccccgtgccttccttgaccctggaaggtgccactcccactgtcctttcctaataaaatgaggaaattgcatcgcattgtctgagtaggtgtcattctattctggggggtggggtggggcaggacagcaagggggaggattgggaagacaatagcaggcatgctggggatgcggtgggctctatggcttctgaggcggaaagaaccagctggggctctagggggtatccccacgcgccctgtagcggcgcattaagcgcggcgggtgtggtggttacgcgcagcgtgaccgctacacttgccagcgccctagcgcccgctcctttcgctttcttcccttcctttctcgccacgttcgccggctttccccgtcaagctctaaatcgggggctccctttagggttccgatttagtgctttacggcacctcgaccccaaaaaacttgattagggtgatggttcacgtagtgggccatcgccctgatagacggtttttcgccctttgacgttggagtccacgttctttaatagtggactcttgttccaaactggaacaacactcaaccctatctcggtctattcttttgatttataagggattttgccgatttcggcctattggttaaaaaatgagctgatttaacaaaaatttaacgcgaattaattctgtggaatgtgtgtcagttagggtgtggaaagtccccaggctccccagcaggcagaagtatgcaaagcatgcatctcaattagtcagcaaccaggtgtggaaagtccccaggctccccagcaggcagaagtatgcaaagcatgcatctcaattagtcagcaaccatagtcccgcccctaactccgcccatcccgcccctaactccgcccagttccgcccattctccgccccatggctgactaattttttttatttatgcagaggccgaggccgcctctgcctctgagctattccagaagtagtgaggaggcttttttggaggcctaggcttttgcaaaaagctcccgggagcttgtatatccattttcggatctgatcaagagacaggatgaggatcgtttcgcatgattgaacaagatggattgcacgcaggttctccggccgcttgggtggagaggctattcggctatgactgggcacaacagacaatcggctgctctgatgccgccgtgttccggctgtcagcgcaggggcgcccggttctttttgtcaagaccgacctgtccggtgccctgaatgaactgcaggacgaggcagcgcggctatcgtggctggccacgacgggcgttccttgcgcagctgtgctcgacgttgtcactgaagcgggaagggactggctgctattgggcgaagtgccggggcaggatctcctgtcatctcaccttgctcctgccgagaaagtatccatcatggctgatgcaatgcggcggctgcatacgcttgatccggctacctgcccattcgaccaccaagcgaaacatcgcatcgagcgagcacgtactcggatggaagccggtcttgtcgatcaggatgatctggacgaagagcatcaggggctcgcgccagccgaactgttcgccaggctcaaggcgcgcatgcccgacggcgaggatctcgtcgtgacccatggcgatgcctgcttgccgaatatcatggtggaaaatggccgcttttctggattcatcgactgtggccggctgggtgtggcggaccgctatcaggacatagcgttggctacccgtgatattgctgaagagcttggcggcgaatgggctgaccgcttcctcgtgctttacggtatcgccgctcccgattcgcagcgcatcgccttctatcgccttcttgacgagttcttctgagcgggactctggggttcgaaatgaccgaccaagcgacgcccaacctgccatcacgagatttcgattccaccgccgccttctatgaaaggttgggcttcggaatcgttttccgggacgccggctggatgatcctccagcgcggggatctcatgctggagttcttcgcccaccccaacttgtttattgcagcttataatggttacaaataaagcaatagcatcacaaatttcacaaataaagcatttttttcactgcattctagttgtggtttgtccaaactcatcaatgtatcttatcatgtctgtataccgtcgacctctagctagagcttggcgtaatcatggtcatagctgtttcctgtgtgaaattgttatccgctcacaattccacacaacatacgagccggaagcataaagtgtaaagcctggggtgcctaatgagtgagctaactcacattaattgcgttgcgctcactgcccgctttccagtcgggaaacctgtcgtgccagctgcattaatgaatcggccaacgcgcggggagaggcggtttgcgtattgggcgctcttccgcttcctcgctcactgactcgctgcgctcggtcgttcggctgcggcgagcggtatcagctcactcaaaggcggtaatacggttatccacagaatcaggggataacgcaggaaagaacatgtgagcaaaaggccagcaaaaggccaggaaccgtaaaaaggccgcgttgctggcgtttttccataggctccgcccccctgacgagcatcacaaaaatcgacgctcaagtcagaggtggcgaaacccgacaggactataaagataccaggcgtttccccctggaagctccctcgtgcgctctcctgttccgaccctgccgcttaccggatacctgtccgcctttctcccttcgggaagcgtggcgctttctcatagctcacgctgtaggtatctcagttcggtgtaggtcgttcgctccaagctgggctgtgtgcacgaaccccccgttcagcccgaccgctgcgccttatccggtaactatcgtcttgagtccaacccggtaagacacgacttatcgccactggcagcagccactggtaacaggattagcagagcgaggtatgtaggcggtgctacagagttcttgaagtggtggcctaactacggctacactagaagaacagtatttggtatctgcgctctgctgaagccagttaccttcggaaaaagagttggtagctcttgatccggcaaacaaaccaccgctggtagcggtttttttgtttgcaagcagcagattacgcgcagaaaaaaaggatctcaagaagatcctttgatcttttctacggggtctgacgctcagtggaacgaaaactcacgttaagggattttggtcatgagattatcaaaaaggatcttcacctagatccttttaaattaaaaatgaagttttaaatcaatctaaagtatatatgagtaaacttggtctgacagttaccaatgcttaatcagtgaggcacctatctcagcgatctgtctatttcgttcatccatagttgcctgactccccgtcgtgtagataactacgatacgggagggcttaccatctggccccagtgctgcaatgataccgcgagacccacgctcaccggctccagatttatcagcaataaaccagccagccggaagggccgagcgcagaagtggtcctgcaactttatccgcctccatccagtctattaattgttgccgggaagctagagtaagtagttcgccagttaatagtttgcgcaacgttgttgccattgctacaggcatcgtggtgtcacgctcgtcgtttggtatggcttcattcagctccggttcccaacgatcaaggcgagttacatgatcccccatgttgtgcaaaaaagcggttagctccttcggtcctccgatcgttgtcagaagtaagttggccgcagtgttatcactcatggttatggcagcactgcataattctcttactgtcatgccatccgtaagatgcttttctgtgactggtgagtactcaaccaagtcattctgagaatagtgtatgcggcgaccgagttgctcttgcccggcgtcaatacgggataataccgcgccacatagcagaactttaaaagtgctcatcattggaaaacgttcttcggggcgaaaactctcaaggatcttaccgctgttgagatccagttcgatgtaacccactcgtgcacccaactgatcttcagcatcttttactttcaccagcgtttctgggtgagcaaaaacaggaaggcaaaatgccgcaaaaaagggaataagggcgacacggaaatgttgaatactcatactcttcctttttcaatattattgaagcatttatcagggttattgtctcatgagcggatacatatttgaatgtatttagaaaaataaacaaataggggttccgcgcacatttccccgaaaagtgccacctgacgtc

SEQ ID NO: 24 - DNA, 7357 bp, synthetic construct
  source 1..7357: mol_type = other DNA
  misc_feature 935..958: note = NLS
  misc_feature 965..1138: note = Cre N-ter
  misc_feature 1145..1594: note = pMag
  misc_feature 1595..2044: note = nMag
  misc_feature 2051..2902: note = Cre C-ter
gacggatcgggagatctcccgatcccctatggtgcactctcagtacaatctgctctgatgccgcatagttaagccagtatctgctccctgcttgtgtgttggaggtcgctgagtagtgcgcgagcaaaatttaagctacaacaaggcaaggcttgaccgacaattgcatgaagaatctgcttagggttaggcgttttgcgctgcttcgcgatgtacgggccagatatacgcgttgacattgattattgactagttattaatagtaatcaattacggggtcattagttcatagcccatatatggagttccgcgttacataacttacggtaaatggcccgcctggctgaccgcccaacgacccccgcccattgacgtcaataatgacgtatgttcccatagtaacgccaatagggactttccattgacgtcaatgggtggagtatttacggtaaactgcccacttggcagtacatcaagtgtatcatatgccaagtacgccccctattgacgtcaatgacggtaaatggcccgcctggcattatgcccagtacatgaccttatgggactttcctacttggcagtacatctacgtattagtcatcgctattaccatggtgatgcggttttggcagtacatcaatgggcgtggatagcggtttgactcacggggatttccaagtctccaccccattgacgtcaatgggagtttgttttggcaccaaaatcaacgggactttccaaaatgtcgtaacaactccgccccattgacgcaaatgggcggtaggcgtgtacggtgggaggtctatataagcagagctctctggctaactagagaacccactgcttactggcttatcgaaattaatacgactcactatagggagacccaagctggctagcgtttaaacttaagcttgaattcgccgccaccatggtgcccaagaagaagaggaaagtcggcggatccaacctgctgactgtgcaccaaaacctgcctgccctccctgtggatgccacctctgatgaagtcaggaagaacctgatggacatgttcagggacaggcaggccttctctgaacacacctggaagatgctcctgtctgtgtgcagatcctgggctgcctggtgcaagctgaacaccggtcataccctgtatgctccagggggatacgacattatgggctatcttcgtcagatcaggaaccggcccaatcctcaggttgaactggggccggttgacaccagttgcgcacttatcctgtgtgacttgaaacagaaagacaccccaattgtgtatgccagtgaggctttcctgtacatgaccggctacagcaacgctgaagtgctggggcgcaactgtcgattcctacaaagtcctgatgggatggtgaaaccgaagagcacacgcaagtatgtggatagcaacaccataaacactatgagaaaggccatagatagaaatgccgaagtccaggtggaggtagtgaactttaagaagaatggccagaggtttgtgaatttcttaactatgattccagttcgcgacgaaaccggagagtatcggtactctatgggctttcagtgcgagacagagcacaccctatacgctcccggaggctacgacatcatgggatatttggaccaaatcgggaatcggccgaatccccaggtagaactcggccctgttgataccagctgtgcgctgatcctttgcgatctgaagcagaaggatactccaatcgtatacgccagtgaagccttcctctatatgactggatatagtaacgccgaggtgctcggccggaattgcagatttctgcaatcccctgacggcatggtcaagcccaaatcaacccgtaagtacgtggattccaatactattaacacgatgcgtaaggcaattgaccggaacgctgaggtgcaggtggaagttgtcaacttcaagaaaaacggtcaacgctttgtcaatttcctcacgatgatcccagtcagggatgagactggcgaatataggtattctatgggattccagtgtgagacagaaggtaccaacaggaaatggttccctgctgaacctgaggatgtgagggactacctcctgtacctgcaagccagaggcctggctgtgaagaccatccaacagcacctgggccagctcaacatgctgcacaggagatctggcctgcctcgcccttctgactccaatgctgtgtccctggtgatgaggagaatcagaaaggagaatgtggatgctggggagagagccaagcaggccctggcctttgaacgcactgactttgaccaagtcagatccctgatggagaactctgacagatgccaggacatcaggaacctggccttcctgggcattgcctacaacaccctgctgcgcattgccgaaattgccagaatcagagtgaaggacatctcccgcaccgatggtgggagaatgctgatccacattggcaggaccaagaccctggtgtccacagctggtgtggagaaggccctgtccctgggggttaccaagctggtggagagatggatctctgtgtctggtgtggctgatgaccccaacaactacctgttctgccgggtcagaaagaatggtgtggctgccccttctgccacctcccaactgtccacccgggccctggaagggatctttgaggccacccaccgcctgatctatggtgccaaggatgactctgggcagagatacctggcctggtctggccactctgccagagtgggtgctgccagggacatggccagggctggtgtgtccatccctgaaatcatgcaggctggtggctggaccaatgtgaacattgtgatgaactacatcagaaacctggactctgagactggggccatggtgaggctgctcgaagatggggactaagcggccgcctcgagtctagagggcccgtttaaacccgctgatcagcctcgactgtgccttctagttgccagccatctgttgtttgcccctcccccgtgccttccttgaccctggaaggtgccactcccactgtcctttcctaataaaatgaggaaattgcatcgcattgtctgagtaggtgtcattctattctggggggtggggtggggcaggacagcaagggggaggattgggaagacaatagcaggcatgctggggatgcggtgggctctatggcttctgaggcggaaagaaccagctggggctctagggggtatccccacgcgccctgtagcggcgcattaagcgcggcgggtgtggtggttacgcgcagcgtgaccgctacacttgccagcgccctagcgcccgctcctttcgctttcttcccttcctttctcgccacgttcgccggctttccccgtcaagctctaaatcgggggctccctttagggttccgatttagtgctttacggcacctcgaccccaaaaaacttgattagggtgatggttcacgtagtgggccatcgccctgatagacggtttttcgccctttgacgttggagtccacgttctttaatagtggactcttgttccaaactggaacaacactcaaccctatctcggtctattcttttgatttataagggattttgccgatttcggcctattggttaaaaaatgagctgatttaacaaaaatttaacgcgaattaattctgtggaatgtgtgtcagttagggtgtggaaagtccccaggctccccagcaggcagaagtatgcaaagcatgcatctcaattagtcagcaaccaggtgtggaaagtccccaggctccccagcaggcagaagtatgcaaagcatgcatctcaattagtcagcaaccatagtcccgcccctaactccgcccatcccgcccctaactccgcccagttccgcccattctccgccccatggctgactaattttttttatttatgcagaggccgaggccgcctctgcctctgagctattccagaagtagtgaggaggcttttttggaggcctaggcttttgcaaaaagctcccgggagcttgtatatccattttcggatctgatcaagagacaggatgaggatcgtttcgcatgattgaacaagatggattgcacgcaggttctccggccgcttgggtggagaggctattcggctatgactgggcacaacagacaatcggctgctctgatgccgccgtgttccggctgtcagcgcaggggcgcccggttctttttgtcaagaccgacctgtccggtgccctgaatgaactgcaggacgaggcagcgcggctatcgtggctggccacgacgggcgttccttgcgcagctgtgctcgacgttgtcactgaagcgggaagggactggctgctattgggcgaagtgccggggcaggatctcctgtcatctcaccttgctcctgccgagaaagtatccatcatggctgatgcaatgcggcggctgcatacgcttgatccggctacctgcccattcgaccaccaagcgaaacatcgcatcgagcgagcacgtactcggatggaagccggtcttgtcgatcaggatgatctggacgaagagcatcaggggctcgcgccagccgaactgttcgccaggctcaaggcgcgcatgcccgacggcgaggatctcgtcgtgacccatggcgatgcctgcttgccgaatatcatggtggaaaatggccgcttttctggattcatcgactgtggccggctgggtgtggcggaccgctatcaggacatagcgttggctacccgtgatattgctgaagagcttggcggcgaatgggctgaccgcttcctcgtgctttacggtatcgccgctcccgattcgcagcgcatcgccttctatcgccttcttgacgagttcttctgagcgggactctggggttcgaaatgaccgaccaagcgacgcccaacctgccatcacgagatttcgattccaccgccgccttctatgaaaggttgggcttcggaatcgttttccgggacgccggctggatgatcctccagcgcggggatctcatgctggagttcttcgcccaccccaacttgtttattgcagcttataatggttacaaataaagcaatagcatcacaaatttcacaaataaagcatttttttcactgcattctagttgtggtttgtccaaactcatcaatgtatcttatcatgtctgtataccgtcgacctctagctagagcttggcgtaatcatggtcatagctgtttcctgtgtgaaattgttatccgctcacaattccacacaacatacgagccggaagcataaagtgtaaagcctggggtgcctaatgagtgagctaactcacattaattgcgttgcgctcactgcccgctttccagtcgggaaacctgtcgtgccagctgcattaatgaatcggccaacgcgcggggagaggcggtttgcgtattgggcgctcttccgcttcctcgctcactgactcgctgcgctcggtcgttcggctgcggcgagcggtatcagctcactcaaaggcggtaatacggttatccacagaatcaggggataacgcaggaaagaacatgtgagcaaaaggccagcaaaaggccaggaaccgtaaaaaggccgcgttgctggcgtttttccataggctccgcccccctgacgagcatcacaaaaatcgacgctcaagtcagaggtggcgaaacccgacaggactataaagataccaggcgtttccccctggaagctccctcgtgcgctctcctgttccgaccctgccgcttaccggatacctgtccgcctttctcccttcgggaagcgtggcgctttctcatagctcacgctgtaggtatctcagttcggtgtaggtcgttcgctccaagctgggctgtgtgcacgaaccccccgttcagcccgaccgctgcgccttatccggtaactatcgtcttgagtccaacccggtaagacacgacttatcgccactggcagcagccactggtaacaggattagcagagcgaggtatgtaggcggtgctacagagttcttgaagtggtggcctaactacggctacactagaagaacagtatttggtatctgcgctctgctgaagccagttaccttcggaaaaagagttggtagctcttgatccggcaaacaaaccaccgctggtagcggtttttttgtttgcaagcagcagattacgcgcagaaaaaaaggatctcaagaagatcctttgatcttttctacggggtctgacgctcagtggaacgaaaactcacgttaagggattttggtcatgagattatcaaaaaggatcttcacctagatccttttaaattaaaaatgaagttttaaatcaatctaaagtatatatgagtaaacttggtctgacagttaccaatgcttaatcagtgaggcacctatctcagcgatctgtctatttcgttcatccatagttgcctgactccccgtcgtgtagataactacgatacgggagggcttaccatctggccccagtgctgcaatgataccgcgagacccacgctcaccggctccagatttatcagcaataaaccagccagccggaagggccgagcgcagaagtggtcctgcaactttatccgcctccatccagtctattaattgttgccgggaagctagagtaagtagttcgccagttaatagtttgcgcaacgttgttgccattgctacaggcatcgtggtgtcacgctcgtcgtttggtatggcttcattcagctccggttcccaacgatcaaggcgagttacatgatcccccatgttgtgcaaaaaagcggttagctccttcggtcctccgatcgttgtcagaagtaagttggccgcagtgttatcactcatggttatggcagcactgcataattctcttactgtcatgccatccgtaagatgcttttctgtgactggtgagtactcaaccaagtcattctgagaatagtgtatgcggcgaccgagttgctcttgcccggcgtcaatacgggataataccgcgccacatagcagaactttaaaagtgctcatcattggaaaacgttcttcggggcgaaaactctcaaggatcttaccgctgttgagatccagttcgatgtaacccactcgtgcacccaactgatcttcagcatcttttactttcaccagcgtttctgggtgagcaaaaacaggaaggcaaaatgccgcaaaaaagggaataagggcgacacggaaatgttgaatactcatactcttcctttttcaatattattgaagcatttatcagggttattgtctcatgagcggatacatatttgaatgtatttagaaaaataaacaaataggggttccgcgcacatttccccgaaaagtgccacctgacgtc

SEQ ID NO: 25 - DNA, 7877 bp, synthetic construct
  source 1..7877: mol_type = other DNA
  misc_feature 917..950: note = loxP
  polyA_site 957..1752
  misc_feature 1759..1792: note = loxP
  misc_feature 1808..3436: note = firefly luciferase
gacggatcgggagatctcccgatcccctatggtgcactctcagtacaatctgctctgatgccgcatagttaagccagtatctgctccctgcttgtgtgttggaggtcgctgagtagtgcgcgagcaaaatttaagctacaacaaggcaaggcttgaccgacaattgcatgaagaatctgcttagggttaggcgttttgcgctgcttcgcgatgtacgggccagatatacgcgttgacattgattattgactagttattaatagtaatcaattacggggtcattagttcatagcccatatatggagttccgcgttacataacttacggtaaatggcccgcctggctgaccgcccaacgacccccgcccattgacgtcaataatgacgtatgttcccatagtaacgccaatagggactttccattgacgtcaatgggtggagtatttacggtaaactgcccacttggcagtacatcaagtgtatcatatgccaagtacgccccctattgacgtcaatgacggtaaatggcccgcctggcattatgcccagtacatgaccttatgggactttcctacttggcagtacatctacgtattagtcatcgctattaccatggtgatgcggttttggcagtacatcaatgggcgtggatagcggtttgactcacggggatttccaagtctccaccccattgacgtcaatgggagtttgttttggcaccaaaatcaacgggactttccaaaatgtcgtaacaactccgccccattgacgcaaatgggcggtaggcgtgtacggtgggaggtctatataagcagagctctctggctaactagagaacccactgcttactggcttatcgaaattaatacgactcactatagggagacccaagctggctagcgtttaaacttaagcttataacttcgtatagcatacattatacgaagttatggtaccgcagatctgcgactctagaggatctgcgactctagaggatcataatcagccataccacatttgtagaggttttacttgctttaaaaaacctcccacacctccccctgaacctgaaacataaaatgaatgcaattgttgttgttaacttgtttattgcagcttataatggttacaaataaagcaatagcatcacaaatttcacaaataaagcatttttttcactgcattctagttgtggtttgtccaaactcatcaatgtatcttatcatgtctggatctgcgactctagaggatcataatcagccataccacatttgtagaggttttacttgctttaaaaaacctcccacacctccccctgaacctgaaacataaaatgaatgcaattgttgttgttaacttgtttattgcagcttataatggttacaaataaagcaatagcatcacaaatttcacaaataaagcatttttttcactgcattctagttgtggtttgtccaaactcatcaatgtatcttatcatgtctggatctgcgactctagaggatcataatcagccataccacatttgtagaggttttacttgctttaaaaaacctcccacacctccccctgaacctgaaacataaaatgaatgcaattgttgttgttaacttgtttattgcagcttataatggttacaaataaagcaatagcatcacaaatttcacaaataaagcatttttttcactgcattctagttgtggtttgtccaaactcatcaatgtatcttatcatgtctggatccccatcaagcatcgatataacttcgtatagcatacattatacgaagttatgaattcgccgccatggaagatgccaaaaacattaagaagggcccagcgccattctacccactcgaagacgggaccgccggcgagcagctgcacaaagccatgaagcgctacgccctggtgcccggcaccatcgcctttaccgacgcacatatcgaggtggacattacctacgccgagtacttcgagatgagcgttcggctggcagaagctatgaagcgctatgggctgaatacaaaccatcggatcgtggtgtgcagcgagaatagcttgcagttcttcatgcccgtgttgggtgccctgttcatcggtgtggctgtggccccagctaacgacatctacaacgagcgcgagctgctgaacagcatgggcatcagccagcccaccgtcgtattcgtgagcaagaaagggctgcaaaagatcctcaacgtgcaaaagaagctaccgatcatacaaaagatcatcatcatggatagcaagaccgactaccagggcttccaaagcatgtacaccttcgtgacttcccatttgccacccggcttcaacgagtacgacttcgtgcccgagagcttcgaccgggacaaaaccatcgccctgatcatgaacagtagtggcagtaccggattgcccaagggcgtagccctaccgcaccgcaccgcttgtgtccgattcagtcatgcccgcgaccccatcttcggcaaccagatcatccccgacaccgctatcctcagcgtggtgccatttcaccacggcttcggcatgttcaccacgctgggctacttgatctgcggctttcgggtcgtgctcatgtaccgcttcgaggaggagctattcttgcgcagcttgcaagactataagattcaatctgccctgctggtgcccacactatttagcttcttcgctaagagcactctcatcgacaagtacgacctaagcaacttgcacgagatcgccagcggcggggcgccgctcagcaaggaggtaggtgaggccgtggccaaacgcttccacctaccaggcatccgccagggctacggcctgacagaaacaaccagcgccattctgatcacccccgaaggggacgacaagcctggcgcagtaggcaaggtggtgcccttcttcgaggctaaggtggtggacttggacaccggtaagacactgggtgtgaaccagcgcggcgagctgtgcgtccgtggccccatgatcatgagcggctacgttaacaaccccgaggctacaaacgctctcatcgacaaggacggctggctgcacagcggcgacatcgcctactgggacgaggacgagcacttcttcatcgtggaccggctgaagagcctgatcaaatacaagggctaccaggtagccccagccgaactggagagcatcctgctgcaacaccccaacatcttcgacgccggggtcgccggcctgcccgacgacgatgccggcgagctgcccgccgcagtcgtcgtgctggaacacggtaaaaccatgaccgagaaggagatcgtggactatgtggccagccaggttacaaccgccaagaagctgcgcggtggtgttgtgttcgtggacgaggtgcctaaaggactgaccggcaagttggacgcccgcaagatccgcgagattctcattaaggccaagaagtaactcgaggggcccgtttaaacccgctgatcagcctcgactgtgccttctagttgccagccatctgttgtttgcccctcccccgtgccttccttgaccctggaaggtgccactcccactgtcctttcctaataaaatgaggaaattgcatcgcattgtctgagtaggtgtcattctattctggggggtggggtggggcaggacagcaagggggaggattgggaagacaatagcaggcatgctggggatgcggtgggctctatggcttctgaggcggaaagaaccagctggggctctagggggtatccccacgcgccctgtagcggcgcattaagcgcggcgggtgtggtggttacgcgcagcgtgaccgctacacttgccagcgccctagcgcccgctcctttcgctttcttcccttcctttctcgccacgttcgccggctttccccgtcaagctctaaatcgggggctccctttagggttccgatttagtgctttacggcacctcgaccccaaaaaacttgattagggtgatggttcacgtagtgggccatcgccctgatagacggtttttcgccctttgacgttggagtccacgttctttaatagtggactcttgttccaaactggaacaacactcaaccctatctcggtctattcttttgatttataagggattttgccgatttcggcctattggttaaaaaatgagctgatttaacaaaaatttaacgcgaattaattctgtggaatgtgtgtcagttagggtgtggaaagtccccaggctccccagcaggcagaagtatgcaaagcatgcatctcaattagtcagcaaccaggtgtggaaagtccccaggctccccagcaggcagaagtatgcaaagcatgcatctcaattagtcagcaaccatagtcccgcccctaactccgcccatcccgcccctaactccgcccagttccgcccattctccgccccatggctgactaattttttttatttatgcagaggccgaggccgcctctgcctctgagctattccagaagtagtgaggaggcttttttggaggcctaggcttttgcaaaaagctcccgggagcttgtatatccattttcggatctgatcaagagacaggatgaggatcgtttcgcatgattgaacaagatggattgcacgcaggttctccggccgcttgggtggagaggctattcggctatgactgggcacaacagacaatcggctgctctgatgccgccgtgttccggctgtcagcgcaggggcgcccggttctttttgtcaagaccgacctgtccggtgccctgaatgaactgcaggacgaggcagcgcggctatcgtggctggccacgacgggcgttccttgcgcagctgtgctcgacgttgtcactgaagcgggaagggactggctgctattgggcgaagtgccggggcaggatctcctgtcatctcaccttgctcctgccgagaaagtatccatcatggctgatgcaatgcggcggctgcatacgcttgatccggctacctgcccattcgaccaccaagcgaaacatcgcatcgagcgagcacgtactcggatggaagccggtcttgtcgatcaggatgatctggacgaagagcatcaggggctcgcgccagccgaactgttcgccaggctcaaggcgcgcatgcccgacggcgaggatctcgtcgtgacccatggcgatgcctgcttgccgaatatcatggtggaaaatggccgcttttctggattcatcgactgtggccggctgggtgtggcggaccgctatcaggacatagcgttggctacccgtgatattgctgaagagcttggcggcgaatgggctgaccgcttcctcgtgctttacggtatcgccgctcccgattcgcagcgcatcgccttctatcgccttcttgacgagttcttctgagcgggactctggggttcgaaatgaccgaccaagcgacgcccaacctgccatcacgagatttcgattccaccgccgccttctatgaaaggttgggcttcggaatcgttttccgggacgccggctggatgatcctccagcgcggggatctcatgctggagttcttcgcccaccccaacttgtttattgcagcttataatggttacaaataaagcaatagcatcacaaatttcacaaataaagcatttttttcactgcattctagttgtggtttgtccaaactcatcaatgtatcttatcatgtctgtataccgtcgacctctagctagagcttggcgtaatcatggtcatagctgtttcctgtgtgaaattgttatccgctcacaattccacacaacatacgagccggaagcataaagtgtaaagcctggggtgcctaatgagtgagctaactcacattaattgcgttgcgctcactgcccgctttccagtcgggaaacctgtcgtgccagctgcattaatgaatcggccaacgcgcggggagaggcggtttgcgtattgggcgctcttccgcttcctcgctcactgactcgctgcgctcggtcgttcggctgcggcgagcggtatcagctcactcaaaggcggtaatacggttatccacagaatcaggggataacgcaggaaagaacatgtgagcaaaaggccagcaaaaggccaggaaccgtaaaaaggccgcgttgctggcgtttttccataggctccgcccccctgacgagcatcacaaaaatcgacgctcaagtcagaggtggcgaaacccgacaggactataaagataccaggcgtttccccctggaagctccctcgtgcgctctcctgttccgaccctgccgcttaccggatacctgtccgcctttctcccttcgggaagcgtggcgctttctcatagctcacgctgtaggtatctcagttcggtgtaggtcgttcgctccaagctgggctgtgtgcacgaaccccccgttcagcccgaccgctgcgccttatccggtaactatcgtcttgagtccaacccggtaagacacgacttatcgccactggcagcagccactggtaacaggattagcagagcgaggtatgtaggcggtgctacagagttcttgaagtggtggcctaactacggctacactagaagaacagtatttggtatctgcgctctgctgaagccagttaccttcggaaaaagagttggtagctcttgatccggcaaacaaaccaccgctggtagcggtttttttgtttgcaagcagcagattacgcgcagaaaaaaaggatctcaagaagatcctttgatcttttctacggggtctgacgctcagtggaacgaaaactcacgttaagggattttggtcatgagattatcaaaaaggatcttcacctagatccttttaaattaaaaatgaagttttaaatcaatctaaagtatatatgagtaaacttggtctgacagttaccaatgcttaatcagtgaggcacctatctcagcgatctgtctatttcgttcatccatagttgcctgactccccgtcgtgtagataactacgatacgggagggcttaccatctggccccagtgctgcaatgataccgcgagacccacgctcaccggctccagatttatcagcaataaaccagccagccggaagggccgagcgcagaagtggtcctgcaactttatccgcctccatccagtctattaattgttgccgggaagctagagtaagtagttcgccagttaatagtttgcgcaacgttgttgccattgctacaggcatcgtggtgtcacgctcgtcgtttggtatggcttcattcagctccggttcccaacgatcaaggcgagttacatgatcccccatgttgtgcaaaaaagcggttagctccttcggtcctccgatcgttgtcagaagtaagttggccgcagtgttatcactcatggttatggcagcactgcataattctcttactgtcatgccatccgtaagatgcttttctgtgactggtgagtactcaaccaagtcattctgagaatagtgtatgcggcgaccgagttgctcttgcccggcgtcaatacgggataataccgcgccacatagcagaactttaaaagtgctcatcattggaaaacgttcttcggggcgaaaactctcaaggatcttaccgctgttgagatccagttcgatgtaacccactcgtgcacccaactgatcttcagcatcttttactttcaccagcgtttctgggtgagcaaaaacaggaaggcaaaatgccgcaaaaaagggaataagggcgacacggaaatgttgaatactcatactcttcctttttcaatattattgaagcatttatcagggttattgtctcatgagcggatacatatttgaatgtatttagaaaaataaacaaataggggttccgcgcacatttccccgaaaagtgccacctgacgtc

SEQ ID NO: 26 - DNA, 5960 bp, synthetic construct
  source 1..5960: mol_type = other DNA
  misc_feature 926..946: note = NLS
  misc_feature 947..1024: note = Flp N-ter
  misc_feature 1070..1519: note = nMagHigh1
gacggatcgggagatctcccgatcccctatggtgcactctcagtacaatctgctctgatgccgcatagttaagccagtatctgctccctgcttgtgtgttggaggtcgctgagtagtgcgcgagcaaaatttaagctacaacaaggcaaggcttgaccgacaattgcatgaagaatctgcttagggttaggcgttttgcgctgcttcgcgatgtacgggccagatatacgcgttgacattgattattgactagttattaatagtaatcaattacggggtcattagttcatagcccatatatggagttccgcgttacataacttacggtaaatggcccgcctggctgaccgcccaacgacccccgcccattgacgtcaataatgacgtatgttcccatagtaacgccaatagggactttccattgacgtcaatgggtggagtatttacggtaaactgcccacttggcagtacatcaagtgtatcatatgccaagtacgccccctattgacgtcaatgacggtaaatggcccgcctggcattatgcccagtacatgaccttatgggactttcctacttggcagtacatctacgtattagtcatcgctattaccatggtgatgcggttttggcagtacatcaatgggcgtggatagcggtttgactcacggggatttccaagtctccaccccattgacgtcaatgggagtttgttttggcaccaaaatcaacgggactttccaaaatgtcgtaacaactccgccccattgacgcaaatgggcggtaggcgtgtacggtgggaggtctatataagcagagctctctggctaactagagaacccactgcttactggcttatcgaaattaatacgactcactatagggagacccaagctggctagcgtttaaacttaagcttaccaccatgcccaagaagaagaggaaggtgagccagttcgacatcctgtgcaagaccccccccaaggtgctggtgcggcagttcgtggagagattcgagaggcccagcggtggaggcggttcaggcggaggtggcagcggcggtggcggatcgcatactctttatgcccccggtggatatgacattatgggatatctggaccagatcggcaaccggccaaacccgcaggtggaactgggccccgtggatacatcctgcgccttgattctttgtgacctgaaacagaaagacaccccgatagtttacgcgagtgaagccttcctctacatgacaggttacagcaacgcagaggtgctgggccggaattgccggtttctgcaaagccctgacggcatggtgaagcccaagagcacccggaagtacgtggatagtaacacaatcaatactatccgcaaggcaatcgacaggaatgccgaggtgcaggttgaagtagtcaattttaaaaagaatggacagcgatttgttaatttcctgactatcatacctgttagggacgaaacaggcgagtatcgatactctatgggattccagtgcgaaacagaataatctagagggcccgtttaaacccgctgatcagcctcgactgtgccttctagttgccagccatctgttgtttgcccctcccccgtgccttccttgaccctggaaggtgccactcccactgtcctttcctaataaaatgaggaaattgcatcgcattgtctgagtaggtgtcattctattctggggggtggggtggggcaggacagcaagggggaggattgggaagacaatagcaggcatgctggggatgcggtgggctctatggcttctgaggcggaaagaaccagctggggctctagggggtatccccacgcgccctgtagcggcgcattaagcgcggcgggtgtggtggttacgcgcagcgtgaccgctacacttgccagcgccctagcgcccgctcctttcgctttcttcccttcctttctcgccacgttcgccggctttccccgtcaagctctaaatcgggggctccctttagggttccgatttagtgctttacggcacctcgaccccaaaaaacttgattagggtgatggttcacgtagtgggccatcgccctgatagacggtttttcgccctttgacgttggagtccacgttctttaatagtggactcttgttccaaactggaacaacactcaaccctatctcggtctattcttttgatttataagggattttgccgatttcggcctattggttaaaaaatgagctgatttaacaaaaatttaacgcgaattaattctgtggaatgtgtgtcagttagggtgtggaaagtccccaggctccccagcaggcagaagtatgcaaagcatgcatctcaattagtcagcaaccaggtgtggaaagtccccaggctccccagcaggcagaagtatgcaaagcatgcatctcaattagtcagcaaccatagtcccgcccctaactccgcccatcccgcccctaactccgcccagttccgcccattctccgccccatggctgactaattttttttatttatgcagaggccgaggccgcctctgcctctgagctattccagaagtagtgaggaggcttttttggaggcctaggcttttgcaaaaagctcccgggagcttgtatatccattttcggatctgatcaagagacaggatgaggatcgtttcgcatgattgaacaagatggattgcacgcaggttctccggccgcttgggtggagaggctattcggctatgactgggcacaacagacaatcggctgctctgatgccgccgtgttccggctgtcagcgcaggggcgcccggttctttttgtcaagaccgacctgtccggtgccctgaatgaactgcaggacgaggcagcgcggctatcgtggctggccacgacgggcgttccttgcgcagctgtgctcgacgttgtcactgaagcgggaagggactggctgctattgggcgaagtgccggggcaggatctcctgtcatctcaccttgctcctgccgagaaagtatccatcatggctgatgcaatgcggcggctgcatacgcttgatccggctacctgcccattcgaccaccaagcgaaacatcgcatcgagcgagcacgtactcggatggaagccggtcttgtcgatcaggatgatctggacgaagagcatcaggggctcgcgccagccgaactgttcgccaggctcaaggcgcgcatgcccgacggcgaggatctcgtcgtgacccatggcgatgcctgcttgccgaatatcatggtggaaaatggccgcttttctggattcatcgactgtggccggctgggtgtggcggaccgctatcaggacatagcgttggctacccgtgatattgctgaagagcttggcggcgaatgggctgaccgcttcctcgtgctttacggtatcgccgctcccgattcgcagcgcatcgccttctatcgccttcttgacgagttcttctgagcgggactctggggttcgaaatgaccgaccaagcgacgcccaacctgccatcacgagatttcgattccaccgccgccttctatgaaaggttgggcttcggaatcgttttccgggacgccggctggatgatcctccagcgcggggatctcatgctggagttcttcgcccaccccaacttgtttattgcagcttataatggttacaaataaagcaatagcatcacaaatttcacaaataaagcatttttttcactgcattctagttgtggtttgtccaaactcatcaatgtatcttatcatgtctgtataccgtcgacctctagctagagcttggcgtaatcatggtcatagctgtttcctgtgtgaaattgttatccgctcacaattccacacaacatacgagccggaagcataaagtgtaaagcctggggtgcctaatgagtgagctaactcacattaattgcgttgcgctcactgcccgctttccagtcgggaaacctgtcgtgccagctgcattaatgaatcggccaacgcgcggggagaggcggtttgcgtattgggcgctcttccgcttcctcgctcactgactcgctgcgctcggtcgttcggctgcggcgagcggtatcagctcactcaaaggcggtaatacggttatccacagaatcaggggataacgcaggaaagaacatgtgagcaaaaggccagcaaaaggccaggaaccgtaaaaaggccgcgttgctggcgtttttccataggctccgcccccctgacgagcatcacaaaaatcgacgctcaagtcagaggtggcgaaacccgacaggactataaagataccaggcgtttccccctggaagctccctcgtgcgctctcctgttccgaccctgccgcttaccggatacctgtccgcctttctcccttcgggaagcgtggcgctttctcatagctcacgctgtaggtatctcagttcggtgtaggtcgttcgctccaagctgggctgtgtgcacgaaccccccgttcagcccgaccgctgcgccttatccggtaactatcgtcttgagtccaacccggtaagacacgacttatcgccactggcagcagccactggtaacaggattagcagagcgaggtatgtaggcggtgctacagagttcttgaagtggtggcctaactacggctacactagaagaacagtatttggtatctgcgctctgctgaagccagttaccttcggaaaaagagttggtagctcttgatccggcaaacaaaccaccgctggtagcggtttttttgtttgcaagcagcagattacgcgcagaaaaaaaggatctcaagaagatcctttgatcttttctacggggtctgacgctcagtggaacgaaaactcacgttaagggattttggtcatgagattatcaaaaaggatcttcacctagatccttttaaattaaaaatgaagttttaaatcaatctaaagtatatatgagtaaacttggtctgacagttaccaatgcttaatcagtgaggcacctatctcagcgatctgtctatttcgttcatccatagttgcctgactccccgtcgtgtagataactacgatacgggagggcttaccatctggccccagtgctgcaatgataccgcgagacccacgctcaccggctccagatttatcagcaataaaccagccagccggaagggccgagcgcagaagtggtcctgcaactttatccgcctccatccagtctattaattgttgccgggaagctagagtaagtagttcgccagttaatagtttgcgcaacgttgttgccattgctacaggcatcgtggtgtcacgctcgtcgtttggtatggcttcattcagctccggttcccaacgatcaaggcgagttacatgatcccccatgttgtgcaaaaaagcggttagctccttcggtcctccgatcgttgtcagaagtaagttggccgcagtgttatcactcatggttatggcagcactgcataattctcttactgtcatgccatccgtaagatgcttttctgtgactggtgagtactcaaccaagtcattctgagaatagtgtatgcggcgaccgagttgctcttgcccggcgtcaatacgggataataccgcgccacatagcagaactttaaaagtgctcatcattggaaaacgttcttcggggcgaaaactctcaaggatcttaccgctgttgagatccagttcgatgtaacccactcgtgcacccaactgatcttcagcatcttttactttcaccagcgtttctgggtgagcaaaaacaggaaggcaaaatgccgcaaaaaagggaataagggcgacacggaaatgttgaatactcatactcttcctttttcaatattattgaagcatttatcagggttattgtctcatgagcggatacatatttgaatgtatttagaaaaataaacaaataggggttccgcgcacatttccccgaaaagtgccacctgacgtc

SEQ ID NO: 27 - DNA, 7049 bp, synthetic construct
  source 1..7049: mol_type = other DNA
  misc_feature 926..1375: note = pMagHigh1
  misc_feature 1421..2608: note = Flp C-ter
gacggatcgggagatctcccgatcccctatggtgcactctcagtacaatctgctctgatgccgcatagttaagccagtatctgctccctgcttgtgtgttggaggtcgctgagtagtgcgcgagcaaaatttaagctacaacaaggcaaggcttgaccgacaattgcatgaagaatctgcttagggttaggcgttttgcgctgcttcgcgatgtacgggccagatatacgcgttgacattgattattgactagttattaatagtaatcaattacggggtcattagttcatagcccatatatggagttccgcgttacataacttacggtaaatggcccgcctggctgaccgcccaacgacccccgcccattgacgtcaataatgacgtatgttcccatagtaacgccaatagggactttccattgacgtcaatgggtggagtatttacggtaaactgcccacttggcagtacatcaagtgtatcatatgccaagtacgccccctattgacgtcaatgacggtaaatggcccgcctggcattatgcccagtacatgaccttatgggactttcctacttggcagtacatctacgtattagtcatcgctattaccatggtgatgcggttttggcagtacatcaatgggcgtggatagcggtttgactcacggggatttccaagtctccaccccattgacgtcaatgggagtttgttttggcaccaaaatcaacgggactttccaaaatgtcgtaacaactccgccccattgacgcaaatgggcggtaggcgtgtacggtgggaggtctatataagcagagctctctggctaactagagaacccactgcttactggcttatcgaaattaatacgactcactatagggagacccaagctggctagcgtttaaacttaagcttaccaccatgcatactctttatgcccccggtggatatgacattatgggatatctgaggcagatcaggaaccggccaaacccgcaggtggaactgggccccgtggatacatcctgcgccttgattctttgtgacctgaaacagaaagacaccccgatagtttacgcgagtgaagccttcctctacatgacaggttacagcaacgcagaggtgctgggccggaattgccggtttctgcaaagccctgacggcatggtgaagcccaagagcacccggaagtacgtggatagtaacacaatcaatactatccgcaaggcaatcgacaggaatgccgaggtgcaggttgaagtagtcaattttaaaaagaatggacagcgatttgttaatttcctgactatcatacctgttagggacgaaacaggcgagtatcgatactctatgggattccagtgcgaaacagaaggtggaggcggttcaggcggaggtggcagcggcggtggcggatcgggcgagaagatcgccagctgtgccgccgagctgacctacctgtgctggatgatcacccacaacggcaccgccatcaagagggccaccttcatgagctacaacaccatcatcagcaacagcctgagcttcgacatcgtgaacaagagcctgcagttcaagtacaagacccagaaggccaccatcctggaggccagcctgaagaagctgatccccgcctgggagttcaccatcatcccttacaacggccagaagcaccagagcgacatcaccgacatcgtgtccagcctgcagctgcagttcgagagcagcgaggaggccgacaagggcaacagccacagcaagaagatgctgaaggccctgctgtccgagggcgagagcatctgggagatcaccgagaagatcctgaacagcttcgagtacaccagcaggttcaccaagaccaagaccctgtaccagttcctgttcctggccacattcatcaactgcggcaggttcagcgacatcaagaacgtggaccccaagagcttcaagctggtgcagaacaagtacctgggcgtgatcattcagtgcctggtgaccgagaccaagacaagcgtgtccaggcacatctactttttcagcgccagaggcaggatcgaccccctggtgtacctggacgagttcctgaggaacagcgagcccgtgctgaagagagtgaacaggaccggcaacagcagcagcaacaagcaggagtaccagctgctgaaggacaacctggtgcgcagctacaacaaggccctgaagaagaacgccccctaccccatcttcgctatcaagaacggccctaagagccacatcggcaggcacctgatgaccagctttctgagcatgaagggcctgaccgagctgacaaacgtggtgggcaactggagcgacaagagggcctccgccgtggccaggaccacctacacccaccagatcaccgccatccccgaccactacttcgccctggtgtccaggtactacgcctacgaccccatcagcaaggagatgatcgccctgaaggacgagaccaaccccatcgaggagtggcagcacatcgagcagctgaagggcagcgccgagggcagcatcagataccccgcctggaacggcatcatcagccaggaggtgctggactacctgagcagctacatcaacaggcggatctgatctagagggcccgtttaaacccgctgatcagcctcgactgtgccttctagttgccagccatctgttgtttgcccctcccccgtgccttccttgaccctggaaggtgccactcccactgtcctttcctaataaaatgaggaaattgcatcgcattgtctgagtaggtgtcattctattctggggggtggggtggggcaggacagcaagggggaggattgggaagacaatagcaggcatgctggggatgcggtgggctctatggcttctgaggcggaaagaaccagctggggctctagggggtatccccacgcgccctgtagcggcgcattaagcgcggcgggtgtggtggttacgcgcagcgtgaccgctacacttgccagcgccctagcgcccgctcctttcgctttcttcccttcctttctcgccacgttcgccggctttccccgtcaagctctaaatcgggggctccctttagggttccgatttagtgctttacggcacctcgaccccaaaaaacttgattagggtgatggttcacgtagtgggccatcgccctgatagacggtttttcgccctttgacgttggagtccacgttctttaatagtggactcttgttccaaactggaacaacactcaaccctatctcggtctattcttttgatttataagggattttgccgatttcggcctattggttaaaaaatgagctgatttaacaaaaatttaacgcgaattaattctgtggaatgtgtgtcagttagggtgtggaaagtccccaggctccccagcaggcagaagtatgcaaagcatgcatctcaattagtcagcaaccaggtgtggaaagtccccaggctccccagcaggcagaagtatgcaaagcatgcatctcaattagtcagcaaccatagtcccgcccctaactccgcccatcccgcccctaactccgcccagttccgcccattctccgccccatggctgactaattttttttatttatgcagaggccgaggccgcctctgcctctgagctattccagaagtagtgaggaggcttttttggaggcctaggcttttgcaaaaagctcccgggagcttgtatatccattttcggatctgatcaagagacaggatgaggatcgtttcgcatgattgaacaagatggattgcacgcaggttctccggccgcttgggtggagaggctattcggctatgactgggcacaacagacaatcggctgctctgatgccgccgtgttccggctgtcagcgcaggggcgcccggttctttttgtcaagaccgacctgtccggtgccctgaatgaactgcaggacgaggcagcgcggctatcgtggctggccacgacgggcgttccttgcgcagctgtgctcgacgttgtcactgaagcgggaagggactggctgctattgggcgaagtgccggggcaggatctcctgtcatctcaccttgctcctgccgagaaagtatccatcatggctgatgcaatgcggcggctgcatacgcttgatccggctacctgcccattcgaccaccaagcgaaacatcgcatcgagcgagcacgtactcggatggaagccggtcttgtcgatcaggatgatctggacgaagagcatcaggggctcgcgccagccgaactgttcgccaggctcaaggcgcgcatgcccgacggcgaggatctcgtcgtgacccatggcgatgcctgcttgccgaatatcatggtggaaaatggccgcttttctggattcatcgactgtggccggctgggtgtggcggaccgctatcaggacatagcgttggctacccgtgatattgctgaagagcttggcggcgaatgggctgaccgcttcctcgtgctttacggtatcgccgctcccgattcgcagcgcatcgccttctatcgccttcttgacgagttcttctgagcgggactctggggttcgaaatgaccgaccaagcgacgcccaacctgccatcacgagatttcgattccaccgccgccttctatgaaaggttgggcttcggaatcgttttccgggacgccggctggatgatcctccagcgcggggatctcatgctggagttcttcgcccaccccaacttgtttattgcagcttataatggttacaaataaagcaatagcatcacaaatttcacaaataaagcatttttttcactgcattctagttgtggtttgtccaaactcatcaatgtatcttatcatgtctgtataccgtcgacctctagctagagcttggcgtaatcatggtcatagctgtttcctgtgtgaaattgttatccgctcacaattccacacaacatacgagccggaagcataaagtgtaaagcctggggtgcctaatgagtgagctaactcacattaattgcgttgcgctcactgcccgctttccagtcgggaaacctgtcgtgccagctgcattaatgaatcggccaacgcgcggggagaggcggtttgcgtattgggcgctcttccgcttcctcgctcactgactcgctgcgctcggtcgttcggctgcggcgagcggtatcagctcactcaaaggcggtaatacggttatccacagaatcaggggataacgcaggaaagaacatgtgagcaaaaggccagcaaaaggccaggaaccgtaaaaaggccgcgttgctggcgtttttccataggctccgcccccctgacgagcatcacaaaaatcgacgctcaagtcagaggtggcgaaacccgacaggactataaagataccaggcgtttccccctggaagctccctcgtgcgctctcctgttccgaccctgccgcttaccggatacctgtccgcctttctcccttcgggaagcgtggcgctttctcatagctcacgctgtaggtatctcagttcggtgtaggtcgttcgctccaagctgggctgtgtgcacgaaccccccgttcagcccgaccgctgcgccttatccggtaactatcgtcttgagtccaacccggtaagacacgacttatcgccactggcagcagccactggtaacaggattagcagagcgaggtatgtaggcggtgctacagagttcttgaagtggtggcctaactacggctacactagaagaacagtatttggtatctgcgctctgctgaagccagttaccttcggaaaaagagttggtagctcttgatccggcaaacaaaccaccgctggtagcggtttttttgtttgcaagcagcagattacgcgcagaaaaaaaggatctcaagaagatcctttgatcttttctacggggtctgacgctcagtggaacgaaaactcacgttaagggattttggtcatgagattatcaaaaaggatcttcacctagatccttttaaattaaaaatgaagttttaaatcaatctaaagtatatatgagtaaacttggtctgacagttaccaatgcttaatcagtgaggcacctatctcagcgatctgtctatttcgttcatccatagttgcctgactccccgtcgtgtagataactacgatacgggagggcttaccatctggccccagtgctgcaatgataccgcgagacccacgctcaccggctccagatttatcagcaataaaccagccagccggaagggccgagcgcagaagtggtcctgcaactttatccgcctccatccagtctattaattgttgccgggaagctagagtaagtagttcgccagttaatagtttgcgcaacgttgttgccattgctacaggcatcgtggtgtcacgctcgtcgtttggtatggcttcattcagctccggttcccaacgatcaaggcgagttacatgatcccccatgttgtgcaaaaaagcggttagctccttcggtcctccgatcgttgtcagaagtaagttggccgcagtgttatcactcatggttatggcagcactgcataattctcttactgtcatgccatccgtaagatgcttttctgtgactggtgagtactcaaccaagtcattctgagaatagtgtatgcggcgaccgagttgctcttgcccggcgtcaatacgggataataccgcgccacatagcagaactttaaaagtgctcatcattggaaaacgttcttcggggcgaaaactctcaaggatcttaccgctgttgagatccagttcgatgtaacccactcgtgcacccaactgatcttcagcatcttttactttcaccagcgtttctgggtgagcaaaaacaggaaggcaaaatgccgcaaaaaagggaataagggcgacacggaaatgttgaatactcatactcttcctttttcaatattattgaagcatttatcagggttattgtctcatgagcggatacatatttgaatgtatttagaaaaataaacaaataggggttccgcgcacatttccccgaaaagtgccacctgacgtc

SEQ ID NO: 28 - DNA, 7628 bp, synthetic construct
  source 1..7628: mol_type = other DNA
  misc_feature 926..997: note = Flp N-term
  misc_feature 1046..1495: note = pMag
  misc_feature 1496..1945: note = nMagHigh1
  misc_feature 1994..3187: note = Flp C-term
gacggatcgggagatctcccgatcccctatggtgcactctcagtacaatctgctctgatgccgcatagttaagccagtatctgctccctgcttgtgtgttggaggtcgctgagtagtgcgcgagcaaaatttaagctacaacaaggcaaggcttgaccgacaattgcatgaagaatctgcttagggttaggcgttttgcgctgcttcgcgatgtacgggccagatatacgcgttgacattgattattgactagttattaatagtaatcaattacggggtcattagttcatagcccatatatggagttccgcgttacataacttacggtaaatggcccgcctggctgaccgcccaacgacccccgcccattgacgtcaataatgacgtatgttcccatagtaacgccaatagggactttccattgacgtcaatgggtggagtatttacggtaaactgcccacttggcagtacatcaagtgtatcatatgccaagtacgccccctattgacgtcaatgacggtaaatggcccgcctggcattatgcccagtacatgaccttatgggactttcctacttggcagtacatctacgtattagtcatcgctattaccatggtgatgcggttttggcagtacatcaatgggcgtggatagcggtttgactcacggggatttccaagtctccaccccattgacgtcaatgggagtttgttttggcaccaaaatcaacgggactttccaaaatgtcgtaacaactccgccccattgacgcaaatgggcggtaggcgtgtacggtgggaggtctatataagcagagctctctggctaactagagaacccactgcttactggcttatcgaaattaatacgactcactatagggagacccaagctggctagcgtttaaacttaagcttaccaccatgagccagttcgacatcctgtgcaagaccccccccaaggtgctggtgcggcagttcgtggagagattcgagaggctcgaggccagcccctctaaccctggagcctccaacggcagcggtacccataccctgtatgctccagggggatacgacattatgggctatcttcgtcagatcaggaaccggcccaatcctcaggttgaactggggccggttgacaccagttgcgcacttatcctgtgtgacttgaaacagaaagacaccccaattgtgtatgccagtgaggctttcctgtacatgaccggctacagcaacgctgaagtgctggggcgcaactgtcgattcctacaaagtcctgatgggatggtgaaaccgaagagcacacgcaagtatgtggatagcaacaccataaacactatgagaaaggccatagatagaaatgccgaagtccaggtggaggtagtgaactttaagaagaatggccagaggtttgtgaatttcttaactatgattccagttcgcgacgaaaccggagagtatcggtactctatgggctttcagtgcgagacagagcacaccctatacgctcccggaggctacgacatcatgggatatttggaccaaatcgggaatcggccgaatccccaggtagaactcggccctgttgataccagctgtgcgctgatcctttgcgatctgaagcagaaggatactccaatcgtatacgccagtgaagccttcctctatatgactggatatagtaacgccgaggtgctcggccggaattgcagatttctgcaatcccctgacggcatggtcaagcccaaatcaacccgtaagtacgtggattccaatactattaacacgatccgtaaggcaattgaccggaacgctgaggtgcaggtggaagttgtcaacttcaagaaaaacggtcaacgctttgtcaatttcctcacgatcatcccagtcagggatgagactggcgaatataggtattctatgggattccagtgtgagacagaactcgaggctagtcccagcaatcctggagcctccaacggctctggtacccccagcggcgagaagatcgccagctgtgccgccgagctgacctacctgtgctggatgatcacccacaacggcaccgccatcaagagggccaccttcatgagctacaacaccatcatcagcaacagcctgagcttcgacatcgtgaacaagagcctgcagttcaagtacaagacccagaaggccaccatcctggaggccagcctgaagaagctgatccccgcctgggagttcaccatcatcccttacaacggccagaagcaccagagcgacatcaccgacatcgtgtccagcctgcagctgcagttcgagagcagcgaggaggccgacaagggcaacagccacagcaagaagatgctgaaggccctgctgtccgagggcgagagcatctgggagatcaccgagaagatcctgaacagcttcgagtacaccagcaggttcaccaagaccaagaccctgtaccagttcctgttcctggccacattcatcaactgcggcaggttcagcgacatcaagaacgtggaccccaagagcttcaagctggtgcagaacaagtacctgggcgtgatcattcagtgcctggtgaccgagaccaagacaagcgtgtccaggcacatctactttttcagcgccagaggcaggatcgaccccctggtgtacctggacgagttcctgaggaacagcgagcccgtgctgaagagagtgaacaggaccggcaacagcagcagcaacaagcaggagtaccagctgctgaaggacaacctggtgcgcagctacaacaaggccctgaagaagaacgccccctaccccatcttcgctatcaagaacggccctaagagccacatcggcaggcacctgatgaccagctttctgagcatgaagggcctgaccgagctgacaaacgtggtgggcaactggagcgacaagagggcctccgccgtggccaggaccacctacacccaccagatcaccgccatccccgaccactacttcgccctggtgtccaggtactacgcctacgaccccatcagcaaggagatgatcgccctgaaggacgagaccaaccccatcgaggagtggcagcacatcgagcagctgaagggcagcgccgagggcagcatcagataccccgcctggaacggcatcatcagccaggaggtgctggactacctgagcagctacatcaacaggcggatctaatctagagggcccgtttaaacccgctgatcagcctcgactgtgccttctagttgccagccatctgttgtttgcccctcccccgtgccttccttgaccctggaaggtgccactcccactgtcctttcctaataaaatgaggaaattgcatcgcattgtctgagtaggtgtcattctattctggggggtggggtggggcaggacagcaagggggaggattgggaagacaatagcaggcatgctggggatgcggtgggctctatggcttctgaggcggaaagaaccagctggggctctagggggtatccccacgcgccctgtagcggcgcattaagcgcggcgggtgtggtggttacgcgcagcgtgaccgctacacttgccagcgccctagcgcccgctcctttcgctttcttcccttcctttctcgccacgttcgccggctttccccgtcaagctctaaatcgggggctccctttagggttccgatttagtgctttacggcacctcgaccccaaaaaacttgattagggtgatggttcacgtagtgggccatcgccctgatagacggtttttcgccctttgacgttggagtccacgttctttaatagtggactcttgttccaaactggaacaacactcaaccctatctcggtctattcttttgatttataagggattttgccgatttcggcctattggttaaaaaatgagctgatttaacaaaaatttaacgcgaattaattctgtggaatgtgtgtcagttagggtgtggaaagtccccaggctccccagcaggcagaagtatgcaaagcatgcatctcaattagtcagcaaccaggtgtggaaagtccccaggctccccagcaggcagaagtatgcaaagcatgcatctcaattagtcagcaaccatagtcccgcccctaactccgcccatcccgcccctaactccgcccagttccgcccattctccgccccatggctgactaattttttttatttatgcagaggccgaggccgcctctgcctctgagctattccagaagtagtgaggaggcttttttggaggcctaggcttttgcaaaaagctcccgggagcttgtatatccattttcggatctgatcaagagacaggatgaggatcgtttcgcatgattgaacaagatggattgcacgcaggttctccggccgcttgggtggagaggctattcggctatgactgggcacaacagacaatcggctgctctgatgccgccgtgttccggctgtcagcgcaggggcgcccggttctttttgtcaagaccgacctgtccggtgccctgaatgaactgcaggacgaggcagcgcggctatcgtggctggccacgacgggcgttccttgcgcagctgtgctcgacgttgtcactgaagcgggaagggactggctgctattgggcgaagtgccggggcaggatctcctgtcatctcaccttgctcctgccgagaaagtatccatcatggctgatgcaatgcggcggctgcatacgcttgatccggctacctgcccattcgaccaccaagcgaaacatcgcatcgagcgagcacgtactcggatggaagccggtcttgtcgatcaggatgatctggacgaagagcatcaggggctcgcgccagccgaactgttcgccaggctcaaggcgcgcatgcccgacggcgaggatctcgtcgtgacccatggcgatgcctgcttgccgaatatcatggtggaaaatggccgcttttctggattcatcgactgtggccggctgggtgtggcggaccgctatcaggacatagcgttggctacccgtgatattgctgaagagcttggcggcgaatgggctgaccgcttcctcgtgctttacggtatcgccgctcccgattcgcagcgcatcgccttctatcgccttcttgacgagttcttctgagcgggactctggggttcgaaatgaccgaccaagcgacgcccaacctgccatcacgagatttcgattccaccgccgccttctatgaaaggttgggcttcggaatcgttttccgggacgccggctggatgatcctccagcgcggggatctcatgctggagttcttcgcccaccccaacttgtttattgcagcttataatggttacaaataaagcaatagcatcacaaatttcacaaataaagcatttttttcactgcattctagttgtggtttgtccaaactcatcaatgtatcttatcatgtctgtataccgtcgacctctagctagagcttggcgtaatcatggtcatagctgtttcctgtgtgaaattgttatccgctcacaattccacacaacatacgagccggaagcataaagtgtaaagcctggggtgcctaatgagtgagctaactcacattaattgcgttgcgctcactgcccgctttccagtcgggaaacctgtcgtgccagctgcattaatgaatcggccaacgcgcggggagaggcggtttgcgtattgggcgctcttccgcttcctcgctcactgactcgctgcgctcggtcgttcggctgcggcgagcggtatcagctcactcaaaggcggtaatacggttatccacagaatcaggggataacgcaggaaagaacatgtgagcaaaaggccagcaaaaggccaggaaccgtaaaaaggccgcgttgctggcgtttttccataggctccgcccccctgacgagcatcacaaaaatcgacgctcaagtcagaggtggcgaaacccgacaggactataaagataccaggcgtttccccctggaagctccctcgtgcgctctcctgttccgaccctgccgcttaccggatacctgtccgcctttctcccttcgggaagcgtggcgctttctcatagctcacgctgtaggtatctcagttcggtgtaggtcgttcgctccaagctgggctgtgtgcacgaaccccccgttcagcccgaccgctgcgccttatccggtaactatcgtcttgagtccaacccggtaagacacgacttatcgccactggcagcagccactggtaacaggattagcagagcgaggtatgtaggcggtgctacagagttcttgaagtggtggcctaactacggctacactagaagaacagtatttggtatctgcgctctgctgaagccagttaccttcggaaaaagagttggtagctcttgatccggcaaacaaaccaccgctggtagcggtttttttgtttgcaagcagcagattacgcgcagaaaaaaaggatctcaagaagatcctttgatcttttctacggggtctgacgctcagtggaacgaaaactcacgttaagggattttggtcatgagattatcaaaaaggatcttcacctagatccttttaaattaaaaatgaagttttaaatcaatctaaagtatatatgagtaaacttggtctgacagttaccaatgcttaatcagtgaggcacctatctcagcgatctgtctatttcgttcatccatagttgcctgactccccgtcgtgtagataactacgatacgggagggcttaccatctggccccagtgctgcaatgataccgcgagacccacgctcaccggctccagatttatcagcaataaaccagccagccggaagggccgagcgcagaagtggtcctgcaactttatccgcctccatccagtctattaattgttgccgggaagctagagtaagtagttcgccagttaatagtttgcgcaacgttgttgccattgctacaggcatcgtggtgtcacgctcgtcgtttggtatggcttcattcagctccggttcccaacgatcaaggcgagttacatgatcccccatgttgtgcaaaaaagcggttagctccttcggtcctccgatcgttgtcagaagtaagttggccgcagtgttatcactcatggttatggcagcactgcataattctcttactgtcatgccatccgtaagatgcttttctgtgactggtgagtactcaaccaagtcattctgagaatagtgtatgcggcgaccgagttgctcttgcccggcgtcaatacgggataataccgcgccacatagcagaactttaaaagtgctcatcattggaaaacgttcttcggggcgaaaactctcaaggatcttaccgctgttgagatccagttcgatgtaacccactcgtgcacccaactgatcttcagcatcttttactttcaccagcgtttctgggtgagcaaaaacaggaaggcaaaatgccgcaaaaaagggaataagggcgacacggaaatgttgaatactcatactcttcctttttcaatattattgaagcatttatcagggttattgtctcatgagcggatacatatttgaatgtatttagaaaaataaacaaataggggttccgcgcacatttccccgaaaagtgccacctgacgtc

SEQ ID NO: 29 - DNA, 7883 bp, synthetic construct
  source 1..7883: mol_type = other DNA
  misc_feature 917..950: note = FRT
  polyA_site 964..1742
  misc_feature 1759..1792: note = FRT
  misc_feature 1808..3436: note = firefly luciferase
gacggatcgggagatctcccgatcccctatggtgcactctcagtacaatctgctctgatgccgcatagttaagccagtatctgctccctgcttgtgtgttggaggtcgctgagtagtgcgcgagcaaaatttaagctacaacaaggcaaggcttgaccgacaattgcatgaagaatctgcttagggttaggcgttttgcgctgcttcgcgatgtacgggccagatatacgcgttgacattgattattgactagttattaatagtaatcaattacggggtcattagttcatagcccatatatggagttccgcgttacataacttacggtaaatggcccgcctggctgaccgcccaacgacccccgcccattgacgtcaataatgacgtatgttcccatagtaacgccaatagggactttccattgacgtcaatgggtggagtatttacggtaaactgcccacttggcagtacatcaagtgtatcatatgccaagtacgccccctattgacgtcaatgacggtaaatggcccgcctggcattatgcccagtacatgaccttatgggactttcctacttggcagtacatctacgtattagtcatcgctattaccatggtgatgcggttttggcagtacatcaatgggcgtggatagcggtttgactcacggggatttccaagtctccaccccattgacgtcaatgggagtttgttttggcaccaaaatcaacgggactttccaaaatgtcgtaacaactccgccccattgacgcaaatgggcggtaggcgtgtacggtgggaggtctatataagcagagctctctggctaactagagaacccactgcttactggcttatcgaaattaatacgactcactatagggagacccaagctggctagcgtttaaacttaagcttgaagttcctatactttctagagaataggaacttcggtaccgcagatctgcgactctagaggatctgcgactctagaggatcataatcagccataccacatttgtagaggttttacttgctttaaaaaacctcccacacctccccctgaacctgaaacataaaatgaatgcaattgttgttgttaacttgtttattgcagcttataatggttacaaataaagcaatagcatcacaaatttcacaaataaagcatttttttcactgcattctagttgtggtttgtccaaactcatcaatgtatcttatcatgtctggatctgcgactctagaggatcataatcagccataccacatttgtagaggttttacttgctttaaaaaacctcccacacctccccctgaacctgaaacataaaatgaatgcaattgttgttgttaacttgtttattgcagcttataatggttacaaataaagcaatagcatcacaaatttcacaaataaagcatttttttcactgcattctagttgtggtttgtccaaactcatcaatgtatcttatcatgtctggatctgcgactctagaggatcataatcagccataccacatttgtagaggttttacttgctttaaaaaacctcccacacctccccctgaacctgaaacataaaatgaatgcaattgttgttgttaacttgtttattgcagcttataatggttacaaataaagcaatagcatcacaaatttcacaaataaagcatttttttcactgcattctagttgtggtttgtccaaactcatcaatgtatcttatcatgtctggatccccatcaagcatcgatgaagttcctatactttctagagaataggaacttcgaatccgccgccatggaagatgccaaaaacattaagaagggcccagcgccattctacccactcgaagacgggaccgccggcgagcagctgcacaaagccatgaagcgctacgccctggtgcccggcaccatcgcctttaccgacgcacatatcgaggtggacattacctacgccgagtacttcgagatgagcgttcggctggcagaagctatgaagcgctatgggctgaatacaaaccatcggatcgtggtgtgcagcgagaatagcttgcagttcttcatgcccgtgttgggtgccctgttcatcggtgtggctgtggccccagctaacgacatctacaacgagcgcgagctgctgaacagcatgggcatcagccagcccaccgtcgtattcgtgagcaagaaagggctgcaaaagatcctcaacgtgcaaaagaagctaccgatcatacaaaagatcatcatcatggatagcaagaccgactaccagggcttccaaagcatgtacaccttcgtgacttcccatttgccacccggcttcaacgagtacgacttcgtgcccgagagcttcgaccgggacaaaaccatcgccctgatcatgaacagtagtggcagtaccggattgcccaagggcgtagccctaccgcaccgcaccgcttgtgtccgattcagtcatgcccgcgaccccatcttcggcaaccagatcatccccgacaccgctatcctcagcgtggtgccatttcaccacggcttcggcatgttcaccacgctgggctacttgatctgcggctttcgggtcgtgctcatgtaccgcttcgaggaggagctattcttgcgcagcttgcaagactataagattcaatctgccctgctggtgcccacactatttagcttcttcgctaagagcactctcatcgacaagtacgacctaagcaacttgcacgagatcgccagcggcggggcgccgctcagcaaggaggtaggtgaggccgtggccaaacgcttccacctaccaggcatccgccagggctacggcctgacagaaacaaccagcgccattctgatcacccccgaaggggacgacaagcctggcgcagtaggcaaggtggtgcccttcttcgaggctaaggtggtggacttggacaccggtaagacactgggtgtgaaccagcgcggcgagctgtgcgtccgtggccccatgatcatgagcggctacgttaacaaccccgaggctacaaacgctctcatcgacaaggacggctggctgcacagcggcgacatcgcctactgggacgaggacgagcacttcttcatcgtggaccggctgaagagcctgatcaaatacaagggctaccaggtagccccagccgaactggagagcatcctgctgcaacaccccaacatcttcgacgccggggtcgccggcctgcccgacgacgatgccggcgagctgcccgccgcagtcgtcgtgctggaacacggtaaaaccatgaccgagaaggagatcgtggactatgtggccagccaggttacaaccgccaagaagctgcgcggtggtgttgtgttcgtggacgaggtgcctaaaggactgaccggcaagttggacgcccgcaagatccgcgagattctcattaaggccaagaagtaactcgagtctagagggcccgtttaaacccgctgatcagcctcgactgtgccttctagttgccagccatctgttgtttgcccctcccccgtgccttccttgaccctggaaggtgccactcccactgtcctttcctaataaaatgaggaaattgcatcgcattgtctgagtaggtgtcattctattctggggggtggggtggggcaggacagcaagggggaggattgggaagacaatagcaggcatgctggggatgcggtgggctctatggcttctgaggcggaaagaaccagctggggctctagggggtatccccacgcgccctgtagcggcgcattaagcgcggcgggtgtggtggttacgcgcagcgtgaccgctacacttgccagcgccctagcgcccgctcctttcgctttcttcccttcctttctcgccacgttcgccggctttccccgtcaagctctaaatcgggggctccctttagggttccgatttagtgctttacggcacctcgaccccaaaaaacttgattagggtgatggttcacgtagtgggccatcgccctgatagacggtttttcgccctttgacgttggagtccacgttctttaatagtggactcttgttccaaactggaacaacactcaaccctatctcggtctattcttttgatttataagggattttgccgatttcggcctattggttaaaaaatgagctgatttaacaaaaatttaacgcgaattaattctgtggaatgtgtgtcagttagggtgtggaaagtccccaggctccccagcaggcagaagtatgcaaagcatgcatctcaattagtcagcaaccaggtgtggaaagtccccaggctccccagcaggcagaagtatgcaaagcatgcatctcaattagtcagcaaccatagtcccgcccctaactccgcccatcccgcccctaactccgcccagttccgcccattctccgccccatggctgactaattttttttatttatgcagaggccgaggccgcctctgcctctgagctattccagaagtagtgaggaggcttttttggaggcctaggcttttgcaaaaagctcccgggagcttgtatatccattttcggatctgatcaagagacaggatgaggatcgtttcgcatgattgaacaagatggattgcacgcaggttctccggccgcttgggtggagaggctattcggctatgactgggcacaacagacaatcggctgctctgatgccgccgtgttccggctgtcagcgcaggggcgcccggttctttttgtcaagaccgacctgtccggtgccctgaatgaactgcaggacgaggcagcgcggctatcgtggctggccacgacgggcgttccttgcgcagctgtgctcgacgttgtcactgaagcgggaagggactggctgctattgggcgaagtgccggggcaggatctcctgtcatctcaccttgctcctgccgagaaagtatccatcatggctgatgcaatgcggcggctgcatacgcttgatccggctacctgcccattcgaccaccaagcgaaacatcgcatcgagcgagcacgtactcggatggaagccggtcttgtcgatcaggatgatctggacgaagagcatcaggggctcgcgccagccgaactgttcgccaggctcaaggcgcgcatgcccgacggcgaggatctcgtcgtgacccatggcgatgcctgcttgccgaatatcatggtggaaaatggccgcttttctggattcatcgactgtggccggctgggtgtggcggaccgctatcaggacatagcgttggctacccgtgatattgctgaagagcttggcggcgaatgggctgaccgcttcctcgtgctttacggtatcgccgctcccgattcgcagcgcatcgccttctatcgccttcttgacgagttcttctgagcgggactctggggttcgaaatgaccgaccaagcgacgcccaacctgccatcacgagatttcgattccaccgccgccttctatgaaaggttgggcttcggaatcgttttccgggacgccggctggatgatcctccagcgcggggatctcatgctggagttcttcgcccaccccaacttgtttattgcagcttataatggttacaaataaagcaatagcatcacaaatttcacaaataaagcatttttttcactgcattctagttgtggtttgtccaaactcatcaatgtatcttatcatgtctgtataccgtcgacctctagctagagcttggcgtaatcatggtcatagctgtttcctgtgtgaaattgttatccgctcacaattccacacaacatacgagccggaagcataaagtgtaaagcctggggtgcctaatgagtgagctaactcacattaattgcgttgcgctcactgcccgctttccagtcgggaaacctgtcgtgccagctgcattaatgaatcggccaacgcgcggggagaggcggtttgcgtattgggcgctcttccgcttcctcgctcactgactcgctgcgctcggtcgttcggctgcggcgagcggtatcagctcactcaaaggcggtaatacggttatccacagaatcaggggataacgcaggaaagaacatgtgagcaaaaggccagcaaaaggccaggaaccgtaaaaaggccgcgttgctggcgtttttccataggctccgcccccctgacgagcatcacaaaaatcgacgctcaagtcagaggtggcgaaacccgacaggactataaagataccaggcgtttccccctggaagctccctcgtgcgctctcctgttccgaccctgccgcttaccggatacctgtccgcctttctcccttcgggaagcgtggcgctttctcatagctcacgctgtaggtatctcagttcggtgtaggtcgttcgctccaagctgggctgtgtgcacgaaccccccgttcagcccgaccgctgcgccttatccggtaactatcgtcttgagtccaacccggtaagacacgacttatcgccactggcagcagccactggtaacaggattagcagagcgaggtatgtaggcggtgctacagagttcttgaagtggtggcctaactacggctacactagaagaacagtatttggtatctgcgctctgctgaagccagttaccttcggaaaaagagttggtagctcttgatccggcaaacaaaccaccgctggtagcggtttttttgtttgcaagcagcagattacgcgcagaaaaaaaggatctcaagaagatcctttgatcttttctacggggtctgacgctcagtggaacgaaaactcacgttaagggattttggtcatgagattatcaaaaaggatcttcacctagatccttttaaattaaaaatgaagttttaaatcaatctaaagtatatatgagtaaacttggtctgacagttaccaatgcttaatcagtgaggcacctatctcagcgatctgtctatttcgttcatccatagttgcctgactccccgtcgtgtagataactacgatacgggagggcttaccatctggccccagtgctgcaatgataccgcgagacccacgctcaccggctccagatttatcagcaataaaccagccagccggaagggccgagcgcagaagtggtcctgcaactttatccgcctccatccagtctattaattgttgccgggaagctagagtaagtagttcgccagttaatagtttgcgcaacgttgttgccattgctacaggcatcgtggtgtcacgctcgtcgtttggtatggcttcattcagctccggttcccaacgatcaaggcgagttacatgatcccccatgttgtgcaaaaaagcggttagctccttcggtcctccgatcgttgtcagaagtaagttggccgcagtgttatcactcatggttatggcagcactgcataattctcttactgtcatgccatccgtaagatgcttttctgtgactggtgagtactcaaccaagtcattctgagaatagtgtatgcggcgaccgagttgctcttgcccggcgtcaatacgggataataccgcgccacatagcagaactttaaaagtgctcatcattggaaaacgttcttcggggcgaaaactctcaaggatcttaccgctgttgagatccagttcgatgtaacccactcgtgcacccaactgatcttcagcatcttttactttcaccagcgtttctgggtgagcaaaaacaggaaggcaaaatgccgcaaaaaagggaataagggcgacacggaaatgttgaatactcatactcttcctttttcaatattattgaagcatttatcagggttattgtctcatgagcggatacatatttgaatgtatttagaaaaataaacaaataggggttccgcgcacatttccccgaaaagtgccacctgacgtc

SEQ ID NO: 30 - DNA, 9038 bp, synthetic construct
  source 1..9038: mol_type = other DNA
  misc_feature 917..950: note = FRT
  polyA_site 964..1742
  misc_feature 1759..1792: note = FRT
  misc_feature 1808..2500: note = mKate2
  misc_feature 2507..4156: note = Alaluc
gacggatcgggagatctcccgatcccctatggtgcactctcagtacaatctgctctgatgccgcatagttaagccagtatctgctccctgcttgtgtgttggaggtcgctgagtagtgcgcgagcaaaatttaagctacaacaaggcaaggcttgaccgacaattgcatgaagaatctgcttagggttaggcgttttgcgctgcttcgcgatgtacgggccagatatacgcgttgacattgattattgactagttattaatagtaatcaattacggggtcattagttcatagcccatatatggagttccgcgttacataacttacggtaaatggcccgcctggctgaccgcccaacgacccccgcccattgacgtcaataatgacgtatgttcccatagtaacgccaatagggactttccattgacgtcaatgggtggagtatttacggtaaactgcccacttggcagtacatcaagtgtatcatatgccaagtacgccccctattgacgtcaatgacggtaaatggcccgcctggcattatgcccagtacatgaccttatgggactttcctacttggcagtacatctacgtattagtcatcgctattaccatggtgatgcggttttggcagtacatcaatgggcgtggatagcggtttgactcacggggatttccaagtctccaccccattgacgtcaatgggagtttgttttggcaccaaaatcaacgggactttccaaaatgtcgtaacaactccgccccattgacgcaaatgggcggtaggcgtgtacggtgggaggtctatataagcagagctctctggctaactagagaacccactgcttactggcttatcgaaattaatacgactcactatagggagacccaagctggctagcgtttaaacttaagcttgaagttcctatactttctagagaataggaacttcggtaccgcagatctgcgactctagaggatctgcgactctagaggatcataatcagccataccacatttgtagaggttttacttgctttaaaaaacctcccacacctccccctgaacctgaaacataaaatgaatgcaattgttgttgttaacttgtttattgcagcttataatggttacaaataaagcaatagcatcacaaatttcacaaataaagcatttttttcactgcattctagttgtggtttgtccaaactcatcaatgtatcttatcatgtctggatctgcgactctagaggatcataatcagccataccacatttgtagaggttttacttgctttaaaaaacctcccacacctccccctgaacctgaaacataaaatgaatgcaattgttgttgttaacttgtttattgcagcttataatggttacaaataaagcaatagcatcacaaatttcacaaataaagcatttttttcactgcattctagttgtggtttgtccaaactcatcaatgtatcttatcatgtctggatctgcgactctagaggatcataatcagccataccacatttgtagaggttttacttgctttaaaaaacctcccacacctccccctgaacctgaaacataaaatgaatgcaattgttgttgttaacttgtttattgcagcttataatggttacaaataaagcaatagcatcacaaatttcacaaataaagcatttttttcactgcattctagttgtggtttgtccaaactcatcaatgtatcttatcatgtctggatccccatcaagcatcgatgaagttcctatactttctagagaataggaacttcgaatccaccaccatggtgagcgagctgattaaggagaacatgcacatgaagctgtacatggagggcaccgtgaacaaccaccacttcaagtgcacatccgagggcgaaggcaagccctacgagggcacccagaccatgagaatcaaggcggtcgagggcggccctctccccttcgccttcgacatcctggctaccagcttcatgtacggcagcaaaaccttcatcaaccacacccagggcatccccgacttctttaagcagtccttccccgagggcttcacatgggagagagtcaccacatacgaagacgggggcgtgctgaccgctacccaggacaccagcctccaggacggctgcctcatctacaacgtcaagatcagaggggtgaacttcccatccaacggccctgtgatgcagaagaaaacactcggctgggaggcctccaccgagaccctgtaccccgctgacggcggcctggaaggcagagccgacatggccctgaagctcgtgggcgggggccacctgatctgcaacttgaagaccacatacagatccaagaaacccgctaagaacctcaagatgcccggcgtctactatgtggacagaagactggaaagaatcaaggaggccgacaaagagacctacgtcgagcagcacgaggtggctgtggccagatactgcgacctccctagcaaactggggcacagaggatccatggaagatgccaaaaacattaagaagggcccagcgccgttctacccactcgaagacgggaccgccggcgagcagctgcacaaagccatgaagcgctacgccctggtgcccggcgccatcgcctttaccgacgcacatattcaggtggacgttacctacgccgagtacttcgagatgagcgttcggctggcagaagctatgaggcgctatgggctgaatacaaaccatcggatcgtggtgtgcagcgagaatagctcgcagttcttcatgcccgtgttgggtgccctgttcatcggtgtggctgtggccccagctaacgacatctacaacgagcgcgagctgctgaacagcatgggcatcagccagcccaccgtcgtattcgtgagcaagaaagggctgcgaaaggtcctcaacgtgcaaaagaagctaccgatcatacgaaagatcatcatcatggatagcaagaccgactaccagggcttccaaagcatgtacaccttcgtgacttcccatttgccacccagcttcaacgagtacgacttcgtgcccgagagcttcgaccgggacaaaaccatcgccctgatcatgaacagtagtggtagtacaggattacccaagggcgtagccctaccgcaccgcaccgcttgtgtccgattcagtcatgcccgcgaccccatcttcggctaccagaacatccccgacaccgctatcctcagcgtggtgccatttcaccacggcttcggcatgttcaccacgctgggctacttgatctgcggctttcgggtcgtgctcatgtaccgcttcgaggaggagctattcttgcgcagcttgcaagactataagattcaatctgccctgctggtgcccacactatttagctgcctcgctaagagcactctcatcgacaagtacgacctaagcagcttgcgcgagatcgccagcggcggggcgccgctcagcaaggaggtaggtgaggccgtggccaaacgcttccgcctaccaggcatccgccagggctatggcctgacagaaacaaccaacgccgtcatgatcacccccgagggggaccgtaagcctggctcagtaggcaaggtggtgcccttcttcgaggctaaggtggtagacttggtcaccggtaagacactgggtgtgaaccagcgcggtgagctgtgcgtccgtggccccatgatcatgagcggctacgttaacaaccccgaggctacgaacgctctcatcgacaaggacggctggctgcacagcggcgacatcgcctactgggacgaggacgagcacttcttcatcgtggaccggctgaagagcctgatcaaatacaagggctaccaggtagccccagccgaactggagggcatcctgctgcaacacccctacatcttcgacgccggagtcgccggcctgcccgacgacgatgccggcgagctgcccgccgcagtcgtcgtgttggaacacggtaaaaccatgaccgagaaagagatcgtggactatgtggccagccaggttacaaccgccaagaagctgcgcggtggtgttgtgtttgtggatgaagtccctagaggatcgaccggcaagttagacgcccgcaagatccgcgagattctcactaaggccaagaaggacggcaagatcgccgtgtaactcgagataatcaacctctggattacaaaatttgtgaaagattgactggtattcttaactatgttgctccttttacgctatgtggatacgctgctttaatgcctttgtatcatgctattgcttcccgtatggctttcattttctcctccttgtataaatcctggttagttcttgccacggcggaactcatcgccgcctgccttgcccgctgctggacaggggctcggctgttgggcactgacaattccgtggtgtttatttgtgaaatttgtgatgctattgctttatttgtaaccatctagctttatttgtgaaatttgtgatgctattgctttatttgtaaccattataagctgcaataaacaagttaacaacaacaattgcattcattttatgtttcaggttcagggggagatgtgggaggttttttaaagcggccgctctagagggcccgtttaaacccgctgatcagcctcgactgtgccttctagttgccagccatctgttgtttgcccctcccccgtgccttccttgaccctggaaggtgccactcccactgtcctttcctaataaaatgaggaaattgcatcgcattgtctgagtaggtgtcattctattctggggggtggggtggggcaggacagcaagggggaggattgggaagacaatagcaggcatgctggggatgcggtgggctctatggcttctgaggcggaaagaaccagctggggctctagggggtatccccacgcgccctgtagcggcgcattaagcgcggcgggtgtggtggttacgcgcagcgtgaccgctacacttgccagcgccctagcgcccgctcctttcgctttcttcccttcctttctcgccacgttcgccggctttccccgtcaagctctaaatcgggggctccctttagggttccgatttagtgctttacggcacctcgaccccaaaaaacttgattagggtgatggttcacgtagtgggccatcgccctgatagacggtttttcgccctttgacgttggagtccacgttctttaatagtggactcttgttccaaactggaacaacactcaaccctatctcggtctattcttttgatttataagggattttgccgatttcggcctattggttaaaaaatgagctgatttaacaaaaatttaacgcgaattaattctgtggaatgtgtgtcagttagggtgtggaaagtccccaggctccccagcaggcagaagtatgcaaagcatgcatctcaattagtcagcaaccaggtgtggaaagtccccaggctccccagcaggcagaagtatgcaaagcatgcatctcaattagtcagcaaccatagtcccgcccctaactccgcccatcccgcccctaactccgcccagttccgcccattctccgccccatggctgactaattttttttatttatgcagaggccgaggccgcctctgcctctgagctattccagaagtagtgaggaggcttttttggaggcctaggcttttgcaaaaagctcccgggagcttgtatatccattttcggatctgatcaagagacaggatgaggatcgtttcgcatgattgaacaagatggattgcacgcaggttctccggccgcttgggtggagaggctattcggctatgactgggcacaacagacaatcggctgctctgatgccgccgtgttccggctgtcagcgcaggggcgcccggttctttttgtcaagaccgacctgtccggtgccctgaatgaactgcaggacgaggcagcgcggctatcgtggctggccacgacgggcgttccttgcgcagctgtgctcgacgttgtcactgaagcgggaagggactggctgctattgggcgaagtgccggggcaggatctcctgtcatctcaccttgctcctgccgagaaagtatccatcatggctgatgcaatgcggcggctgcatacgcttgatccggctacctgcccattcgaccaccaagcgaaacatcgcatcgagcgagcacgtactcggatggaagccggtcttgtcgatcaggatgatctggacgaagagcatcaggggctcgcgccagccgaactgttcgccaggctcaaggcgcgcatgcccgacggcgaggatctcgtcgtgacccatggcgatgcctgcttgccgaatatcatggtggaaaatggccgcttttctggattcatcgactgtggccggctgggtgtggcggaccgctatcaggacatagcgttggctacccgtgatattgctgaagagcttggcggcgaatgggctgaccgcttcctcgtgctttacggtatcgccgctcccgattcgcagcgcatcgccttctatcgccttcttgacgagttcttctgagcgggactctggggttcgaaatgaccgaccaagcgacgcccaacctgccatcacgagatttcgattccaccgccgccttctatgaaaggttgggcttcggaatcgttttccgggacgccggctggatgatcctccagcgcggggatctcatgctggagttcttcgcccaccccaacttgtttattgcagcttataatggttacaaataaagcaatagcatcacaaatttcacaaataaagcatttttttcactgcattctagttgtggtttgtccaaactcatcaatgtatcttatcatgtctgtataccgtcgacctctagctagagcttggcgtaatcatggtcatagctgtttcctgtgtgaaattgttatccgctcacaattccacacaacatacgagccggaagcataaagtgtaaagcctggggtgcctaatgagtgagctaactcacattaattgcgttgcgctcactgcccgctttccagtcgggaaacctgtcgtgccagctgcattaatgaatcggccaacgcgcggggagaggcggtttgcgtattgggcgctcttccgcttcctcgctcactgactcgctgcgctcggtcgttcggctgcggcgagcggtatcagctcactcaaaggcggtaatacggttatccacagaatcaggggataacgcaggaaagaacatgtgagcaaaaggccagcaaaaggccaggaaccgtaaaaaggccgcgttgctggcgtttttccataggctccgcccccctgacgagcatcacaaaaatcgacgctcaagtcagaggtggcgaaacccgacaggactataaagataccaggcgtttccccctggaagctccctcgtgcgctctcctgttccgaccctgccgcttaccggatacctgtccgcctttctcccttcgggaagcgtggcgctttctcatagctcacgctgtaggtatctcagttcggtgtaggtcgttcgctccaagctgggctgtgtgcacgaaccccccgttcagcccgaccgctgcgccttatccggtaactatcgtcttgagtccaacccggtaagacacgacttatcgccactggcagcagccactggtaacaggattagcagagcgaggtatgtaggcggtgctacagagttcttgaagtggtggcctaactacggctacactagaagaacagtatttggtatctgcgctctgctgaagccagttaccttcggaaaaagagttggtagctcttgatccggcaaacaaaccaccgctggtagcggtttttttgtttgcaagcagcagattacgcgcagaaaaaaaggatctcaagaagatcctttgatcttttctacggggtctgacgctcagtggaacgaaaactcacgttaagggattttggtcatgagattatcaaaaaggatcttcacctagatccttttaaattaaaaatgaagttttaaatcaatctaaagtatatatgagtaaacttggtctgacagttaccaatgcttaatcagtgaggcacctatctcagcgatctgtctatttcgttcatccatagttgcctgactccccgtcgtgtagataactacgatacgggagggcttaccatctggccccagtgctgcaatgataccgcgagacccacgctcaccggctccagatttatcagcaataaaccagccagccggaagggccgagcgcagaagtggtcctgcaactttatccgcctccatccagtctattaattgttgccgggaagctagagtaagtagttcgccagttaatagtttgcgcaacgttgttgccattgctacaggcatcgtggtgtcacgctcgtcgtttggtatggcttcattcagctccggttcccaacgatcaaggcgagttacatgatcccccatgttgtgcaaaaaagcggttagctccttcggtcctccgatcgttgtcagaagtaagttggccgcagtgttatcactcatggttatggcagcactgcataattctcttactgtcatgccatccgtaagatgcttttctgtgactggtgagtactcaaccaagtcattctgagaatagtgtatgcggcgaccgagttgctcttgcccggcgtcaatacgggataataccgcgccacatagcagaactttaaaagtgctcatcattggaaaacgttcttcggggcgaaaactctcaaggatcttaccgctgttgagatccagttcgatgtaacccactcgtgcacccaactgatcttcagcatcttttactttcaccagcgtttctgggtgagcaaaaacaggaaggcaaaatgccgcaaaaaagggaataagggcgacacggaaatgttgaatactcatactcttcctttttcaatattattgaagcatttatcagggttattgtctcatgagcggatacatatttgaatgtatttagaaaaataaacaaataggggttccgcgcacatttccccgaaaagtgccacctgacgtc

SEQ ID NO: 31 - DNA, 8567 bp, synthetic construct
  source 1..8567: mol_type = other DNA
  misc_feature 917..950: note = loxP
  polyA_site 964..1742
  misc_feature 1758..1791: note = loxP
  misc_feature 1807..1878: note = Flp N-ter
  misc_feature 1927..2376: note = pMag
  misc_feature 2377..2826: note = nMagHigh1
  misc_feature 2875..4068: note = Flp C-ter
gacggatcgggagatctcccgatcccctatggtgcactctcagtacaatctgctctgatgccgcatagttaagccagtatctgctccctgcttgtgtgttggaggtcgctgagtagtgcgcgagcaaaatttaagctacaacaaggcaaggcttgaccgacaattgcatgaagaatctgcttagggttaggcgttttgcgctgcttcgcgatgtacgggccagatatacgcgttgacattgattattgactagttattaatagtaatcaattacggggtcattagttcatagcccatatatggagttccgcgttacataacttacggtaaatggcccgcctggctgaccgcccaacgacccccgcccattgacgtcaataatgacgtatgttcccatagtaacgccaatagggactttccattgacgtcaatgggtggagtatttacggtaaactgcccacttggcagtacatcaagtgtatcatatgccaagtacgccccctattgacgtcaatgacggtaaatggcccgcctggcattatgcccagtacatgaccttatgggactttcctacttggcagtacatctacgtattagtcatcgctattaccatggtgatgcggttttggcagtacatcaatgggcgtggatagcggtttgactcacggggatttccaagtctccaccccattgacgtcaatgggagtttgttttggcaccaaaatcaacgggactttccaaaatgtcgtaacaactccgccccattgacgcaaatgggcggtaggcgtgtacggtgggaggtctatataagcagagctctctggctaactagagaacccactgcttactggcttatcgaaattaatacgactcactatagggagacccaagctggctagcgtttaaacttaagcttataacttcgtatagcatacattatacgaagttatggtaccgcagatctgcgactctagaggatctgcgactctagaggatcataatcagccataccacatttgtagaggttttacttgctttaaaaaacctcccacacctccccctgaacctgaaacataaaatgaatgcaattgttgttgttaacttgtttattgcagcttataatggttacaaataaagcaatagcatcacaaatttcacaaataaagcatttttttcactgcattctagttgtggtttgtccaaactcatcaatgtatcttatcatgtctggatctgcgactctagaggatcataatcagccataccacatttgtagaggttttacttgctttaaaaaacctcccacacctccccctgaacctgaaacataaaatgaatgcaattgttgttgttaacttgtttattgcagcttataatggttacaaataaagcaatagcatcacaaatttcacaaataaagcatttttttcactgcattctagttgtggtttgtccaaactcatcaatgtatcttatcatgtctggatctgcgactctagaggatcataatcagccataccacatttgtagaggttttacttgctttaaaaaacctcccacacctccccctgaacctgaaacataaaatgaatgcaattgttgttgttaacttgtttattgcagcttataatggttacaaataaagcaatagcatcacaaatttcacaaataaagcatttttttcactgcattctagttgtggtttgtccaaactcatcaatgtatcttatcatgtctggatccccatcaagcatcgatataacttcgtatagcatacattatacgaagttataagcttaccaccatgagccagttcgacatcctgtgcaagaccccccccaaggtgctggtgcggcagttcgtggagagattcgagaggctcgaggccagcccctctaaccctggagcctccaacggcagcggtacccataccctgtatgctccagggggatacgacattatgggctatcttcgtcagatcaggaaccggcccaatcctcaggttgaactggggccggttgacaccagttgcgcacttatcctgtgtgacttgaaacagaaagacaccccaattgtgtatgccagtgaggctttcctgtacatgaccggctacagcaacgctgaagtgctggggcgcaactgtcgattcctacaaagtcctgatgggatggtgaaaccgaagagcacacgcaagtatgtggatagcaacaccataaacactatgagaaaggccatagatagaaatgccgaagtccaggtggaggtagtgaactttaagaagaatggccagaggtttgtgaatttcttaactatgattccagttcgcgacgaaaccggagagtatcggtactctatgggctttcagtgcgagacagagcacaccctatacgctcccggaggctacgacatcatgggatatttggaccaaatcgggaatcggccgaatccccaggtagaactcggccctgttgataccagctgtgcgctgatcctttgcgatctgaagcagaaggatactccaatcgtatacgccagtgaagccttcctctatatgactggatatagtaacgccgaggtgctcggccggaattgcagatttctgcaatcccctgacggcatggtcaagcccaaatcaacccgtaagtacgtggattccaatactattaacacgatccgtaaggcaattgaccggaacgctgaggtgcaggtggaagttgtcaacttcaagaaaaacggtcaacgctttgtcaatttcctcacgatcatcccagtcagggatgagactggcgaatataggtattctatgggattccagtgtgagacagaactcgaggctagtcccagcaatcctggagcctccaacggctctggtacccccagcggcgagaagatcgccagctgtgccgccgagctgacctacctgtgctggatgatcacccacaacggcaccgccatcaagagggccaccttcatgagctacaacaccatcatcagcaacagcctgagcttcgacatcgtgaacaagagcctgcagttcaagtacaagacccagaaggccaccatcctggaggccagcctgaagaagctgatccccgcctgggagttcaccatcatcccttacaacggccagaagcaccagagcgacatcaccgacatcgtgtccagcctgcagctgcagttcgagagcagcgaggaggccgacaagggcaacagccacagcaagaagatgctgaaggccctgctgtccgagggcgagagcatctgggagatcaccgagaagatcctgaacagcttcgagtacaccagcaggttcaccaagaccaagaccctgtaccagttcctgttcctggccacattcatcaactgcggcaggttcagcgacatcaagaacgtggaccccaagagcttcaagctggtgcagaacaagtacctgggcgtgatcattcagtgcctggtgaccgagaccaagacaagcgtgtccaggcacatctactttttcagcgccagaggcaggatcgaccccctggtgtacctggacgagttcctgaggaacagcgagcccgtgctgaagagagtgaacaggaccggcaacagcagcagcaacaagcaggagtaccagctgctgaaggacaacctggtgcgcagctacaacaaggccctgaagaagaacgccccctaccccatcttcgctatcaagaacggccctaagagccacatcggcaggcacctgatgaccagctttctgagcatgaagggcctgaccgagctgacaaacgtggtgggcaactggagcgacaagagggcctccgccgtggccaggaccacctacacccaccagatcaccgccatccccgaccactacttcgccctggtgtccaggtactacgcctacgaccccatcagcaaggagatgatcgccctgaaggacgagaccaaccccatcgaggagtggcagcacatcgagcagctgaagggcagcgccgagggcagcatcagataccccgcctggaacggcatcatcagccaggaggtgctggactacctgagcagctacatcaacaggcggatctaatctagaaataaaagatctttattttcattagatctgtgtgttggttttttgtgtggcggccgcgggcccgtttaaacccgctgatcagcctcgactgtgccttctagttgccagccatctgttgtttgcccctcccccgtgccttccttgaccctggaaggtgccactcccactgtcctttcctaataaaatgaggaaattgcatcgcattgtctgagtaggtgtcattctattctggggggtggggtggggcaggacagcaagggggaggattgggaagacaatagcaggcatgctggggatgcggtgggctctatggcttctgaggcggaaagaaccagctggggctctagggggtatccccacgcgccctgtagcggcgcattaagcgcggcgggtgtggtggttacgcgcagcgtgaccgctacacttgccagcgccctagcgcccgctcctttcgctttcttcccttcctttctcgccacgttcgccggctttccccgtcaagctctaaatcgggggctccctttagggttccgatttagtgctttacggcacctcgaccccaaaaaacttgattagggtgatggttcacgtagtgggccatcgccctgatagacggtttttcgccctttgacgttggagtccacgttctttaatagtggactcttgttccaaactggaacaacactcaaccctatctcggtctattcttttgatttataagggattttgccgatttcggcctattggttaaaaaatgagctgatttaacaaaaatttaacgcgaattaattctgtggaatgtgtgtcagttagggtgtggaaagtccccaggctccccagcaggcagaagtatgcaaagcatgcatctcaattagtcagcaaccaggtgtggaaagtccccaggctccccagcaggcagaagtatgcaaagcatgcatctcaattagtcagcaaccatagtcccgcccctaactccgcccatcccgcccctaactccgcccagttccgcccattctccgccccatggctgactaattttttttatttatgcagaggccgaggccgcctctgcctctgagctattccagaagtagtgaggaggcttttttggaggcctaggcttttgcaaaaagctcccgggagcttgtatatccattttcggatctgatcaagagacaggatgaggatcgtttcgcatgattgaacaagatggattgcacgcaggttctccggccgcttgggtggagaggctattcggctatgactgggcacaacagacaatcggctgctctgatgccgccgtgttccggctgtcagcgcaggggcgcccggttctttttgtcaagaccgacctgtccggtgccctgaatgaactgcaggacgaggcagcgcggctatcgtggctggccacgacgggcgttccttgcgcagctgtgctcgacgttgtcactgaagcgggaagggactggctgctattgggcgaagtgccggggcaggatctcctgtcatctcaccttgctcctgccgagaaagtatccatcatggctgatgcaatgcggcggctgcatacgcttgatccggctacctgcccattcgaccaccaagcgaaacatcgcatcgagcgagcacgtactcggatggaagccggtcttgtcgatcaggatgatctggacgaagagcatcaggggctcgcgccagccgaactgttcgccaggctcaaggcgcgcatgcccgacggcgaggatctcgtcgtgacccatggcgatgcctgcttgccgaatatcatggtggaaaatggccgcttttctggattcatcgactgtggccggctgggtgtggcggaccgctatcaggacatagcgttggctacccgtgatattgctgaagagcttggcggcgaatgggctgaccgcttcctcgtgctttacggtatcgccgctcccgattcgcagcgcatcgccttctatcgccttcttgacgagttcttctgagcgggactctggggttcgaaatgaccgaccaagcgacgcccaacctgccatcacgagatttcgattccaccgccgccttctatgaaaggttgggcttcggaatcgttttccgggacgccggctggatgatcctccagcgcggggatctcatgctggagttcttcgcccaccccaacttgtttattgcagcttataatggttacaaataaagcaatagcatcacaaatttcacaaataaagcatttttttcactgcattctagttgtggtttgtccaaactcatcaatgtatcttatcatgtctgtataccgtcgacctctagctagagcttggcgtaatcatggtcatagctgtttcctgtgtgaaattgttatccgctcacaattccacacaacatacgagccggaagcataaagtgtaaagcctggggtgcctaatgagtgagctaactcacattaattgcgttgcgctcactgcccgctttccagtcgggaaacctgtcgtgccagctgcattaatgaatcggccaacgcgcggggagaggcggtttgcgtattgggcgctcttccgcttcctcgctcactgactcgctgcgctcggtcgttcggctgcggcgagcggtatcagctcactcaaaggcggtaatacggttatccacagaatcaggggataacgcaggaaagaacatgtgagcaaaaggccagcaaaaggccaggaaccgtaaaaaggccgcgttgctggcgtttttccataggctccgcccccctgacgagcatcacaaaaatcgacgctcaagtcagaggtggcgaaacccgacaggactataaagataccaggcgtttccccctggaagctccctcgtgcgctctcctgttccgaccctgccgcttaccggatacctgtccgcctttctcccttcgggaagcgtggcgctttctcatagctcacgctgtaggtatctcagttcggtgtaggtcgttcgctccaagctgggctgtgtgcacgaaccccccgttcagcccgaccgctgcgccttatccggtaactatcgtcttgagtccaacccggtaagacacgacttatcgccactggcagcagccactggtaacaggattagcagagcgaggtatgtaggcggtgctacagagttcttgaagtggtggcctaactacggctacactagaagaacagtatttggtatctgcgctctgctgaagccagttaccttcggaaaaagagttggtagctcttgatccggcaaacaaaccaccgctggtagcggtttttttgtttgcaagcagcagattacgcgcagaaaaaaaggatctcaagaagatcctttgatcttttctacggggtctgacgctcagtggaacgaaaactcacgttaagggattttggtcatgagattatcaaaaaggatcttcacctagatccttttaaattaaaaatgaagttttaaatcaatctaaagtatatatgagtaaacttggtctgacagttaccaatgcttaatcagtgaggcacctatctcagcgatctgtctatttcgttcatccatagttgcctgactccccgtcgtgtagataactacgatacgggagggcttaccatctggccccagtgctgcaatgataccgcgagacccacgctcaccggctccagatttatcagcaataaaccagccagccggaagggccgagcgcagaagtggtcctgcaactttatccgcctccatccagtctattaattgttgccgggaagctagagtaagtagttcgccagttaatagtttgcgcaacgttgttgccattgctacaggcatcgtggtgtcacgctcgtcgtttggtatggcttcattcagctccggttcccaacgatcaaggcgagttacatgatcccccatgttgtgcaaaaaagcggttagctccttcggtcctccgatcgttgtcagaagtaagttggccgcagtgttatcactcatggttatggcagcactgcataattctcttactgtcatgccatccgtaagatgcttttctgtgactggtgagtactcaaccaagtcattctgagaatagtgtatgcggcgaccgagttgctcttgcccggcgtcaatacgggataataccgcgccacatagcagaactttaaaagtgctcatcattggaaaacgttcttcggggcgaaaactctcaaggatcttaccgctgttgagatccagttcgatgtaacccactcgtgcacccaactgatcttcagcatcttttactttcaccagcgtttctgggtgagcaaaaacaggaaggcaaaatgccgcaaaaaagggaataagggcgacacggaaatgttgaatactcatactcttcctttttcaatattattgaagcatttatcagggttattgtctcatgagcggatacatatttgaatgtatttagaaaaataaacaaataggggttccgcgcacatttccccgaaaagtgccacctgacgtc

SEQ ID NO: 32 - DNA, 10249 bp, synthetic construct
  source 1..10249: mol_type = other DNA
  misc_feature 1766..1813: note = Lifeact
  misc_feature 1835..2542: note = mcherry
  misc_feature 2543..2608: note = P2A
  misc_feature 2612..3649: note = mVav2 N-ter
  misc_feature 3656..4105: note = pMag
  misc_feature 4106..4555: note = nMag
  misc_feature 4562..6208: note = mVav2 C-ter
aatattattgaagcatttatcagggttattgtctcatgagcggatacatatttgaatgtatttagaaaaataaacaaataggggttccgcgcacatttccccgaaaagtgccacctgacgtcgacggatcgggagatctcccgatcccctatggtgcactctcagtacaatctgctctgatgccgcatagttaagccagtatctgctccctgcttgtgtgttggaggtcgctgagtagtgcgcgagcaaaatttaagctacaacaaggcaaggcttgaccgacaattgcatgaagaatctgcttagggttaggcgttttgcgctgcttcgcgatgtacgggccagatatacgcgttgacattgattattgactaggcttttgcaaaaagctttgcaaagatggataaagttttaaacagagaggaatctttgcagctaatggaccttctaggtcttgaaaggagtgggaattggctccggtgcccgtcagtgggcagagcgcacatcgcccacagtccccgagaagttggggggaggggtcggcaattgaaccggtgcctagagaaggtggcgcggggtaaactgggaaagtgatgtcgtgtactggctccgcctttttcccgagggtgggggagaaccgtatataagtgcagtagtcgccgtgaacgttctttttcgcaacgggtttgccgccagaacacaggtaagtgccgtgtgtggttcccgcgggcctggcctctttacgggttatggcccttgcgtgccttgaattacttccacctggctgcagtacgtgattcttgatcccgagcttcgggttggaagtgggtgggagagttcgaggccttgcgcttaaggagccccttcgcctcgtgcttgagttgaggcctggcctgggcgctggggccgccgcgtgcgaatctggtggcaccttcgcgcctgtctcgctgctttcgataagtctctagccatttaaaatttttgatgacctgctgcgacgctttttttctggcaagatagtcttgtaaatgcgggccaagatctgcacactggtatttcggtttttggggccgcgggcggcgacggggcccgtgcgtcccagcgcacatgttcggcgaggcggggcctgcgagcgcggccaccgagaatcggacgggggtagtctcaagctggccggcctgctctggtgcctggcctcgcgccgccgtgtatcgccccgccctgggcggcaaggctggcccggtcggcaccagttgcgtgagcggaaagatggccgcttcccggccctgctgcagggagctcaaaatggaggacgcggcgctcgggagagcgggcgggtgagtcacccacacaaaggaaaagggcctttccgtcctcagccgtcgcttcatgtgactccacggagtaccgggcgccgtccaggcacctcgattagttctcgagcttttggagtacgtcgtctttaggttggggggaggggttttatgcgatggagtttccccacactgagtgggtggagactgaagttaggccagcttggcacttgatgtaattctccttggaatttgccctttttgagtttggatcttggttcattctcaagcctcagacagtggttcaaagtttttttcttccatttcaggtgtcgtgaggaattagcttggtactaatacgactcactatagggagacccaagctggctaggtaagcttggtaccgagctcggatccactagtccagtgtggtggaattcgccgccaccatgggcgtggccgacctgatcaagaagttcgagagcatcagcaaggaggagggcgacccacctgtggccaccatggtgagcaagggcgaggaggataacatggccatcatcaaggagttcatgcgcttcaaggtgcacatggagggctccgtgaacggccacgagttcgagatcgagggcgagggcgagggccgcccctacgagggcacccagaccgccaagctgaaggtgaccaagggtggccccctgcccttcgcctgggacatcctgtcccctcagttcatgtacggctccaaggcctacgtgaagcaccccgccgacatccccgactacttgaagctgtccttccccgagggcttcaagtgggagcgcgtgatgaacttcgaggacggcggcgtggtgaccgtgacccaggactcctccctgcaggacggcgagttcatctacaaggtgaagctgcgcggcaccaacttcccctccgacggccccgtaatgcagaagaagaccatgggctgggaggcctcctccgagcggatgtaccccgaggacggcgccctgaagggcgagatcaagcagaggctgaagctgaaggacggcggccactacgacgctgaggtcaagaccacctacaaggccaagaagcccgtgcagctgcccggcgcctacaacgtcaacatcaagttggacatcacctcccacaacgaggactacaccatcgtggaacagtacgaacgcgccgagggccgccactccaccggcggcatggacgagctgtacaagggaagtggtgctactaattttagtctccttaaacaagcaggtgatgtcgaagaaaatccagggccacatatggagcaatggcgccagtgtggaaggtggctgattgactgtaaagtcctgcctccgaatcacagggtggtttggccgtctgctgtcgtgtttgacctggcccaggcccttcgggacggcgtcctgctgtgccagttgctgcacaatctgtctcctggttctattgatctgaaagatatcaactttcggcctcaaatgtcccagtttctgtgcctgaagaatatccgaaccttcctgaaagtatgccatgacaaattcggtctgcgaaacagtgagcttttcgacccgtttgatctgtttgacgtgagagactttgggaaagtcatctccgctgttagtcgactgtccctgcatagcattgcccagtctaagggcattaggccattcccatccgaggagacagccgagaatgatgatgatgtgtatcgctcattggaggaactcgcagacgaacatgatcttggcgaggacatatacgactgtgttccctgcgaggacgaaggagatgacatttacgaagatatcataaaagtggaggttcagcaacctatgaaaatggggatgacagaggacgataagagatcttgctgtttgctggaaatccaggaaacagaggcaaaatactacaggactctcgaagatattgagaagaactacatggggcccctccgactcgttctgagccccgccgatatggctgccgtgtttataaatctggaggacctgatcaaggtccatcattcctttcttcgcgctatcgatgtgagcatgatggccggcggctccacacttgccaaggtgtttcttgaatttaaggaacgcttgctgatctatggcgagtattgttcacacatggaacacgcccagtcaaccctcaatcaattgctggcatccagagaggacttcaggcaaaaggtagaggaatgcaccctgagagtgcaagatggcaaatttaagttgcaggacttgttggttgtacccatgcagagggtgctcaagtaccatctgctgcttaaagaacttctctcacactctgcgaccggtcataccctgtatgctccagggggatacgacattatgggctatcttcgtcagatcaggaaccggcccaatcctcaggttgaactggggccggttgacaccagttgcgcacttatcctgtgtgacttgaaacagaaagacaccccaattgtgtatgccagtgaggctttcctgtacatgaccggctacagcaacgctgaagtgctggggcgcaactgtcgattcctacaaagtcctgatgggatggtgaaaccgaagagcacacgcaagtatgtggatagcaacaccataaacactatgagaaaggccatagatagaaatgccgaagtccaggtggaggtagtgaactttaagaagaatggccagaggtttgtgaatttcttaactatgattccagttcgcgacgaaaccggagagtatcggtactctatgggctttcagtgcgagacagagcacaccctatacgctcccggaggctacgacatcatgggatatttggaccaaatcgggaatcggccgaatccccaggtagaactcggccctgttgataccagctgtgcgctgatcctttgcgatctgaagcagaaggatactccaatcgtatacgccagtgaagccttcctctatatgactggatatagtaacgccgaggtgctcggccggaattgcagatttctgcaatcccctgacggcatggtcaagcccaaatcaacccgtaagtacgtggattccaatactattaacacgatgcgtaaggcaattgaccggaacgctgaggtgcaggtggaagttgtcaacttcaagaaaaacggtcaacgctttgtcaatttcctcacgatgatcccagtcagggatgagactggcgaatataggtattctatgggattccagtgtgagacagaaggtacccggccagagcgtcagcaactgaaggaggccctggaagccatgcaggacctggctatgtatattaacgaggttaaaagggacaaggagacactgaagaaaatctccgagtttcagtgttcaatcgagaatctccaagtgaagctggaagagttcggacggccgaagatcgacggcgaactcaaggtccggagtatagtgaatcacaccaagcaggatcgttaccttttccttttcgacaaggtggtgattgtatgcaaacggaaagggtattcatacgagctcaaggaggtcatagaactcctgttccacaagatgaccgatgaccctatgcacaacaaagacatcaagaaatggagttacgggttctacctgatccatctgcagggaaagcagggatttcagttcttctgcaagacagaagatatgaaaagaaaatggatggagcagttcgagatggccatgtctaacatcaaaccagacaaggcaaacgcgaaccatcattcttttcagatgtacactttcgacaaaaccactaactgcaaggcttgcaagatgttcctgaggggaaccttttaccagggctacctgtgtacacgatgtggcgtcggggcacacaaggagtgtctggaggttatccctccatgcaagatgagcagccctgccgatgtggatgcccctggggctggccccggtcctaaaatggttgcggtccagaattaccatgggaatcccgcaccgccaggaaaacccgtgctgactttccagacgggagatgttatagaactgttgagaggcgatcctgacagcccttggtgggaagggaggctggtgcagacgaggaagtccggatactttccaagtagtagtgtaaagccctgtcccgtggacggccggccacccactggacgcccacccagccgggagatcgattataccgcttatccatggtttgccggtaatatggaaagacaacagaccgacaacctcctgaaaagtcacgctagcggtacgtatctcatccgggaacggcccgcagaagcggaaagattcgccattagtataaagttcaacgacgaggtcaagcacatcaaggtcgtggagaaagatagctggattcacattactgaagcgaagaaatttgagtctcttctcgaactcgtggagtattatcagtgccactcactcaaagaaagcttcaagcagctggacacgacattgaaattcccatacaaaagccgcgaacgtaccacctctcgcgccagctccagaagccccgcatcctgcgcttcctataatttcagctttctgtcaccacagggcctgagcttcgctccacaagcaccctccgcacccttctggtctgtgtttactccacgagtgattggaactgccgtggctcgctataactttgcagcccgtgatatgagagagctgagcctgcgcgagggcgatgtcgtgaagatctacagcagaattggaggggaccagggttggtggaagggcgagacaaacggtaggattgggtggttcccttcaacctatgtcgaggaggagggtgtacagtaatctagagggcccttcgaaggtaagcctatccctaaccctctcctcggtctcgattctacgcgtaccggtcatcatcaccatcaccattgagtttaaacccgctgatcagcctcgactgtgccttctagttgccagccatctgttgtttgcccctcccccgtgccttccttgaccctggaaggtgccactcccactgtcctttcctaataaaatgaggaaattgcatcgcattgtctgagtaggtgtcattctattctggggggtggggtggggcaggacagcaagggggaggattgggaagacaatagcaggcatgctggggatgcggtgggctctatggcttctgaggcggaaagaaccagctggggctctagggggtatccccacgcgccctgtagcggcgcattaagcgcggcgggtgtggtggttacgcgcagcgtgaccgctacacttgccagcgccctagcgcccgctcctttcgctttcttcccttcctttctcgccacgttcgccggctttccccgtcaagctctaaatcgggggctccctttagggttccgatttagtgctttacggcacctcgaccccaaaaaacttgattagggtgatggttcacgtagtgggccatcgccctgatagacggtttttcgccctttgacgttggagtccacgttctttaatagtggactcttgttccaaactggaacaacactcaaccctatctcggtctattcttttgatttataagggattttgccgatttcggcctattggttaaaaaatgagctgatttaacaaaaatttaacgcgaattaattctgtggaatgtgtgtcagttagggtgtggaaagtccccaggctccccagcaggcagaagtatgcaaagcatgcatctcaattagtcagcaaccaggtgtggaaagtccccaggctccccagcaggcagaagtatgcaaagcatgcatctcaattagtcagcaaccatagtcccgcccctaactccgcccatcccgcccctaactccgcccagttccgcccattctccgccccatggctgactaattttttttatttatgcagaggccgaggccgcctctgcctctgagctattccagaagtagtgaggaggcttttttggaggcctaggcttttgcaaaaagctcccgggagcttgtatatccattttcggatctgatcagcacgtgttgacaattaatcatcggcatagtatatcggcatagtataatacgacaaggtgaggaactaaaccatggccaagcctttgtctcaagaagaatccaccctcattgaaagagcaacggctacaatcaacagcatccccatctctgaagactacagcgtcgccagcgcagctctctctagcgacggccgcatcttcactggtgtcaatgtatatcattttactgggggaccttgtgcagaactcgtggtgctgggcactgctgctgctgcggcagctggcaacctgacttgtatcgtcgcgatcggaaatgagaacaggggcatcttgagcccctgcggacggtgccgacaggtgcttctcgatctgcatcctgggatcaaagccatagtgaaggacagtgatggacagccgacggcagttgggattcgtgaattgctgccctctggttatgtgtgggagggctaagcacttcgtggccgaggagcaggactgacacgtgctacgagatttcgattccaccgccgccttctatgaaaggttgggcttcggaatcgttttccgggacgccggctggatgatcctccagcgcggggatctcatgctggagttcttcgcccaccccaacttgtttattgcagcttataatggttacaaataaagcaatagcatcacaaatttcacaaataaagcatttttttcactgcattctagttgtggtttgtccaaactcatcaatgtatcttatcatgtctgtatactcacggtctcgaagccgcggtgcgggtgccagggcgtgcccttgggctccccgggcgcgtactccacctcacccatctggtccagtataccgtcgacctctagctagagcttggcgtaatcatggtcatagctgtttcctgtgtgaaattgttatccgctcacaattccacacaacatacgagccggaagcataaagtgtaaagcctggggtgcctaatgagtgagctaactcacattaattgcgttgcgctcactgcccgctttccagtcgggaaacctgtcgtgccagctgcattaatgaatcggccaacgcgcggggagaggcggtttgcgtattgggcgctcttccgcttcctcgctcactgactcgctgcgctcggtcgttcggctgcggcgagcggtatcagctcactcaaaggcggtaatacggttatccacagaatcaggggataacgcaggaaagagcatgtgagcaaaaggccagcaaaaggccaggaaccgtaaaaaggccgcgttgctggcgtttttccataggctccgcccccctgacgagcatcacaaaaatcgacgctcaagtcagaggtggcgaaacccgacaggactataaagataccaggcgtttccccctggaagctccctcgtgcgctctcctgttccgaccctgccgcttaccggatacctgtccgcctttctcccttcgggaagcgtggcgctttctcatagctcacgctgtaggtatctcagttcggtgtaggtcgttcgctccaagctgggctgtgtgcacgaaccccccgttcagcccgaccgctgcgccttatccggtaactatcgtcttgagtccaacccggtaagacacgacttatcgccactggcagcagccactggtaacaggattagcagagcgaggtatgtaggcggtgctacagagttcttgaagtggtggcctaactacggctacactagaagaacagtatttggtatctgcgctctgctgaagccagttaccttcggaaaaagagttggtagctcttgatccggcaaacaaaccaccgctggtagcggtggtttttttgtttgcaagcagcagattacgcgcagaaaaaaaggatctcaagaagatcctttgatcttttctacggggtctgacgctcagtggaacgaaaactcacgttaagggattttggtcatgagattatcaaaaaggatcttcacctagatccttttaaattaaaaatgaagttttaaatcaatctaaagtatatatgagtaaacttggtctgacagttaccaatgcttaatcagtgaggcacctatctcagcgatctgtctatttcgttcatccatagttgcctgactccccgtcgtgtagataactacgatacgggagggcttaccatctggccccagtgctgcaatgataccgcgagacccacgctcaccggctccagatttatcagcaataaaccagccagccggaagggccgagcgcagaagtggtcctgcaactttatccgcctccatccagtctattaattgttgccgggaagctagagtaagtagttcgccagttaatagtttgcgcaacgttgttgccattgctacaggcatcgtggtgtcacgctcgtcgtttggtatggcttcattcagctccggttcccaacgatcaaggcgagttacatgatcccccatgttgtgcaaaaaagcggttagctccttcggtcctccgatcgttgtcagaagtaagttggccgcagtgttatcactcatggttatggcagcactgcataattctcttactgtcatgccatccgtaagatgcttttctgtgactggtgagtactcaaccaagtcattctgagaatagtgtatgcggcgaccgagttgctcttgcccggcgtcaatacgggataataccgcgccacatagcagaactttaaaagtgctcatcattggaaaacgttcttcggggcgaaaactctcaaggatcttaccgctgttgagatccagttcgatgtaacccactcgtgcacccaactgatcttcagcatcttttactttcaccagcgtttctgggtgagcaaaaacaggaaggcaaaatgccgcaaaaaagggaataagggcgacacggaaatgttgaatactcatactcttcctttttc

SEQ ID NO: 33 - DNA, 10915 bp, synthetic construct
  source 1..10915: mol_type = other DNA
  misc_feature 1766..1813: note = Lifeact
  misc_feature 1835..2542: note = mcherry
  misc_feature 2543..2608: note = P2A
  misc_feature 2612..3649: note = mVav2 N-ter
  misc_feature 3656..4105: note = pMag
  misc_feature 4106..4771: note = mTagBFP2
  misc_feature 4772..5221: note = nMag
  misc_feature 5228..6790: note = mVav2 C-ter
aatattattgaagcatttatcagggttattgtctcatgagcggatacatatttgaatgtatttagaaaaataaacaaataggggttccgcgcacatttccccgaaaagtgccacctgacgtcgacggatcgggagatctcccgatcccctatggtgcactctcagtacaatctgctctgatgccgcatagttaagccagtatctgctccctgcttgtgtgttggaggtcgctgagtagtgcgcgagcaaaatttaagctacaacaaggcaaggcttgaccgacaattgcatgaagaatctgcttagggttaggcgttttgcgctgcttcgcgatgtacgggccagatatacgcgttgacattgattattgactaggcttttgcaaaaagctttgcaaagatggataaagttttaaacagagaggaatctttgcagctaatggaccttctaggtcttgaaaggagtgggaattggctccggtgcccgtcagtgggcagagcgcacatcgcccacagtccccgagaagttggggggaggggtcggcaattgaaccggtgcctagagaaggtggcgcggggtaaactgggaaagtgatgtcgtgtactggctccgcctttttcccgagggtgggggagaaccgtatataagtgcagtagtcgccgtgaacgttctttttcgcaacgggtttgccgccagaacacaggtaagtgccgtgtgtggttcccgcgggcctggcctctttacgggttatggcccttgcgtgccttgaattacttccacctggctgcagtacgtgattcttgatcccgagcttcgggttggaagtgggtgggagagttcgaggccttgcgcttaaggagccccttcgcctcgtgcttgagttgaggcctggcctgggcgctggggccgccgcgtgcgaatctggtggcaccttcgcgcctgtctcgctgctttcgataagtctctagccatttaaaatttttgatgacctgctgcgacgctttttttctggcaagatagtcttgtaaatgcgggccaagatctgcacactggtatttcggtttttggggccgcgggcggcgacggggcccgtgcgtcccagcgcacatgttcggcgaggcggggcctgcgagcgcggccaccgagaatcggacgggggtagtctcaagctggccggcctgctctggtgcctggcctcgcgccgccgtgtatcgccccgccctgggcggcaaggctggcccggtcggcaccagttgcgtgagcggaaagatggccgcttcccggccctgctgcagggagctcaaaatggaggacgcggcgctcgggagagcgggcgggtgagtcacccacacaaaggaaaagggcctttccgtcctcagccgtcgcttcatgtgactccacggagtaccgggcgccgtccaggcacctcgattagttctcgagcttttggagtacgtcgtctttaggttggggggaggggttttatgcgatggagtttccccacactgagtgggtggagactgaagttaggccagcttggcacttgatgtaattctccttggaatttgccctttttgagtttggatcttggttcattctcaagcctcagacagtggttcaaagtttttttcttccatttcaggtgtcgtgaggaattagcttggtactaatacgactcactatagggagacccaagctggctaggtaagcttggtaccgagctcggatccactagtccagtgtggtggaattcgccgccaccatgggcgtggccgacctgatcaagaagttcgagagcatcagcaaggaggagggcgacccacctgtggccaccatggtgagcaagggcgaggaggataacatggccatcatcaaggagttcatgcgcttcaaggtgcacatggagggctccgtgaacggccacgagttcgagatcgagggcgagggcgagggccgcccctacgagggcacccagaccgccaagctgaaggtgaccaagggtggccccctgcccttcgcctgggacatcctgtcccctcagttcatgtacggctccaaggcctacgtgaagcaccccgccgacatccccgactacttgaagctgtccttccccgagggcttcaagtgggagcgcgtgatgaacttcgaggacggcggcgtggtgaccgtgacccaggactcctccctgcaggacggcgagttcatctacaaggtgaagctgcgcggcaccaacttcccctccgacggccccgtaatgcagaagaagaccatgggctgggaggcctcctccgagcggatgtaccccgaggacggcgccctgaagggcgagatcaagcagaggctgaagctgaaggacggcggccactacgacgctgaggtcaagaccacctacaaggccaagaagcccgtgcagctgcccggcgcctacaacgtcaacatcaagttggacatcacctcccacaacgaggactacaccatcgtggaacagtacgaacgcgccgagggccgccactccaccggcggcatggacgagctgtacaagggaagtggtgctactaattttagtctccttaaacaagcaggtgatgtcgaagaaaatccagggccacatatggagcaatggcgccagtgtggaaggtggctgattgactgtaaagtcctgcctccgaatcacagggtggtttggccgtctgctgtcgtgtttgacctggcccaggcccttcgggacggcgtcctgctgtgccagttgctgcacaatctgtctcctggttctattgatctgaaagatatcaactttcggcctcaaatgtcccagtttctgtgcctgaagaatatccgaaccttcctgaaagtatgccatgacaaattcggtctgcgaaacagtgagcttttcgacccgtttgatctgtttgacgtgagagactttgggaaagtcatctccgctgttagtcgactgtccctgcatagcattgcccagtctaagggcattaggccattcccatccgaggagacagccgagaatgatgatgatgtgtatcgctcattggaggaactcgcagacgaacatgatcttggcgaggacatatacgactgtgttccctgcgaggacgaaggagatgacatttacgaagatatcataaaagtggaggttcagcaacctatgaaaatggggatgacagaggacgataagagatcttgctgtttgctggaaatccaggaaacagaggcaaaatactacaggactctcgaagatattgagaagaactacatggggcccctccgactcgttctgagccccgccgatatggctgccgtgtttataaatctggaggacctgatcaaggtccatcattcctttcttcgcgctatcgatgtgagcatgatggccggcggctccacacttgccaaggtgtttcttgaatttaaggaacgcttgctgatctatggcgagtattgttcacacatggaacacgcccagtcaaccctcaatcaattgctggcatccagagaggacttcaggcaaaaggtagaggaatgcaccctgagagtgcaagatggcaaatttaagttgcaggacttgttggttgtacccatgcagagggtgctcaagtaccatctgctgcttaaagaacttctctcacactctgcgaccggtcataccctgtatgctccagggggatacgacattatgggctatcttcgtcagatcaggaaccggcccaatcctcaggttgaactggggccggttgacaccagttgcgcacttatcctgtgtgacttgaaacagaaagacaccccaattgtgtatgccagtgaggctttcctgtacatgaccggctacagcaacgctgaagtgctggggcgcaactgtcgattcctacaaagtcctgatgggatggtgaaaccgaagagcacacgcaagtatgtggatagcaacaccataaacactatgagaaaggccatagatagaaatgccgaagtccaggtggaggtagtgaactttaagaagaatggccagaggtttgtgaatttcttaactatgattccagttcgcgacgaaaccggagagtatcggtactctatgggctttcagtgcgagacagaggagctgattaaggagaacatgcacatgaagctgtacatggagggcaccgtggacaaccatcacttcaagtgcacatccgagggcgaaggcaagccctacgagggcacccagaccatgagaatcaaggtggtcgagggcggccctctccccttcgccttcgacatcctggctactagcttcctctacggcagcaagaccttcatcaaccacacccagggcatccccgacttcttcaagcagtccttccctgagggcttcacatgggagagagtcaccacatacgaagacgggggcgtgctgaccgctacccaggacaccagcctccaggacggctgcctcatctacaacgtcaagatcagaggggtgaacttcacatccaacggccctgtgatgcagaagaaaacactcggctgggaggccttcaccgagacgctgtaccccgctgacggcggcctggaaggcagaaacgacatggccctgaagctcgtgggcgggagccatctgatcgcaaacgccaagaccacatatagatccaagaaacccgctaagaacctcaagatgcctggcgtctactatgtggactacagactggaaagaatcaaggaggccaacaacgagacctacgtcgagcagcacgaggtggcagtggccagatactgcgacctccacaccctatacgctcccggaggctacgacatcatgggatatttggaccaaatcgggaatcggccgaatccccaggtagaactcggccctgttgataccagctgtgcgctgatcctttgcgatctgaagcagaaggatactccaatcgtatacgccagtgaagccttcctctatatgactggatatagtaacgccgaggtgctcggccggaattgcagatttctgcaatcccctgacggcatggtcaagcccaaatcaacccgtaagtacgtggattccaatactattaacacgatgcgtaaggcaattgaccggaacgctgaggtgcaggtggaagttgtcaacttcaagaaaaacggtcaacgctttgtcaatttcctcacgatgatcccagtcagggatgagactggcgaatataggtattctatgggattccagtgtgagacagaaggtacccggccagagcgtcagcaactgaaggaggccctggaagccatgcaggacctggctatgtatattaacgaggttaaaagggacaaggagacactgaagaaaatctccgagtttcagtgttcaatcgagaatctccaagtgaagctggaagagttcggacggccgaagatcgacggcgaactcaaggtccggagtatagtgaatcacaccaagcaggatcgttaccttttccttttcgacaaggtggtgattgtatgcaaacggaaagggtattcatacgagctcaaggaggtcatagaactcctgttccacaagatgaccgatgaccctatgcacaacaaagacatcaagaaatggagttacgggttctacctgatccatctgcagggaaagcagggatttcagttcttctgcaagacagaagatatgaaaagaaaatggatggagcagttcgagatggccatgtctaacatcaaaccagacaaggcaaacgcgaaccatcattcttttcagatgtacactttcgacaaaaccactaactgcaaggcttgcaagatgttcctgaggggaaccttttaccagggctacctgtgtacacgatgtggcgtcggggcacacaaggagtgtctggaggttatccctccatgcaagatgagcagccctgccgatgtggatgcccctggggctggccccggtcctaaaatggttgcggtccagaattaccatgggaatcccgcaccgccaggaaaacccgtgctgactttccagacgggagatgttatagaactgttgagaggcgatcctgacagcccttggtgggaagggaggctggtgcagacgaggaagtccggatactttccaagtagtagtgtaaagccctgtcccgtggacggccggccacccactggacgcccacccagccgggagatcgattataccgcttatccatggtttgccggtaatatggaaagacaacagaccgacaacctcctgaaaagtcacgctagcggtacgtatctcatccgggaacggcccgcagaagcggaaagattcgccattagtataaagttcaacgacgaggtcaagcacatcaaggtcgtggagaaagatagctggattcacattactgaagcgaagaaatttgagtctcttctcgaactcgtggagtattatcagtgccactcactcaaagaaagcttcaagcagctggacacgacattgaaattcccatacaaaagccgcgaacgtaccacctctcgcgccagctccagaagccccgcatcctgcgcttcctataatttcagctttctgtcaccacagggcctgagcttcgctccacaagcaccctccgcacccttctggtctgtgtttactccacgagtgattggaactgccgtggctcgctataactttgcagcccgtgatatgagagagctgagcctgcgcgagggcgatgtcgtgaagatctacagcagaattggaggggaccagggttggtggaagggcgagacaaacggtaggattgggtggttcccttcaacctatgtcgaggaggagggtgtacagtaatctagagggcccttcgaaggtaagcctatccctaaccctctcctcggtctcgattctacgcgtaccggtcatcatcaccatcaccattgagtttaaacccgctgatcagcctcgactgtgccttctagttgccagccatctgttgtttgcccctcccccgtgccttccttgaccctggaaggtgccactcccactgtcctttcctaataaaatgaggaaattgcatcgcattgtctgagtaggtgtcattctattctggggggtggggtggggcaggacagcaagggggaggattgggaagacaatagcaggcatgctggggatgcggtgggctctatggcttctgaggcggaaagaaccagctggggctctagggggtatccccacgcgccctgtagcggcgcattaagcgcggcgggtgtggtggttacgcgcagcgtgaccgctacacttgccagcgccctagcgcccgctcctttcgctttcttcccttcctttctcgccacgttcgccggctttccccgtcaagctctaaatcgggggctccctttagggttccgatttagtgctttacggcacctcgaccccaaaaaacttgattagggtgatggttcacgtagtgggccatcgccctgatagacggtttttcgccctttgacgttggagtccacgttctttaatagtggactcttgttccaaactggaacaacactcaaccctatctcggtctattcttttgatttataagggattttgccgatttcggcctattggttaaaaaatgagctgatttaacaaaaatttaacgcgaattaattctgtggaatgtgtgtcagttagggtgtggaaagtccccaggctccccagcaggcagaagtatgcaaagcatgcatctcaattagtcagcaaccaggtgtggaaagtccccaggctccccagcaggcagaagtatgcaaagcatgcatctcaattagtcagcaaccatagtcccgcccctaactccgcccatcccgcccctaactccgcccagttccgcccattctccgccccatggctgactaattttttttatttatgcagaggccgaggccgcctctgcctctgagctattccagaagtagtgaggaggcttttttggaggcctaggcttttgcaaaaagctcccgggagcttgtatatccattttcggatctgatcagcacgtgttgacaattaatcatcggcatagtatatcggcatagtataatacgacaaggtgaggaactaaaccatggccaagcctttgtctcaagaagaatccaccctcattgaaagagcaacggctacaatcaacagcatccccatctctgaagactacagcgtcgccagcgcagctctctctagcgacggccgcatcttcactggtgtcaatgtatatcattttactgggggaccttgtgcagaactcgtggtgctgggcactgctgctgctgcggcagctggcaacctgacttgtatcgtcgcgatcggaaatgagaacaggggcatcttgagcccctgcggacggtgccgacaggtgcttctcgatctgcatcctgggatcaaagccatagtgaaggacagtgatggacagccgacggcagttgggattcgtgaattgctgccctctggttatgtgtgggagggctaagcacttcgtggccgaggagcaggactgacacgtgctacgagatttcgattccaccgccgccttctatgaaaggttgggcttcggaatcgttttccgggacgccggctggatgatcctccagcgcggggatctcatgctggagttcttcgcccaccccaacttgtttattgcagcttataatggttacaaataaagcaatagcatcacaaatttcacaaataaagcatttttttcactgcattctagttgtggtttgtccaaactcatcaatgtatcttatcatgtctgtatactcacggtctcgaagccgcggtgcgggtgccagggcgtgcccttgggctccccgggcgcgtactccacctcacccatctggtccagtataccgtcgacctctagctagagcttggcgtaatcatggtcatagctgtttcctgtgtgaaattgttatccgctcacaattccacacaacatacgagccggaagcataaagtgtaaagcctggggtgcctaatgagtgagctaactcacattaattgcgttgcgctcactgcccgctttccagtcgggaaacctgtcgtgccagctgcattaatgaatcggccaacgcgcggggagaggcggtttgcgtattgggcgctcttccgcttcctcgctcactgactcgctgcgctcggtcgttcggctgcggcgagcggtatcagctcactcaaaggcggtaatacggttatccacagaatcaggggataacgcaggaaagagcatgtgagcaaaaggccagcaaaaggccaggaaccgtaaaaaggccgcgttgctggcgtttttccataggctccgcccccctgacgagcatcacaaaaatcgacgctcaagtcagaggtggcgaaacccgacaggactataaagataccaggcgtttccccctggaagctccctcgtgcgctctcctgttccgaccctgccgcttaccggatacctgtccgcctttctcccttcgggaagcgtggcgctttctcatagctcacgctgtaggtatctcagttcggtgtaggtcgttcgctccaagctgggctgtgtgcacgaaccccccgttcagcccgaccgctgcgccttatccggtaactatcgtcttgagtccaacccggtaagacacgacttatcgccactggcagcagccactggtaacaggattagcagagcgaggtatgtaggcggtgctacagagttcttgaagtggtggcctaactacggctacactagaagaacagtatttggtatctgcgctctgctgaagccagttaccttcggaaaaagagttggtagctcttgatccggcaaacaaaccaccgctggtagcggtggtttttttgtttgcaagcagcagattacgcgcagaaaaaaaggatctcaagaagatcctttgatcttttctacggggtctgacgctcagtggaacgaaaactcacgttaagggattttggtcatgagattatcaaaaaggatcttcacctagatccttttaaattaaaaatgaagttttaaatcaatctaaagtatatatgagtaaacttggtctgacagttaccaatgcttaatcagtgaggcacctatctcagcgatctgtctatttcgttcatccatagttgcctgactccccgtcgtgtagataactacgatacgggagggcttaccatctggccccagtgctgcaatgataccgcgagacccacgctcaccggctccagatttatcagcaataaaccagccagccggaagggccgagcgcagaagtggtcctgcaactttatccgcctccatccagtctattaattgttgccgggaagctagagtaagtagttcgccagttaatagtttgcgcaacgttgttgccattgctacaggcatcgtggtgtcacgctcgtcgtttggtatggcttcattcagctccggttcccaacgatcaaggcgagttacatgatcccccatgttgtgcaaaaaagcggttagctccttcggtcctccgatcgttgtcagaagtaagttggccgcagtgttatcactcatggttatggcagcactgcataattctcttactgtcatgccatccgtaagatgcttttctgtgactggtgagtactcaaccaagtcattctgagaatagtgtatgcggcgaccgagttgctcttgcccggcgtcaatacgggataataccgcgccacatagcagaactttaaaagtgctcatcattggaaaacgttcttcggggcgaaaactctcaaggatcttaccgctgttgagatccagttcgatgtaacccactcgtgcacccaactgatcttcagcatcttttactttcaccagcgtttctgggtgagcaaaaacaggaaggcaaaatgccgcaaaaaagggaataagggcgacacggaaatgttgaatactcatactcttcctttttc

SEQ ID NO: 34 - protein, 20 aa, synthetic peptide
GSGGGSGGGSGGGSGGGSGS

SEQ ID NO: 35 - protein, 20 aa, synthetic peptide
GSAEAAAKAGSAEAAAKAGS

SEQ ID NO: 36 - protein, 150 aa, Neurospora crassa
HTLYAPGGYDIMGYLIQIMNRPNPQVELGPVDTSCALILCDLKQKDTPIVYASEAFLYMTGYSNAEVLGRNCRFLQSPDGMVKPKSTRKYVDSNTINTMRKAIDRNAEVQVEVVNFKKNGQRFVNFLTMIPVRDETGEYRYSMGFQCETE

SEQ ID NO: 37 - protein, 150 aa, Neurospora crassa
HTLYAPGGYDIMGYLRQIRNRPNPQVELGPVDTSCALILCDLKQKDTPIVYASEAFLYMTGYSNAEVLGRNCRFLQSPDGMVKPKSTRKYVDSNTINTMRKAIDRNAEVQVEVVNFKKNGQRFVNFLTMIPVRDETGEYRYSMGFQCETE

SEQ ID NO: 38 - protein, 150 aa, Neurospora crassa
HTLYAPGGYDIMGYLDQIGNRPNPQVELGPVDTSCALILCDLKQKDTPIVYASEAFLYMTGYSNAEVLGRNCRFLQSPDGMVKPKSTRKYVDSNTINTMRKAIDRNAEVQVEVVNFKKNGQRFVNFLTMIPVRDETGEYRYSMGFQCETE